European Patent Application EP 4 382 913 A2, published June 12, 2024. Title: MODULATING EXPRESSION OF POLYPEPTIDES VIA NEW GENE SWITCH EXPRESSION SYSTEMS. Applicant: Intrexon Corporation. Application US, filed January 10, 2018. The sequence listing filed with the application follows.

SEQUENCE LISTING (244 sequences)

SEQ ID NO: 1 - DNA, 54 bp, synthetic construct
  misc_feature 1..54: note = source = /note="Description of Artificial Sequence: Synthetic oligonucleotide"
  misc_feature 1..54: note = source = /note="Whitlow Linker"
  source 1..54: mol_type = other DNA
ggcagcacctccggcagcggcaagcctggcagcggcgagggcagcaccaagggc

SEQ ID NO: 2 - DNA, 78 bp, synthetic construct
  misc_feature 1..78: note = source = /note="Description of Artificial Sequence: Synthetic oligonucleotide"
  misc_feature 1..78: note = source = /note="Linker"
  source 1..78: mol_type = other DNA
tctggcggaggatctggaggaggcggatctggaggaggaggcagtggaggcggaggatctggcggaggatctctgcag

SEQ ID NO: 3 - skipped

SEQ ID NO: 4 - DNA, 12 bp, synthetic construct
  misc_feature 1..12: note = source = /note="Description of Artificial Sequence: Synthetic oligonucleotide"
  misc_feature 1..12: note = source = /note="SGSG linker"
  source 1..12: mol_type = other DNA
agtggcagcggc

SEQ ID NO: 5 - DNA, 45 bp, synthetic construct
  misc_feature 1..45: note = source = /note="Description of Artificial Sequence: Synthetic oligonucleotide"
  misc_feature 1..45: note = source = /note="(G4S)3 linker"
  source 1..45: mol_type = other DNA
ggtggcggtggctcgggcggtggtgggtcgggtggcggcggatct

SEQ ID NO: 6 - DNA, 12 bp, synthetic construct
  misc_feature 1..12: note = source = /note="Description of Artificial Sequence: Synthetic oligonucleotide"
  misc_feature 1..12: note = source = /note="Furin cleavage site/ Furinlink1"
  source 1..12: mol_type = other DNA
cgtgcaaagcgt

SEQ ID NO: 7 - DNA, 84 bp, Foot-and-mouth disease virus
  misc_feature 1..84: note = source = /note="Fmdv"
  source 1..84: mol_type = unassigned DNA
agagccaagagggcaccggtgaaacagactttgaattttgaccttctgaagttggcaggagacgttgagtccaaccctgggccc

SEQ ID NO: 8 - DNA, 54 bp, Thosea asigna virus
  misc_feature 1..54: note = source = /note="Thosea asigna virus 2A region (T2A)"
  source 1..54: mol_type = unassigned DNA
gagggcagaggaagtctgctaacatgcggtgacgtcgaggagaatcctggacct

SEQ ID NO: 9 - DNA, 75 bp, synthetic construct
  misc_feature 1..75: note = source = /note="Description of Artificial Sequence: Synthetic oligonucleotide"
  misc_feature 1..75: note = source = /note="Furin-GSG-T2A"
  source 1..75: mol_type = other DNA
agagctaagaggggaagcggagagggcagaggaagtctgctaacatgcggtgacgtcgaggagaatcctggacct

SEQ ID NO: 10 - DNA, 78 bp, synthetic construct
  misc_feature 1..78: note = source = /note="Description of Artificial Sequence: Synthetic oligonucleotide"
  misc_feature 1..78: note = source = /note="Furin-SGSG-T2A"
  source 1..78: mol_type = other DNA
agggccaagaggagtggcagcggcgagggcagaggaagtcttctaacatgcggtgacgtggaggagaatcccggccct

SEQ ID NO: 11 - DNA, 57 bp, Porcine teschovirus
  misc_feature 1..57: note = source = /note="Porcine teschovirus-1 2A region (P2A)"
  source 1..57: mol_type = unassigned DNA
gcaacgaacttctctctcctaaaacaggctggtgatgtggaggagaatcctggtcca

SEQ ID NO: 12 - DNA, 66 bp, synthetic construct
  misc_feature 1..66: note = source = /note="Description of Artificial Sequence: Synthetic oligonucleotide"
  misc_feature 1..66: note = source = /note="GSG-P2A"
  source 1..66: mol_type = other DNA
ggaagcggagctactaacttcagcctgctgaagcaggctggagacgtggaggagaaccctggacct

SEQ ID NO: 13 - DNA, 60 bp, Equine rhinitis A virus
  misc_feature 1..60: note = source = /note="Equine rhinitis A virus 2A region (E2A)"
  source 1..60: mol_type = unassigned DNA
cagtgtactaattatgctctcttgaaattggctggagatgttgagagcaaccctggacct

SEQ ID NO: 14 - DNA, 66 bp, Foot-and-mouth disease virus
  misc_feature 1..66: note = source = /note="Foot-and-mouth disease virus 2A region (F2A)"
  source 1..66: mol_type = unassigned DNA
gtcaaacagaccctaaactttgatctgctaaaactggccggggatgtggaaagtaatcccggcccc

SEQ ID NO: 15 - DNA, 93 bp, synthetic construct
  misc_feature 1..93: note = source = /note="Description of Artificial Sequence: Synthetic oligonucleotide"
  misc_feature 1..93: note = source = /note="FP2A"
  source 1..93: mol_type = other DNA
cgtgcaaagcgtgcaccggtgaaacagggaagcggagctactaacttcagcctgctgaagcaggctggagacgtggaggagaaccctggacct

SEQ ID NO: 16 - DNA, 24 bp, synthetic construct
  misc_feature 1..24: note = source = /note="Description of Artificial Sequence: Synthetic oligonucleotide"
  misc_feature 1..24: note = source = /note="Linker-GSG"
  source 1..24: mol_type = other DNA
gcaccggtgaaacagggaagcgga

SEQ ID NO: 17 - DNA, 15 bp, synthetic construct
  misc_feature 1..15: note = source = /note="Description of Artificial Sequence: Synthetic oligonucleotide"
  misc_feature 1..15: note = source = /note="Linker"
  source 1..15: mol_type = other DNA
gcaccggtgaaacag

SEQ ID NO: 18 - DNA, 570 bp, Encephalomyocarditis virus
  misc_feature 1..570: note = source = /note="EMCV IRES"
  source 1..570: mol_type = unassigned DNA
ccccctctccctcccccccccctaacgttactggccgaagccgcttggaataaggccggtgtgcgtttgtctatatgttattttccaccatattgccgtcttttggcaatgtgagggcccggaaacctggccctgtcttcttgacgagcattcctaggggtctttcccctctcgccaaaggaatgcaaggtctgttgaatgtcgtgaaggaagcagttcctctggaagcttcttgaagacaaacaacgtctgtagcgaccctttgcaggcagcggaaccccccacctggcgacaggtgcctctgcggccaaaagccacgtgtataagatacacctgcaaaggcggcacaaccccagtgccacgttgtgagttggatagttgtggaaagagtcaaatggctctcctcaagcgtattcaacaaggggctgaaggatgcccagaaggtaccccattgtatgggatctgatctggggcctcggtgcacatgctttacatgtgtttagtcgaggttaaaaaacgtctaggccccccgaaccacggggacgtggttttcctttgaaaaacacgatc

SEQ ID NO: 19 - DNA, 73 bp, synthetic construct
  misc_feature 1..73: note = source = /note="Description of Artificial Sequence: Synthetic oligonucleotide"
  misc_feature 1..73: note = source = /note="2xRbm3 IRES"
  source 1..73: mol_type = other DNA
actagttttataatttcttcttccagaatttctgacattttataatttcttcttccagaagactcacaacctc

SEQ ID NO: 20 - DNA, 66 bp, synthetic construct
  misc_feature 1..66: note = source = /note="Description of Artificial Sequence: Synthetic oligonucleotide"
  misc_feature 1..66: note = source = /note="GM-CSFR-alpha signal peptide"
  source 1..66: mol_type = other DNA
atgcttctcctggtgacaagccttctgctctgtgagttaccacacccagcattcctcctgatccca

SEQ ID NO: 21 - DNA, 66 bp, synthetic construct
  misc_feature 1..66: note = source = /note="Description of Artificial Sequence: Synthetic oligonucleotide"
  misc_feature 1..66: note = source = /note="GM-CSFR-alpha signal peptide"
  source 1..66: mol_type = other DNA
atgctgctgctggtgaccagcctgctgctgtgtgagctgccccaccccgcctttctgctgatcccc

SEQ ID NO: 22 - DNA, 60 bp, synthetic construct
  misc_feature 1..60: note = source = /note="Description of Artificial Sequence: Synthetic oligonucleotide"
  misc_feature 1..60: note = source = /note="Ig Kappa signal peptide"
  source 1..60: mol_type = other DNA
atgaggctccctgctcagctcctggggctgctaatgctctgggtcccaggatccagtggg

SEQ ID NO: 23 - DNA, 54 bp, synthetic construct
  misc_feature 1..54: note = source = /note="Description of Artificial Sequence: Synthetic oligonucleotide"
  misc_feature 1..54: note = source = /note="IgE signal peptide"
  source 1..54: mol_type = other DNA
atggattggacctggattctgtttctggtggccgctgccacaagagtgcacagc

SEQ ID NO: 24 - DNA, 63 bp, synthetic construct
  misc_feature 1..63: note = source = /note="Description of Artificial Sequence: Synthetic oligonucleotide"
  misc_feature 1..63: note = source = /note="CD8-alpha signal peptide"
  source 1..63: mol_type = other DNA
atggcgctgcccgtgaccgccttgctcctgccgctggccttgctgctccacgccgccaggccg

SEQ ID NO: 25 - DNA, 63 bp, synthetic construct
  misc_feature 1..63: note = source = /note="Description of Artificial Sequence: Synthetic oligonucleotide"
  misc_feature 1..63: note = source = /note="CD8-alpha signal peptide"
  source 1..63: mol_type = other DNA
atggccttaccagtgaccgccttgctcctgccgctggccttgctgctccacgccgccaggccg

SEQ ID NO: 26 - DNA, 63 bp, synthetic construct
  misc_feature 1..63: note = source = /note="Description of Artificial Sequence: Synthetic oligonucleotide"
  misc_feature 1..63: note = source = /note="TVB2(T21A)signal peptide"
  source 1..63: mol_type = other DNA
atgggcaccagcctcctctgctggatggccctgtgtctcctgggggcagatcacgcagatgct

SEQ ID NO: 27 - DNA, 72 bp, synthetic construct
  misc_feature 1..72: note = source = /note="Description of Artificial Sequence: Synthetic oligonucleotide"
  misc_feature 1..72: note = source = /note="CD52 signal peptide"
  source 1..72: mol_type = other DNA
atgaagcgcttcctcttcctcctactcaccatcagcctcctggttatggtacagatacaaactggactctca

SEQ ID NO: 28 - DNA, 84 bp, synthetic construct
  misc_feature 1..84: note = source = /note="Description of Artificial Sequence: Synthetic oligonucleotide"
  misc_feature 1..84: note = source = /note="Low-affinity nerve growth factor receptor (LNGFR, TNFRSF16) signal peptide"
  source 1..84: mol_type = other DNA
atgggggcaggtgccaccggccgcgccatggacgggccgcgcctgctgctgttgctgcttctgggggtgtcccttggaggtgcc

SEQ ID NO: 29 - DNA, 141 bp, synthetic construct
  misc_feature 1..141: note = source = /note="Description of Artificial Sequence: Synthetic polynucleotide"
  misc_feature 1..141: note = source = /note="CD8-alpha hinge region"
  source 1..141: mol_type = other DNA
aagcccaccaccacccctgcccctagacctccaaccccagcccctacaatcgccagccagcccctgagcctgaggcccgaagcctgtagacctgccgctggcggagccgtgcacaccagaggcctggatttcgcctgcgac

SEQ ID NO: 30 - DNA, 282 bp, synthetic construct
  misc_feature 1..282: note = source = /note="Description of Artificial Sequence: Synthetic polynucleotide"
  misc_feature 1..282: note = source = /note="CD8 alpha 2x"
  source 1..282: mol_type = other DNA
aaacctactacaactcctgccccccggcctcctacaccagctcctactatcgcctcccagccactcagtctcagacccgaggcttctaggccagcggccggaggcgcggtccacacccgcgggctggactttgcatccgataagcccaccaccacccctgcccctagacctccaaccccagcccctacaatcgccagccagcccctgagcctgaggcccgaagcctgtagacctgccgctggcggagccgtgcacaccagaggcctggatttcgcctgcgac

SEQ ID NO: 31 - DNA, 423 bp, synthetic construct
  misc_feature 1..423: note = source = /note="Description of Artificial Sequence: Synthetic polynucleotide"
  misc_feature 1..423: note = source = /note="CD8 alpha 3x"
  source 1..423: mol_type = other DNA
aagcctaccaccacccccgcacctcgtcctccaacccctgcacctacgattgccagtcagcctctttcactgcggcctgaggccagcagaccagctgccggcggtgccgtccatacaagaggactggacttcgcgtccgataaacctactaccactccagccccaaggcccccaaccccagcaccgactatcgcatcacagcctttgtcactgcgtcctgaagccagccggccagctgcagggggggccgtccacacaaggggactcgactttgcgagtgataagcccaccaccacccctgcccctagacctccaaccccagcccctacaatcgccagccagcccctgagcctgaggcccgaagcctgtagacctgccgctggcggagccgtgcacaccagaggcctggatttcgcctgcgac

SEQ ID NO: 32 - DNA, 564 bp, synthetic construct
  misc_feature 1..564: note = source = /note="Description of Artificial Sequence: Synthetic polynucleotide"
  misc_feature 1..564: note = source = /note="CD8 alpha 4x"
  source 1..564: mol_type = other DNA
aagcctaccaccacccccgcacctcgtcctccaacccctgcacctacgattgccagtcagcctctttcactgcggcctgaggccagcagaccagctgccggcggtgccgtccatacaagaggactggacttcgcgtccgataaacctactaccactccagccccaaggcccccaaccccagcaccgactatcgcatcacagcctttgtcactgcgtcctgaagccagccggccagctgcagggggggccgtccacacaaggggactcgactttgcgagtgataaacctactacaactcctgccccccggcctcctacaccagctcctactatcgcctcccagccactcagtctcagacccgaggcttctaggccagcggccggaggcgcggtccacacccgcgggctggactttgcatccgataagcccaccaccacccctgcccctagacctccaaccccagcccctacaatcgccagccagcccctgagcctgaggcccgaagcctgtagacctgccgctggcggagccgtgcacaccagaggcctggatttcgcctgcgac

SEQ ID NO: 33 - DNA, 84 bp, synthetic construct
  misc_feature 1..84: note = source = /note="Description of Artificial Sequence: Synthetic oligonucleotide"
  misc_feature 1..84: note = source = /note="CD8-alpha TM domain"
  source 1..84: mol_type = other DNA
atctacatctgggcccctctggccggcacctgtggcgtgctgctgctgagcctggtcatcaccctgtactgcaaccaccggaat

SEQ ID NO: 34 - DNA, 81 bp, synthetic construct
  misc_feature 1..81: note = source = /note="Description of Artificial Sequence: Synthetic oligonucleotide"
  misc_feature 1..81: note = source = /note="CD28 TM domain"
  source 1..81: mol_type = other DNA
ttttgggtgctggtggtggttggtggagtcctggcttgctatagcttgctagtaacagtggcctttattattttctgggtg

SEQ ID NO: 35 - DNA, 123 bp, synthetic construct
  misc_feature 1..123: note = source = /note="Description of Artificial Sequence: Synthetic polynucleotide"
  misc_feature 1..123: note = source = /note="CD28 signaling domain"
  source 1..123: mol_type = other DNA
aggagcaagcggagcagaggcggccacagcgactacatgaacatgaccccccggaggcctggccccacccggaagcactaccagccctacgcccctcccagggacttcgccgcctaccggagc

SEQ ID NO: 36 - DNA, 336 bp, synthetic construct
  misc_feature 1..336: note = source = /note="Description of Artificial Sequence: Synthetic polynucleotide"
  misc_feature 1..336: note = source = /note="CD3 zeta signaling domain"
  source 1..336: mol_type = other DNA
cgggtgaagttcagccggagcgccgacgcccctgcctaccagcagggccagaaccagctgtacaacgagctgaacctgggccggagggaggagtacgacgtgctggacaagcggagaggccgggaccctgagatgggcggcaagccccggagaaagaaccctcaggagggcctgtataacgaactgcagaaagacaagatggccgaggcctacagcgagatcggcatgaagggcgagcggcggaggggcaagggccacgacggcctgtaccagggcctgagcaccgccaccaaggatacctacgacgccctgcacatgcaggccctgccccccaga

SEQ ID NO: 37 - DNA, 126 bp, synthetic construct
  misc_feature 1..126: note = source = /note="Description of Artificial Sequence: Synthetic polynucleotide"
  misc_feature 1..126: note = source = /note="4-1BB signaling domain"
  source 1..126: mol_type = other DNA
aagagaggccggaagaaactgctgtacatcttcaagcagcccttcatgcggcccgtgcagaccacccaggaagaggacggctgcagctgccggttccccgaggaagaggaaggcggctgcgaactg

SEQ ID NO: 38 - DNA, 72 bp, synthetic construct
  misc_feature 1..72: note = source = /note="Description of Artificial Sequence: Synthetic oligonucleotide"
  misc_feature 1..72: note = source = /note="DNAX-activation protein 10 (DAP 10) Signaling Domain"
  source 1..72: mol_type = other DNA
ctgtgcgcacgcccacgccgcagccccgcccaagaagatggcaaagtctacatcaacatgccaggcaggggc

SEQ ID NO: 39 - DNA, 156 bp, synthetic construct
  misc_feature 1..156: note = source = /note="Description of Artificial Sequence: Synthetic polynucleotide"
  misc_feature 1..156: note = source = /note="DNAX-activation protein 12 (DAP12) Signaling Domain"
  source 1..156: mol_type = other DNA
tacttcctgggccggctggtccctcgggggcgaggggctgcggaggcagcgacccggaaacagcgtatcactgagaccgagtcgccttatcaggagctccagggtcagaggtcggatgtctacagcgacctcaacacacagaggccgtattacaaa

SEQ ID NO: 40 - DNA, 114 bp, synthetic construct
  misc_feature 1..114: note = source = /note="Description of Artificial Sequence: Synthetic polynucleotide"
  misc_feature 1..114: note = source = /note="IL-2 core promoter"
  source 1..114: mol_type = other DNA
acattttgacacccccataatatttttccagaattaacagtataaattgcatctcttgttcaagagttccctatcactctctttaatcactactcacagtaacctcaactcctg

SEQ ID NO: 41 - DNA, 55 bp, synthetic construct
  misc_feature 1..55: note = source = /note="Description of Artificial Sequence: Synthetic oligonucleotide"
  misc_feature 1..55: note = source = /note="IL-2 minimal promoter"
  source 1..55: mol_type = other DNA
tcaagagttccctatcactctctttaatcactactcacagtaacctcaactcctg

SEQ ID NO: 42 - DNA, 380 bp, synthetic construct
  misc_feature 1..380: note = source = /note="Description of Artificial Sequence: Synthetic polynucleotide"
  misc_feature 1..380: note = source = /note="IL-2 enhancer and promoter variant"
  source 1..380: mol_type = other DNA
tgatatcttttctgagttacttttgtatccccacccccttaaagaaaggaggaaaaactgtttcatacagaaggcgttaattgcatgaattagagctatcacctaagtgtgggctaatgtaacaaagagggatttcacctacatccattcagtcagtctttgggggtttaaagaaattccaaagagtcatcagaagaggaaaaatgaaggtaatgttttttcagactggtaaagtctttgaaaatatgtgtaatatgtaaaacattttgacacccccataatatttttccagaattaacagtataaattgcatctcttgttcaagagttccctatcactctctttaatcactactcacagtaacctcaactcctgccaca

SEQ ID NO: 43 - DNA, 373 bp, synthetic construct
  misc_feature 1..373: note = source = /note="Description of Artificial Sequence: Synthetic polynucleotide"
  misc_feature 1..373: note = source = /note="IL-2 enhancer and promoter variant"
  source 1..373: mol_type = other DNA
ttttctgagttacttttgtatccccacccccttaaagaaaggaggaaaaactgtttcatacagaaggcgttaattgcatgaattagagctatcacctaagtgtgggctaatgtaacaaagagggatttcacctacatccattcagtcagtctttgggggtttaaagaaattccaaagagtcatcagaagaggaaaaatgaaggtaatgttttttcagactggtaaagtctttgaaaatatgtgtaatatgtaaaacattttgacacccccataatatttttccagaattaacagtataaattgcatctcttgttcaagagttccctatcactctctttaatcactactcacagtaacctcaactcctgccaca

SEQ ID NO: 44 - DNA, 20 bp, synthetic construct
  misc_feature 1..20: note = source = /note="Description of Artificial Sequence: Synthetic oligonucleotide"
  misc_feature 1..20: note = source = /note="NF-kappa-B binding site"
  source 1..20: mol_type = other DNA
aagagggatttcacctacat

SEQ ID NO: 45 - DNA, 11 bp, synthetic construct
  misc_feature 1..11: note = source = /note="Description of Artificial Sequence: Synthetic oligonucleotide"
  misc_feature 1..11: note = source = /note="NF-kappa-B binding site"
  source 1..11: mol_type = other DNA
aagagggattt

SEQ ID NO: 46 - DNA, 20 bp, synthetic construct
  misc_feature 1..20: note = source = /note="Description of Artificial Sequence: Synthetic oligonucleotide"
  misc_feature 1..20: note = source = /note="NF-kappa-B binding site"
  source 1..20: mol_type = other DNA
agagggatttcacctacatc

SEQ ID NO: 47 - DNA, 161 bp, synthetic construct
  misc_feature 1..161: note = source = /note="Description of Artificial Sequence: Synthetic polynucleotide"
  misc_feature 1..161: note = source = /note="(NF-kappa-B)1-IL2 promoter variant"
  source 1..161: mol_type = other DNA
aattggtcccatcgaagagggatttcacctacataattggtcccgggacattttgacacccccataatatttttccagaattaacagtataaattgcatctcttgttcaagagttccctatcactctctttaatcactactcacagtaacctcaactcctg

SEQ ID NO: 48 - DNA, 201 bp, synthetic construct
  misc_feature 1..201: note = source = /note="Description of Artificial Sequence: Synthetic polynucleotide"
  misc_feature 1..201: note = source = /note="(NF-kappa-B)3-IL2 promoter variant"
  source 1..201: mol_type = other DNA
aattggtcccatcgaagagggatttcacctacataagagggatttcacctacataagagggatttcacctacataattggtcccgggacattttgacacccccataatatttttccagaattaacagtataaattgcatctcttgttcaagagttccctatcactctctttaatcactactcacagtaacctcaactcctg

SEQ ID NO: 49 - DNA, 268 bp, synthetic construct
  misc_feature 1..268: note = source = /note="Description of Artificial Sequence: Synthetic polynucleotide"
  misc_feature 1..268: note = source = /note="(NF-kappa-B)6-IL2 promoter variant"
  source 1..268: mol_type = other DNA
aattggtcccatcgaagagggatttcacctacataagagggatttcacctacataagagggatttcacctacataattggtaagagggatttcacctacataagagggatttcacctacataagagggatttcacctacataattggtcccgggacattttgacacccccataatatttttccagaattaacagtataaattgcatctcttgttcaagagttccctatcactctctttaatcactactcacagtaacctcaactcctg

SEQ ID NO: 50 - DNA, 177 bp, synthetic construct
  misc_feature 1..177: note = source = /note="Description of Artificial Sequence: Synthetic polynucleotide"
  misc_feature 1..177: note = source = /note="1X NFAT Response Elements-IL2 Promoter variant"
  source 1..177: mol_type = other DNA
aattggtcccatcgaattaggaggaaaaactgtttcatacagaaggcgtcaattggtcccgggacattttgacacccccataatatttttccagaattaacagtataaattgcatctcttgttcaagagttccctatcactctctttaatcactactcacagtaacctcaactcctg

SEQ ID NO: 51 - DNA, 36 bp, synthetic construct
  misc_feature 1..36: note = source = /note="Description of Artificial Sequence: Synthetic oligonucleotide"
  misc_feature 1..36: note = source = /note="Nuclear factor of activated T-cells (NFAT) response element"
  source 1..36: mol_type = other DNA
aattaggaggaaaaactgtttcatacagaaggcgtc

SEQ ID NO: 52 - DNA, 358 bp, synthetic construct
  misc_feature 1..358: note = source = /note="Description of Artificial Sequence: Synthetic polynucleotide"
  misc_feature 1..358: note = source = /note="6X NFAT Response Elements-IL2 Promoter variant"
  source 1..358: mol_type = other DNA
gaattaggaggaaaaactgtttcatacagaaggcgtcaattaggaggaaaaactgtttcatacagaaggcgtcaattaggaggaaaaactgtttcatacagaaggcgtcaattggtcccatcgaattaggaggaaaaactgtttcatacagaaggcgtcaattaggaggaaaaactgtttcatacagaaggcgtcaattaggaggaaaaactgtttcatacagaaggcgtcaattggtcccgggacattttgacacccccataatatttttccagaattaacagtataaattgcatctcttgttcaagagttccctatcactctccttaatcactactcacagtaacctcaactcctg

SEQ ID NO: 53 - DNA, 374 bp, synthetic construct
  misc_feature 1..374: note = source = /note="Description of Artificial Sequence: Synthetic polynucleotide"
  misc_feature 1..374: note = source = /note="6X NFAT Response Elements-IL2 Promoter variant"
  source 1..374: mol_type = other DNA
tgatatcgaattaggaggaaaaactgtttcatacagaaggcgtcaattaggaggaaaaactgtttcatacagaaggcgtcaattaggaggaaaaactgtttcatacagaaggcgtcaattggtcccatcgaattaggaggaaaaactgtttcatacagaaggcgtcaattaggaggaaaaactgtttcatacagaaggcgtcaattaggaggaaaaactgtttcatacagaaggcgtcaattggtcccgggacattttgacacccccataatatttttccagaattaacagtataaattgcatctcttgttcaagagttccctatcactctctttaatcactactcacagtaacctcaactcctgaattccatg

SEQ ID NO: 54 - DNA, 358 bp, synthetic construct
  misc_feature 1..358: note = source = /note="Description of Artificial Sequence: Synthetic polynucleotide"
  misc_feature 1..358: note = source = /note="6X NFAT Response Elements-IL2 Promoter variant"
  source 1..358: mol_type = other DNA
gaattaggaggaaaaactgtttcatacagaaggcgtcaattaggaggaaaaactgtttcatacagaaggcgtcaattaggaggaaaaactgtttcatacagaaggcgtcaattggtcccatcgaattaggaggaaaaactgtttcatacagaaggcgtcaattaggaggaaaaactgtttcatacagaaggcgtcaattaggaggaaaaactgtttcatacagaaggcgtcaattggtcccgggacattttgacacccccataatatttttccagaattaacagtataaattgcatctcttgttcaagagttccctatcactctctttaatcactactcacagtaacctcaactcctg

SEQ ID NO: 55 - DNA, 365 bp, synthetic construct
  misc_feature 1..365: note = source = /note="Description of Artificial Sequence: Synthetic polynucleotide"
  misc_feature 1..365: note = source = /note="6X NFAT Response Elements-IL2 Promoter variant"
  source 1..365: mol_type = other DNA
tgatatcgaattaggaggaaaaactgtttcatacagaaggcgtcaattaggaggaaaaactgtttcatacagaaggcgtcaattaggaggaaaaactgtttcatacagaaggcgtcaattggtcccatcgaattaggaggaaaaactgtttcatacagaaggcgtcaattaggaggaaaaactgtttcatacagaaggcgtcaattaggaggaaaaactgtttcatacagaaggcgtcaattggtcccgggacattttgacacccccataatatttttccagaattaacagtataaattgcatctcttgttcaagagttccctatcactctctttaatcactactcacagtaacctcaactcctg

SEQ ID NO: 56 - DNA, 256 bp, synthetic construct
  misc_feature 1..256: note = source = /note="Description of Artificial Sequence: Synthetic polynucleotide"
  misc_feature 1..256: note = source = /note="3X NFAT Response Elements-IL2 Promoter variant"
  source 1..256: mol_type = other DNA
tgatatcaattggtcccatcgaattaggaggaaaaactgtttcatacagaaggcgtcaattaggaggaaaaactgtttcatacagaaggcgtcaattaggaggaaaaactgtttcatacagaaggcgtcaattggtcccgggacattttgacacccccataatatttttccagaattaacagtataaattgcatctcttgttcaagagttccctatcactctctttaatcactactcacagtaacctcaactcctg

SEQ ID NO: 57 - DNA, 249 bp, synthetic construct
  misc_feature 1..249: note = source = /note="Description of Artificial Sequence: Synthetic polynucleotide"
  misc_feature 1..249: note = source = /note="3X NFAT Response Elements-IL2 Promoter variant"
  source 1..249: mol_type = other DNA
aattggtcccatcgaattaggaggaaaaactgtttcatacagaaggcgtcaattaggaggaaaaactgtttcatacagaaggcgtcaattaggaggaaaaactgtttcatacagaaggcgtcaattggtcccgggacattttgacacccccataatatttttccagaattaacagtataaattgcatctcttgttcaagagttccctatcactctctttaatcactactcacagtaacctcaactcctg

SEQ ID NO: 58 - DNA, 244 bp, Homo sapiens
  misc_feature 1..244: note = source = /note="human EEF1A1 promoter variant"
  source 1..244: mol_type = genomic DNA
gagcgtgcgtgaggctccggtgcccgtcagtgggcagagcgcacatcgcccacagtccccgagaagttggggggagggggtcggcgattgaaccggtgcctagagaaggtggcgcggggtaaactgggaaagtgatgtcgtgtactggctccgcctttttcccgagggtgggggagaaccgtatataagtgcagtagtcgccgtgaacgttctttttcgcaacgggtttgccgccagaacacag

SEQ ID NO: 59 - DNA, 236 bp, Homo sapiens
  misc_feature 1..236: note = source = /note="human EEF1A1 promoter variant"
  source 1..236: mol_type = genomic DNA
gcgtgaggctccggtgcccgtcagtgggcagagcgcacatcgcccacagtccccgagaagttggggggaggggtcggcaattgaaccggtgcctagagaaggtggcgcggggtaaactgggaaagtgatgtcgtgtactggctccgcctttttcccgagggtgggggagaaccgtatataagtgcagtagtcgccgtgaacgttctttttcgcaacgggtttgccgccagaacaca

SEQ ID NO: 60 - DNA, 1266 bp, Homo sapiens
  misc_feature 1..1266: note = source = /note="human EEF1A1 promoter and enhancer"
  source 1..1266: mol_type = genomic DNA
gagctttgcaaagatggataaagttttaaacagagaggaatctttgcagctaatggaccttctaggtcttgaaaggagtgggaattggctccggtgcccgtcagtgggcagagcgcacatcgcccacagtccccgagaagttggggggaggggtcggcaattgaaccggtgcctagagaaggtggcgcggggtaaactgggaaagtgatgtcgtgtactggctccgcctttttcccgagggtgggggagaaccgtatataagtgcagtagtcgccgtgaacgttctttttcgcaacgggtttgccgccagaacacaggtaagtgccgtgtgtggttcccgcgggcctggcctctttacgggttatggcccttgcgtgccttgaattacttccacctggctgcagtacgtgattcttgatcccgagcttcgggttggaagtgggtgggagagttcgaggccttgcgcttaaggagccccttcgcctcgtgcttgagttgaggcctggcctgggcgctggggccgccgcgtgcgaatctggtggcaccttcgcgcctgtctcgctgctttcgataagtctctagccatttaaaatttttgatgacctgctgcgacgctttttttctggcaagatagtcttgtaaatgcgggccaagatctgcacactggtatttcggtttttggggccgcgggcggcgacggggcccgtgcgtcccagcgcacatgttcggcgaggcggggcctgcgagcgcggccaccgagaatcggacgggggtagtctcaagctggccggcctgctctggtgcctggcctcgcgccgccgtgtatcgccccgccctgggcggcaaggctggcccggtcggcaccagttgcgtgagcggaaagatggccgcttcccggccctgctgcagggagctcaaaatggaggacgcggcgctcgggagagcgggcgggtgagtcacccacacaaaggaaaagggcctttccgtcctcagccgtcgcttcatgtgactccacggagtaccgggcgccgtccaggcacctcgattagttctcgagcttttggagtacgtcgtctttaggttggggggaggggttttatgcgatggagtttccccacactgagtgggtggagactgaagttaggccagcttggcacttgatgtaattctccttggaatttgccctttttgagtttggatcttggttcattctcaagcctcagacagtggttcaaagtttttttcttccatttcaggtgtcgtgag

SEQ ID NO: 61 - DNA, 571 bp, Homo sapiens
  misc_feature 1..571: note = source = /note="Human UBC promoter"
  source 1..571: mol_type = genomic DNA
ggcctccgcgccgggttttggcgcctcccgcgggcgcccccctcctcacggcgagcgctgccacgtcagacgaagggcgcagcgagcgtcctgatccttccgcccggacgctcaggacagcggcccgctgctcataagactcggccttagaaccccagtatcagcagaaggacattttaggacgggacttgggtgactctagggcactggttttctttccagagagcggaacaggcgaggaaaagtagtcccttctcggcgattctgcggagggatctccgtggggcggtgaacgccgatgattatataaggacgcgccgggtgtggcacagctagttccgtcgcagccgggatttgggtcgcggttcttgtttgtggatcgctgtgatcgtcacttggtgagtagcgggctgctgggctgggtacgtgcgctcggggttggcgagtgtgttttgtgaagttttttaggcaccttttgaaatgtaatcatttgggtcaatatgtaattttcagtgttagactagtaaattgtccgctaaattctggccgtttttggcttttttgttagacg

SEQ ID NO: 62 - DNA, 148 bp, synthetic construct
  misc_feature 1..148: note = source = /note="Description of Artificial Sequence: Synthetic polynucleotide"
  misc_feature 1..148: note = source = /note="6 site GAL4-inducible proximal factor binding element (PFB)"
  source 1..148: mol_type = other DNA
attgttcggagcagtgcggcgcgtttagcggagtactgtcctccgatattaatcggggcagactattccggggtttaccggcgcactctcgcccgaacttcaccggcggtctttcgtccgtgctttatcggggcggatcactccgaac

SEQ ID NO: 63 - DNA, 81 bp, synthetic construct
  misc_feature 1..81: note = source = /note="Description of Artificial Sequence: Synthetic oligonucleotide"
  misc_feature 1..81: note = source = /note="Synthetic minimal promoter 1 [Inducible Promoter]"
  source 1..81: mol_type = other DNA
aggtctatataagcagagctcgtttagtgaaccctcattctggagacggatcccgagccgagtgttttgacctccatagaa

SEQ ID NO: 64 - DNA, 31 bp, synthetic construct
  misc_feature 1..31: note = source = /note="Description of Artificial Sequence: Synthetic oligonucleotide"
  misc_feature 1..31: note = source = /note="Synthetic 5' UTR based on RPL6"
  source 1..31: mol_type = other DNA
cagccgctaaatccaaggtaaggtcagaaga

SEQ ID NO: 65 - DNA, 132 bp, Simian virus 40
  misc_feature 1..132: note = source = /note="SV40e polyA"
  source 1..132: mol_type = unassigned DNA
aacttgtttattgcagcttataatggttacaaataaagcaatagcatcacaaatttcacaaataaagcatttttttcactgcattctagttgtggtttgtccaaactcatcaatgtatcttatcatgtctgg

SEQ ID NO: 66 - DNA, 275 bp, synthetic construct
  misc_feature 1..275: note = source = /note="Description of Artificial Sequence: Synthetic polynucleotide"
  misc_feature 1..275: note = source = /note="Bidirectional aCA polyA [bidirectional polyA]"
  source 1..275: mol_type = other DNA
atcgattaatctagcggccctagacgagcagacatgataagatacattgatgagtttggacaaaccacaactagaatgcagtgaaaaaaatgctttatttgtgaaatttgtgatgctattgctttatttgtaaccattataagctgcaataaacaagttaacaacaacaattgcattcattttatgtttcaggttcagggggagatgtgggaggttttttaaagcaagtaaaacctctacaaatgtggtaaaatccgataagcgtacctagaggc

SEQ ID NO: 67 - DNA, 57 bp, synthetic construct
  misc_feature 1..57: note = source = /note="Description of Artificial Sequence: Synthetic oligonucleotide"
  misc_feature 1..57: note = source = /note="PA2 polyA"
  source 1..57: mol_type = other DNA
ggccgcaataaaatatctttattttcattacatctgtgtgttggttttttgtgtgag

SEQ ID NO: 68 - DNA, 258 bp, synthetic construct
  misc_feature 1..258: note = source = /note="Description of Artificial Sequence: Synthetic polynucleotide"
  misc_feature 1..258: note = source = /note="VP16 activation domain"
  source 1..258: mol_type = other DNA
ggccccaagaagaaaaggaaggtggccccccccaccgacgtgagcctgggcgacgagctgcacctggacggcgaggacgtggccatggcccacgccgacgccctggacgacttcgacctggacatgctgggcgacggcgacagccccggccccggcttcaccccccacgacagcgccccctacggcgccctggacatggccgacttcgagttcgagcagatgttcaccgacgccctgggcatcgacgagtacggcggc

SEQ ID NO: 69 - DNA, 705 bp, synthetic construct
  misc_feature 1..705: note = source = /note="Description of Artificial Sequence: Synthetic polynucleotide"
  misc_feature 1..705: note = source = /note="Retinoid x receptor (RxR)"
  source 1..705: mol_type = other DNA
gagatgcccgtggacaggattctggaggccgaactcgccgtggagcagaaaagcgaccagggcgtggagggccccggcggaaccggcggcagcggcagcagccccaacgaccccgtgaccaacatctgccaggccgccgacaagcagctgttcaccctggtggagtgggccaagaggattccccacttcagcagcctgcccctggacgaccaggtgatcctgctgagggccggatggaacgagctgctgatcgccagcttcagccacaggagcatcgacgtgagggacggcatcctgctggccaccggcctgcacgtccataggaacagcgcccacagcgccggagtgggcgccatcttcgacagggtgctgaccgagctggtgagcaagatgagggacatgaggatggacaagaccgagctgggctgcctgagggccatcatcctgttcaaccccgaggtgaggggcctgaaaagcgcccaggaggtggagctgctgagggagaaggtgtacgccgccctggaggagtacaccaggaccacccaccccgacgagcccggcagattcgccaagctgctgctgaggctgcccagcctgaggagcatcggcctgaagtgcctggagcacctgttcttcttcaggctgatcggcgacgtgcccatcgacaccttcctgatggagatgctggagagccccagcgacagc

SEQ ID NO: 70 - DNA, 969 bp, synthetic construct
  misc_feature 1..969: note = source = /note="Description of Artificial Sequence: Synthetic polynucleotide"
  misc_feature 1..969: note = source = /note="VP16-linker-RxR"
  source 1..969: mol_type = other DNA
ggccccaagaagaaaaggaaggtggccccccccaccgacgtgagcctgggcgacgagctgcacctggacggcgaggacgtggccatggcccacgccgacgccctggacgacttcgacctggacatgctgggcgacggcgacagccccggccccggcttcaccccccacgacagcgccccctacggcgccctggacatggccgacttcgagttcgagcagatgttcaccgacgccctgggcatcgacgagtacggcggcgaattcgagatgcccgtggacaggattctggaggccgaactcgccgtggagcagaaaagcgaccagggcgtggagggccccggcggaaccggcggcagcggcagcagccccaacgaccccgtgaccaacatctgccaggccgccgacaagcagctgttcaccctggtggagtgggccaagaggattccccacttcagcagcctgcccctggacgaccaggtgatcctgctgagggccggatggaacgagctgctgatcgccagcttcagccacaggagcatcgacgtgagggacggcatcctgctggccaccggcctgcacgtccataggaacagcgcccacagcgccggagtgggcgccatcttcgacagggtgctgaccgagctggtgagcaagatgagggacatgaggatggacaagaccgagctgggctgcctgagggccatcatcctgttcaaccccgaggtgaggggcctgaaaagcgcccaggaggtggagctgctgagggagaaggtgtacgccgccctggaggagtacaccaggaccacccaccccgacgagcccggcagattcgccaagctgctgctgaggctgcccagcctgaggagcatcggcctgaagtgcctggagcacctgttcttcttcaggctgatcggcgacgtgcccatcgacaccttcctgatggagatgctggagagccccagcgacagc

SEQ ID NO: 71 - DNA, 450 bp, synthetic construct
  misc_feature 1..450: note = source = /note="Description of Artificial Sequence: Synthetic polynucleotide"
  misc_feature 1..450: note = source = /note="GAL4 DNA Binding Domain"
  source 1..450: mol_type = other DNA
atgaagctgctgagcagcatcgagcaggcttgcgacatctgcaggctgaagaagctgaagtgcagcaaggagaagcccaagtgcgccaagtgcctgaagaacaactgggagtgcagatacagccccaagaccaagaggagccccctgaccagggcccacctgaccgaggtggagagcaggctggagaggctggagcagctgttcctgctgatcttccccagggaggacctggacatgatcctgaagatggacagcctgcaagacatcaaggccctgctgaccggcctgttcgtgcaggacaacgtgaacaaggacgccgtgaccgacaggctggccagcgtggagaccgacatgcccctgaccctgaggcagcacaggatcagcgccaccagcagcagcgaggagagcagcaacaagggccagaggcagctgaccgtgagccccgagttt

SEQ ID NO: 72 - DNA, 1008 bp, synthetic construct
  misc_feature 1..1008: note = source = /note="Description of Artificial Sequence: Synthetic polynucleotide"
  misc_feature 1..1008: note = source = /note="Ecdysone Receptor Ligand Binding Domain - VY variant (EcR)"
  source 1..1008: mol_type = other DNA
atcaggcccgagtgcgtggtgcccgagacccagtgcgccatgaaaaggaaggagaagaaggcccagaaggagaaggacaagctgcccgtgagcaccaccaccgtcgatgaccacatgccccccatcatgcagtgcgagccccccccccccgaggccgccaggattcacgaggtcgtgcccaggttcctgagcgacaagctgctggtgaccaacaggcagaagaacatcccccagctgaccgccaaccagcagttcctgatcgccaggctgatctggtatcaggacggctacgagcagcccagcgacgaggacctgaaaaggatcacccagacctggcagcaggccgacgacgagaacgaggagagcgacacccccttcaggcagatcaccgagatgaccatcctgaccgtgcagctgatcgtggagttcgccaagggcctgcccggattcgccaagatcagccagcccgaccagatcaccctgctgaaggcttgcagcagcgaggtgatgatgctgagggtggccaggaggtacgacgccgccagcgacagcatcctgttcgccaacaaccaggcttacaccagggacaactacaggaaggctggcatggccgaggtgatcgaggacctcctgcacttctgcagatgtatgtacagcatggccctggacaacatccactacgccctgctgaccgccgtggtgatcttcagcgacaggcccggcctggagcagccccagctggtggaggagatccagaggtactacctgaacaccctgaggatctacatcctgaaccagctgagcggcagcgccaggagcagcgtgatctacggcaagatcctgagcatcctgagcgagctgaggaccctgggaatgcagaacagcaatatgtgtatcagcctgaagctgaagaacaggaagctgccccccttcctggaggagatttgggacgtggccgacatgagccacacccagcccccccccatcctggagagccccaccaacctg

SEQ ID NO: 73 - DNA, 1008 bp, synthetic construct
  misc_feature 1..1008: note = source = /note="Description of Artificial Sequence: Synthetic polynucleotide"
  misc_feature 1..1008: note = source = /note="Ecdysone Receptor Ligand Binding Domain - VY variant (EcR)"
  source 1..1008: mol_type = other DNA
cggcctgagtgcgtagtacccgagactcagtgcgccatgaagcggaaagagaagaaagcacagaaggagaaggacaaactgcctgtcagcacgacgacggtggacgaccacatgccgcccattatgcagtgtgaacctccacctcctgaagcagcaaggattcacgaagtggtcccaaggtttctctccgacaagctgttggtgacaaaccggcagaaaaacatcccccagttgacagccaaccagcagttccttatcgccaggctcatctggtaccaggacgggtacgagcagccttctgatgaagatttgaagaggattacgcagacgtggcagcaagcggacgatgaaaacgaagagtcggacactcccttccgccagatcacagagatgactatcctcacggtccaacttatcgtggagttcgcgaagggattgccagggttcgccaagatctcgcagcctgatcaaattacgctgcttaaggcttgctcaagtgaggtaatgatgctccgagtcgcgcgacgatacgatgcggcctcagacagtattctgttcgcgaacaaccaagcgtacactcgcgacaactaccgcaaggctggcatggccgaggtcatcgaggatctactgcacttctgccggtgcatgtactctatggcgttggacaacatccattacgcgctgctcacggctgtcgtcatcttttctgaccggccagggttggagcagccgcaactggtggaagagatccagcggtactacctgaatacgctccgcatctatatcctgaaccagctgagcgggtcggcgcgttcgtccgtcatatacggcaagatcctctcaatcctctctgagctacgcacgctcggcatgcaaaactccaacatgtgcatctccctcaagctcaagaacagaaagctgccgcctttcctcgaggagatctgggatgtggcggacatgtcgcacacccaaccgccgcctatcctcgagtcccccacgaatctctag

SEQ ID NO: 74 - DNA, 1467 bp, synthetic construct
  misc_feature 1..1467: note = source = /note="Description of Artificial Sequence: Synthetic polynucleotide"
  misc_feature 1..1467: note = source = /note="GAL4-Linker-EcR"
  source 1..1467: mol_type = other DNA
atgaagctactgtcttctatcgaacaagcatgcgatatttgccgacttaaaaagctcaagtgctccaaagaaaaaccgaagtgcgccaagtgtctgaagaacaactgggagtgtcgctactctcccaaaaccaaaaggtctccgctgactagggcacatctgacagaagtggaatcaaggctagaaagactggaacagctatttctactgatttttcctcgagaagaccttgacatgattttgaaaatggattctttacaggatataaaagcattgttaacaggattatttgtacaagataatgtgaataaagatgccgtcacagatagattggcttcagtggagactgatatgcctctaacattgagacagcatagaataagtgcgacatcatcatcggaagagagtagtaacaaaggtcaaagacagttgactgtatcgccggaattcccggggatccggcctgagtgcgtagtacccgagactcagtgcgccatgaagcggaaagagaagaaagcacagaaggagaaggacaaactgcctgtcagcacgacgacggtggacgaccacatgccgcccattatgcagtgtgaacctccacctcctgaagcagcaaggattcacgaagtggtcccaaggtttctctccgacaagctgttggtgacaaaccggcagaaaaacatcccccagttgacagccaaccagcagttccttatcgccaggctcatctggtaccaggacgggtacgagcagccttctgatgaagatttgaagaggattacgcagacgtggcagcaagcggacgatgaaaacgaagagtcggacactcccttccgccagatcacagagatgactatcctcacggtccaacttatcgtggagttcgcgaagggattgccagggttcgccaagatctcgcagcctgatcaaattacgctgcttaaggcttgctcaagtgaggtaatgatgctccgagtcgcgcgacgatacgatgcggcctcagacagtattctgttcgcgaacaaccaagcgtacactcgcgacaactaccgcaaggctggcatggccgaggtcatcgaggatctactgcacttctgccggtgcatgtactctatggcgttggacaacatccattacgcgctgctcacggctgtcgtcatcttttctgaccggccagggttggagcagccgcaactggtggaagagatccagcggtactacctgaatacgctccgcatctatatcctgaaccagctgagcgggtcggcgcgttcgtccgtcatatacggcaagatcctctcaatcctctctgagctacgcacgctcggcatgcaaaactccaacatgtgcatctccctcaagctcaagaacagaaagctgccgcctttcctcgaggagatctgggatgtggcggacatgtcgcacacccaaccgccgcctatcctcgagtcccccacgaatctctag

SEQ ID NO: 75 - DNA, 1464 bp, synthetic construct
  misc_feature 1..1464: note = source = /note="Description of Artificial Sequence: Synthetic polynucleotide"
  misc_feature 1..1464: note = source = /note="GAL4-Linker-EcR"
  source 1..1464: mol_type = other DNA
atgaagctgctgagcagcatcgagcaggcttgcgacatctgcaggctgaagaagctgaagtgcagcaaggagaagcccaagtgcgccaagtgcctgaagaacaactgggagtgcagatacagccccaagaccaagaggagccccctgaccagggcccacctgaccgaggtggagagcaggctggagaggctggagcagctgttcctgctgatcttccccagggaggacctggacatgatcctgaagatggacagcctgcaagacatcaaggccctgctgaccggcctgttcgtgcaggacaacgtgaacaaggacgccgtgaccgacaggctggccagcgtggagaccgacatgcccctgaccctgaggcagcacaggatcagcgccaccagcagcagcgaggagagcagcaacaagggccagaggcagctgaccgtgagccccgagtttcccgggcggcctgagtgcgtagtacccgagactcagtgcgccatgaagcggaaagagaagaaagcacagaaggagaaggacaaactgcctgtcagcacgacgacggtggacgaccacatgccgcccattatgcagtgtgaacctccacctcctgaagcagcaaggattcacgaagtggtcccaaggtttctctccgacaagctgttggtgacaaaccggcagaaaaacatcccccagttgacagccaaccagcagttccttatcgccaggctcatctggtaccaggacgggtacgagcagccttctgatgaagatttgaagaggattacgcagacgtggcagcaagcggacgatgaaaacgaagagtcggacactcccttccgccagatcacagagatgactatcctcacggtccaacttatcgtggagttcgcgaagggattgccagggttcgccaagatctcgcagcctgatcaaattacgctgcttaaggcttgctcaagtgaggtaatgatgctccgagtcgcgcgacgatacgatgcggcctcagacagtattctgttcgcgaacaaccaagcgtacactcgcgacaactaccgcaaggctggcatggccgaggtcatcgaggatctactgcacttctgccggtgcatgtactctatggcgttggacaacatccattacgcgctgctcacggctgtcgtcatcttttctgaccggccagggttggagcagccgcaactggtggaagagatccagcggtactacctgaatacgctccgcatctatatcctgaaccagctgagcgggtcggcgcgttcgtccgtcatatacggcaagatcctctcaatcctctctgagctacgcacgctcggcatgcaaaactccaacatgtgcatctccctcaagctcaagaacagaaagctgccgcctttcctcgaggagatctgggatgtggcggacatgtcgcacacccaaccgccgcctatcctcgagtcccccacgaatctctag

SEQ ID NO: 76 - DNA, 1005 bp, synthetic construct
  misc_feature 1..1005: note = source = /note="Description of Artificial Sequence: Synthetic polynucleotide"
  misc_feature 1..1005: note = source = /note="Truncated EGFR (huEGFRt) (Her1t)"
  source 1..1005: mol_type = other DNA
cgcaaagtgtgtaacggaataggtattggtgaatttaaagactcactctccataaatgctacgaatattaaacacttcaaaaactgcacctccatcagtggcgatctccacatcctgccggtggcatttaggggtgactccttcacacatactcctcctctggatccacaggaactggatattctgaaaaccgtaaaggaaatcacagggtttttgctgattcaggcttggcctgaaaacaggacggacctccatgcctttgagaacctagaaatcatacgcggcaggaccaagcaacatggtcagttttctcttgcagtcgtcagcctgaacataacatccttgggattacgctccctcaaggagataagtgatggagatgtgataatttcaggaaacaaaaatttgtgctatgcaaatacaataaactggaaaaaactgtttgggacctccggtcagaaaaccaaaattataagcaacagaggtgaaaacagctgcaaggccacaggccaggtctgccatgccttgtgctcccccgagggctgctggggcccggagcccagggactgcgtctcttgccggaatgtcagccgaggcagggaatgcgtggacaagtgcaaccttctggagggtgagccaagggagtttgtggagaactctgagtgcatacagtgccacccagagtgcctgcctcaggccatgaacatcacctgcacaggacggggaccagacaactgtatccagtgtgcccactacattgacggcccccactgcgtcaagacctgcccggcaggagtcatgggagaaaacaacaccctggtctggaagtacgcagacgccggccatgtgtgccacctgtgccatccaaactgcacctacggatgcactgggccaggtcttgaaggctgtccaacgaatgggcctaagatcccgtccatcgccactgggatggtgggggccctcctcttgctgctggtggtggccctggggatcggcctcttcatg

SEQ ID NO: 77 - DNA, 732 bp, synthetic construct
  misc_feature 1..732: note = source = /note="Description of Artificial Sequence: Synthetic polynucleotide"
  misc_feature 1..732: note = source = /note="EGFR truncated design 1 (Her1 truncated design 1) (HER1t1)"
  source 1..732: mol_type = other DNA
cgcaaagtgtgtaacggaataggtattggtgaatttaaagactcactctccataaatgctacgaatattaaacacttcaaaaactgcacctccatcagtggcgatctccacatcctgccggtggcatttaggggtgactccttcacacatactcctcctctggatccacaggaactggatattctgaaaaccgtaaaggaaatcacagggtttttgctgattcaggcttggcctgaaaacaggacggacctccatgcctttgagaacctagaaatcatacgcggcaggaccaagcaacatggtcagttttctcttgcagtcgtcagcctgaacataacatccttgggattacgctccctcaaggagataagtgatggagatgtgataatttcaggaaacaaaaatttgtgctatgcaaatacaataaactggaaaaaactgtttgggacctccggtcagaaaaccaaaattataagcaacagaggtgaaaacagctgcaaggccacaggccaggtctgccatgccttgtgctcccccgagggctgctggggcccggagcccagggactgcgtctctggtggcggtggctcgggcggtggtgggtcgggtggcggcggatctggtggcggtggctcgttttgggtgctggtggtggttggtggagtcctggcttgctatagcttgctagtaacagtggcctttattattttctgggtgaggagtaagaggagc

SEQ ID NO: 78 - DNA, 771 bp, synthetic construct
  misc_feature 1..771: note = source = /note="Description of Artificial Sequence: Synthetic polynucleotide"
  misc_feature 1..771: note = source = /note="EGFR truncated design 2 (Her1 truncated design 2) (HER1t2)"
  source 1..771: mol_type = other DNA
cgcaaagtgtgtaacggaataggtattggtgaatttaaagactcactctccataaatgctacgaatattaaacacttcaaaaactgcacctccatcagtggcgatctccacatcctgccggtggcatttaggggtgactccttcacacatactcctcctctggatccacaggaactggatattctgaaaaccgtaaaggaaatcacagggtttttgctgattcaggcttggcctgaaaacaggacggacctccatgcctttgagaacctagaaatcatacgcggcaggaccaagcaacatggtcagttttctcttgcagtcgtcagcctgaacataacatccttgggattacgctccctcaaggagataagtgatggagatgtgataatttcaggaaacaaaaatttgtgctatgcaaatacaataaactggaaaaaactgtttgggacctccggtcagaaaaccaaaattataagcaacagaggtgaaaacagctgcaaggccacaggccaggtctgccatgccttgtgctcccccgagggctgctggggcccggagcccagggactgcgtctcttgccggaatgtcagccgaggcagggaatgcgtggacaagggtggcggtggctcgggcggtggtgggtcgggtggcggcggatctggtggcggtggctcgttttgggtgctggtggtggttggtggagtcctggcttgctatagcttgctagtaacagtggcctttattattttctgggtgaggagtaagaggagc

SEQ ID NO: 79 - DNA, 828 bp, synthetic construct
  misc_feature 1..828: note = source = /note="Description of Artificial Sequence: Synthetic polynucleotide"
  misc_feature 1..828: note = source = /note="EGFR truncated design 3 (Her1 truncated design 3) (HER1t3)"
  source 1..828: mol_type = other DNA
cgcaaagtgtgtaacggaataggtattggtgaatttaaagactcactctccataaatgctacgaatattaaacacttcaaaaactgcacctccatcagtggcgatctccacatcctgccggtggcatttaggggtgactccttcacacatactcctcctctggatccacaggaactggatattctgaaaaccgtaaaggaaatcacagggtttttgctgattcaggcttggcctgaaaacaggacggacctccatgcctttgagaacctagaaatcatacgcggcaggaccaagcaacatggtcagttttctcttgcagtcgtcagcctgaacataacatccttgggattacgctccctcaaggagataagtgatggagatgtgataatttcaggaaacaaaaatttgtgctatgcaaatacaataaactggaaaaaactgtttgggacctccggtcagaaaaccaaaattataagcaacagaggtgaaaacagctgcaaggccacaggccaggtctgccatgccttgtgctcccccgagggctgctggggcccggagcccagggactgcgtctcttgccggaatgtcagccgaggcagggaatgcgtggacaagtgcaaccttctggagggtgagccaagggagtttgtggagaactctgagtgcatacagggtggcggtggctcgggcggtggtgggtcgggtggcggcggatctggtggcggtggctcgttttgggtgctggtggtggttggtggagtcctggcttgctatagcttgctagtaacagtggcctttattattttctgggtgaggagtaagaggagc

SEQ ID NO: 80 - DNA, 885 bp, synthetic construct
  misc_feature 1..885: note = source = /note="Description of Artificial Sequence: Synthetic polynucleotide"
  misc_feature 1..885: note = source = /note="EGFR truncated design 4 (Her1 truncated design 4) (HER1t4)"
  source 1..885: mol_type = other DNA
cgcaaagtgtgtaacggaataggtattggtgaatttaaagactcactctccataaatgctacgaatattaaacacttcaaaaactgcacctccatcagtggcgatctccacatcctgccggtggcatttaggggtgactccttcacacatactcctcctctggatccacaggaactggatattctgaaaaccgtaaaggaaatcacagggtttttgctgattcaggcttggcctgaaaacaggacggacctccatgcctttgagaacctagaaatcatacgcggcaggaccaagcaacatggtcagttttctcttgcagtcgtcagcctgaacataacatccttgggattacgctccctcaaggagataagtgatggagatgtgataatttcaggaaacaaaaatttgtgctatgcaaatacaataaactggaaaaaactgtttgggacctccggtcagaaaaccaaaattataagcaacagaggtgaaaacagctgcaaggccacaggccaggtctgccatgccttgtgctcccccgagggctgctggggcccggagcccagggactgcgtctcttgccggaatgtcagccgaggcagggaatgcgtggacaagtgcaaccttctggagggtgagccaagggagtttgtggagaactctgagtgcatacagtgccacccagagtgcctgcctcaggccatgaacatcacctgcacaggacggggaccagacaactgtatccagggcggaggcggaagcggaggcggaggctccggcggaggcggaagcttttgggtgctggtggtggttggtggagtcctggcttgctatagcttgctagtaacagtggcctttattattttctgggtgaggagtaagaggagc

SEQ ID NO: 81 - DNA, 924 bp, synthetic construct
  misc_feature 1..924: note = source = /note="Description of Artificial Sequence: Synthetic polynucleotide"
  misc_feature 1..924: note = source = /note="EGFR truncated design 5 (Her1 truncated design 5) (HER1t5)"
  source 1..924: mol_type = other DNA
cgcaaagtgtgtaacggaataggtattggtgaatttaaagactcactctccataaatgctacgaatattaaacacttcaaaaactgcacctccatcagtggcgatctccacatcctgccggtggcatttaggggtgactccttcacacatactcctcctctggatccacaggaactggatattctgaaaaccgtaaaggaaatcacagggtttttgctgattcaggcttggcctgaaaacaggacggacctccatgcctttgagaacctagaaatcatacgcggcaggaccaagcaacatggtcagttttctcttgcagtcgtcagcctgaacataacatccttgggattacgctccctcaaggagataagtgatggagatgtgataatttcaggaaacaaaaatttgtgctatgcaaatacaataaactggaaaaaactgtttgggacctccggtcagaaaaccaaaattataagcaacagaggtgaaaacagctgcaaggccacaggccaggtctgccatgccttgtgctcccccgagggctgctggggcccggagcccagggactgcgtctcttgccggaatgtcagccgaggcagggaatgcgtggacaagtgcaaccttctggagggtgagccaagggagtttgtggagaactctgagtgcatacagtgccacccagagtgcctgcctcaggccatgaacatcacctgcacaggacggggaccagacaactgtatccagtgtgcccactacattgacggcccccactgcgtcaagaccggcggaggcggaagcggaggcggaggctccggcggaggcggaagcttttgggtgctggtggtggttggtggagtcctggcttgctatagcttgctagtaacagtggcctttattattttctgggtgaggagtaagaggagc

SEQ ID NO: 82 - DNA, 984 bp, synthetic construct
  misc_feature 1..984: note = source = /note="Description of Artificial Sequence: Synthetic polynucleotide"
  misc_feature 1..984: note = source = /note="EGFR truncated design 6 (Her1 truncated design 6) (HER1t6)"
  source 1..984: mol_type = other DNA
cgcaaagtgtgtaacggaataggtattggtgaatttaaagactcactctccataaatgctacgaatattaaacacttcaaaaactgcacctccatcagtggcgatctccacatcctgccggtggcatttaggggtgactccttcacacatactcctcctctggatccacaggaactggatattctgaaaaccgtaaaggaaatcacagggtttttgctgattcaggcttggcctgaaaacaggacggacctccatgcctttgagaacctagaaatcatacgcggcaggaccaagcaacatggtcagttttctcttgcagtcgtcagcctgaacataacatccttgggattacgctccctcaaggagataagtgatggagatgtgataatttcaggaaacaaaaatttgtgctatgcaaatacaataaactggaaaaaactgtttgggacctccggtcagaaaaccaaaattataagcaacagaggtgaaaacagctgcaaggccacaggccaggtctgccatgccttgtgctcccccgagggctgctggggcccggagcccagggactgcgtctcttgccggaatgtcagccgaggcagggaatgcgtggacaagtgcaaccttctggagggtgagccaagggagtttgtggagaactctgagtgcatacagtgccacccagagtgcctgcctcaggccatgaacatcacctgcacaggacggggaccagacaactgtatccagtgtgcccactacattgacggcccccactgcgtcaagacctgcccggcaggagtcatgggagaaaacaacaccctggtctggaagtacgcagacgccggccatgtgtgccacctgggcggaggcggaagcggaggcggaggctccttttgggtgctggtggtggttggtggagtcctggcttgctatagcttgctagtaacagtggcctttattattttctgggtgaggagtaagaggagc

SEQ ID NO: 83 - DNA, 1032 bp, synthetic construct
  misc_feature 1..1032: note = source = /note="Description of Artificial Sequence: Synthetic polynucleotide"
  misc_feature 1..1032: note = source = /note="EGFR truncated design 7 (Her1 truncated design 7) (HER1t7)"
  source 1..1032: mol_type = other DNA
cgcaaagtgtgtaacggaataggtattggtgaatttaaagactcactctccataaatgctacgaatattaaacacttcaaaaactgcacctccatcagtggcgatctccacatcctgccggtggcatttaggggtgactccttcacacatactcctcctctggatccacaggaactggatattctgaaaaccgtaaaggaaatcacagggtttttgctgattcaggcttggcctgaaaacaggacggacctccatgcctttgagaacctagaaatcatacgcggcaggaccaagcaacatggtcagttttctcttgcagtcgtcagcctgaacataacatccttgggattacgctccctcaaggagataagtgatggagatgtgataatttcaggaaacaaaaatttgtgctatgcaaatacaataaactggaaaaaactgtttgggacctccggtcagaaaaccaaaattataagcaacagaggtgaaaacagctgcaaggccacaggccaggtctgccatgccttgtgctcccccgagggctgctggggcccggagcccagggactgcgtctcttgccggaatgtcagccgaggcagggaatgcgtggacaagtgcaaccttctggagggtgagccaagggagtttgtggagaactctgagtgcatacagtgccacccagagtgcctgcctcaggccatgaacatcacctgcacaggacggggaccagacaactgtatccagtgtgcccactacattgacggcccccactgcgtcaagacctgcccggcaggagtcatgggagaaaacaacaccctggtctggaagtacgcagacgccggccatgtgtgccacctgtgccatccaaactgcacctacggatgcactgggccaggtcttgaaggctgtccaggtggcggtggcggcggatctttttgggtgctggtggtggttggtggagtcctggcttgctatagcttgctagtaacagtggcctttattattttctgggtgaggagtaagaggagctaa

SEQ ID NO: 84 - DNA, 726 bp, synthetic construct
  misc_feature 1..726: note = source = /note="Description of Artificial Sequence: Synthetic polynucleotide"
  misc_feature 1..726: note = source = /note="EGFR truncated design 8 (Her1 truncated design 8) (HER1t8)"
  source 1..726: mol_type = other DNA
cgcaaagtgtgtaacggaataggtattggtgaatttaaagactcactctccataaatgctacgaatattaaacacttcaaaaactgcacctccatcagtggcgatctccacatcctgccggtggcatttaggggtgactccttcacacatactcctcctctggatccacaggaactggatattctgaaaaccgtaaaggaaatcacagggtttttgctgattcaggcttggcctgaaaacaggacggacctccatgcctttgagaacctagaaatcatacgcggcaggaccaagcaacatggtcagttttctcttgcagtcgtcagcctgaacataacatccttgggattacgctccctcaaggagataagtgatggagatgtgataatttcaggaaacaaaaatttgtgctatgcaaatacaataaactggaaaaaactgtttgggacctccggtcagaaaaccaaaattataagcaacagaggtgaaaacagctgcaaggccacaggccaggtctgccatgccttgtgctcccccgagggctgctggggcccggagcccagggactgcgtctctggtggcggtggctcgggcggtggtgggtcgggtggcggcggatctggtggcggtggctcggagataacactcattatttttggggtgatggctggtgttattggaacgatcctcttaatttcttacggtattcgccgaggaggtggaagc

SEQ ID NO: 85 - DNA, 717 bp, synthetic construct
  misc_feature 1..717: note = source = /note="Description of Artificial Sequence: Synthetic polynucleotide"
  misc_feature 1..717: note = source = /note="EGFR truncated design 9 (Her1 truncated design 9) (HER1t9)"
  source 1..717: mol_type = other DNA
cgcaaagtgtgtaacggaataggtattggtgaatttaaagactcactctccataaatgctacgaatattaaacacttcaaaaactgcacctccatcagtggcgatctccacatcctgccggtggcatttaggggtgactccttcacacatactcctcctctggatccacaggaactggatattctgaaaaccgtaaaggaaatcacagggtttttgctgattcaggcttggcctgaaaacaggacggacctccatgcctttgagaacctagaaatcatacgcggcaggaccaagcaacatggtcagttttctcttgcagtcgtcagcctgaacataacatccttgggattacgctccctcaaggagataagtgatggagatgtgataatttcaggaaacaaaaatttgtgctatgcaaatacaataaactggaaaaaactgtttgggacctccggtcagaaaaccaaaattataagcaacagaggtgaaaacagctgcaaggccacaggccaggtctgccatgccttgtgctcccccgagggctgctggggcccggagcccagggactgcgtctctggtggcggtggctcgggcggtggtgggtcgggtggcggcggatctggtggcggtggctcgataacactcattatttttggggtgatggctggtgttattggaacgatcctcttaatttcttacggtattggaggtggaagc

SEQ ID NO: 86 - DNA, 717 bp, synthetic construct
  misc_feature 1..717: note = source = /note="Description of Artificial Sequence: Synthetic polynucleotide"
  misc_feature 1..717: note = source = /note="EGFR truncated design 10 (Her1 truncated design 10) (HER1t10)"
  source 1..717: mol_type = other DNA
cgcaaagtgtgtaacggaataggtattggtgaatttaaagactcactctccataaatgctacgaatattaaacacttcaaaaactgcacctccatcagtggcgatctccacatcctgccggtggcatttaggggtgactccttcacacatactcctcctctggatccacaggaactggatattctgaaaaccgtaaaggaaatcacagggtttttgctgattcaggcttggcctgaaaacaggacggacctccatgcctttgagaacctagaaatcatacgcggcaggaccaagcaacatggtcagttttctcttgcagtcgtcagcctgaacataacatccttgggattacgctccctcaaggagataagtgatggagatgtgataatttcaggaaacaaaaatttgtgctatgcaaatacaataaactggaaaaaactgtttgggacctccggtcagaaaaccaaaattataagcaacagaggtgaaaacagctgcaaggccacaggccaggtctgccatgccttgtgctcccccgagggctgctggggcccggagcccagggactgcgtctctggtggcggtggctcgggcggtggtgggtcgggtggcggcggatctggtggcggtggctcgataacactcattatttttggggtgatggctggtgttattggaacgatcctcttagccctgctcatctggggaggtggaagc

SEQ ID NO: 87 - DNA, 711 bp, synthetic construct
  misc_feature 1..711: note = source = /note="Description of Artificial Sequence: Synthetic polynucleotide"
  misc_feature 1..711: note = source = /note="EGFR truncated design 11 (Her1 truncated design 11) (HER1t11)"
  source 1..711: mol_type = other DNA
cgcaaagtgtgtaacggaataggtattggtgaatttaaagactcactctccataaatgctacgaatattaaacacttcaaaaactgcacctccatcagtggcgatctccacatcctgccggtggcatttaggggtgactccttcacacatactcctcctctggatccacaggaactggatattctgaaaaccgtaaaggaaatcacagggtttttgctgattcaggcttggcctgaaaacaggacggacctccatgcctttgagaacctagaaatcatacgcggcaggaccaagcaacatggtcagttttctcttgcagtcgtcagcctgaacataacatccttgggattacgctccctcaaggagataagtgatggagatgtgataatttcaggaaacaaaaatttgtgctatgcaaatacaataaactggaaaaaactgtttgggacctccggtcagaaaaccaaaattataagcaacagaggtgaaaacagctgcaaggccacaggccaggtctgccatgccttgtgctcccccgagggctgctggggcccggagcccagggactgcgtctctggtggcggtggctcgggcggtggtgggtcgggtggcggcggatctggtggcggtggctcgctctgctacctgctggatggaatcctcttcatctatggtgtcattctcactgccttgttcctgggaggtggaagc

SEQ ID NO: 88 - DNA, 891 bp, synthetic construct
  misc_feature 1..891: note = source = /note="Description of Artificial Sequence: Synthetic polynucleotide"
  misc_feature 1..891: note = source = /note="FL CD20"
  source 1..891: mol_type = other DNA
atgacaacacccagaaattcagtaaatgggactttcccggcagagccaatgaaaggccctattgctatgcaatctggtccaaaaccactcttcaggaggatgtcttcactggtgggccccacgcaaagcttcttcatgagggaatctaagactttgggggctgtccagattatgaatgggctcttccacattgccctggggggtcttctgatgatcccagcagggatctatgcacccatctgtgtgactgtgtggtaccctctctggggaggcattatgtatattatttccggatcactcctggcagcaacggagaaaaactccaggaagtgtttggtcaaaggaaaaatgataatgaattcattgagcctctttgctgccatttctggaatgattctttcaatcatggacatacttaatattaaaatttcccattttttaaaaatggagagtctgaattttattagagctcacacaccatatattaacatatacaactgtgaaccagctaatccctctgagaaaaactccccatctacccaatactgttacagcatacaatctctgttcttgggcattttgtcagtgatgctgatctttgccttcttccaggaacttgtaatagctggcatcgttgagaatgaatggaaaagaacgtgctccagacccaaatctaacatagttctcctgtcagcagaagaaaaaaaagaacagactattgaaataaaagaagaagtggttgggctaactgaaacatcttcccaaccaaagaatgaagaagacattgaaattattccaatccaagaagaggaagaagaagaaacagagacgaactttccagaacctccccaagatcaggaatcctcaccaatagaaaatgacagctctcct

SEQ ID NO: 89 - DNA, 789 bp, synthetic construct
  misc_feature 1..789: note = source = /note="Description of Artificial Sequence: Synthetic polynucleotide"
  misc_feature 1..789: note = source = /note="Truncated CD20 design 1 (CD20t1) [CD20(M1-E263]"
  source 1..789: mol_type = other DNA
atgaccacaccacggaactctgtgaatggcaccttcccagcagagccaatgaagggaccaatcgcaatgcagagcggacccaagcctctgtttcggagaatgagctccctggtgggcccaacccagtccttctttatgagagagtctaagacactgggcgccgtgcagatcatgaacggactgttccacatcgccctgggaggactgctgatgatcccagccggcatctacgcccctatctgcgtgaccgtgtggtaccctctgtggggcggcatcatgtatatcatctccggctctctgctggccgccacagagaagaacagcaggaagtgtctggtgaagggcaagatgatcatgaatagcctgtccctgtttgccgccatctctggcatgatcctgagcatcatggacatcctgaacatcaagatcagccacttcctgaagatggagagcctgaacttcatcagagcccacaccccttacatcaacatctataattgcgagcctgccaacccatccgagaagaattctccaagcacacagtactgttattccatccagtctctgttcctgggcatcctgtctgtgatgctgatctttgccttctttcaggagctggtcatcgccggcatcgtggagaacgagtggaagaggacctgcagccgccccaagtccaatatcgtgctgctgtccgccgaggagaagaaggagcagacaatcgagatcaaggaggaggtggtgggcctgaccgagacatctagccagcctaagaatgaggaggatatcgag

SEQ ID NO: 90 - DNA, 342 bp, synthetic construct
  misc_feature 1..342: note = source = /note="Description of Artificial Sequence: Synthetic polynucleotide"
  misc_feature 1..342: note = source = /note="Interleukin-15"
  source 1..342: mol_type = other DNA
aactgggtgaatgtgatcagcgacctgaagaagatcgaggatctgatccagagcatgcacattgatgccaccctgtacacagaatctgatgtgcaccctagctgtaaagtgaccgccatgaagtgttttctgctggagctgcaggtgatttctctggaaagcggagatgcctctatccacgacacagtggagaatctgatcatcctggccaacaatagcctgagcagcaatggcaatgtgacagagtctggctgtaaggagtgtgaggagctggaggagaagaacatcaaggagtttctgcagagctttgtgcacatcgtgcagatgttcatcaatacaagc

SEQ ID NO: 91 - DNA, 711 bp, synthetic construct
  misc_feature 1..711: note = source = /note="Description of Artificial Sequence: Synthetic polynucleotide"
  misc_feature 1..711: note = source = /note="Interleukin-15 receptor alpha"
  source 1..711: mol_type = other DNA
attacatgccctcctccaatgtctgtggagcacgccgatatttgggtgaagtcctacagcctgtacagcagagagagatacatctgcaacagcggctttaagagaaaggccggcacctcttctctgacagagtgcgtgctgaataaggccacaaatgtggcccactggacaacacctagcctgaagtgcattagagatcctgccctggtccaccagaggcctgcccctccatctacagtgacaacagccggagtgacacctcagcctgaatctctgagcccttctggaaaagaacctgccgccagctctcctagctctaataataccgccgccacaacagccgccattgtgcctggatctcagctgatgcctagcaagtctcctagcacaggcacaacagagatcagcagccacgaatcttctcacggaacaccttctcagaccaccgccaagaattgggagctgacagcctctgcctctcaccagcctccaggagtgtatcctcagggccactctgatacaacagtggccatcagcacatctacagtgctgctgtgtggactgtctgccgtgtctctgctggcctgttacctgaagtctagacagacacctcctctggcctctgtggagatggaggccatggaagccctgcctgtgacatggggaacaagcagcagagatgaggacctggagaattgttctcaccacctg

SEQ ID NO: 92 - DNA, 1185 bp, synthetic construct
  misc_feature 1..1185: note = source = /note="Description of Artificial Sequence: Synthetic polynucleotide"
  misc_feature 1..1185: note = source = /note="Membrane bound Interleukin-15 with signal peptide"
  source 1..1185: mol_type = other DNA
atggattggacctggattctgtttctggtggccgctgccacaagagtgcacagcaactgggtgaatgtgatcagcgacctgaagaagatcgaggatctgatccagagcatgcacattgatgccaccctgtacacagaatctgatgtgcaccctagctgtaaagtgaccgccatgaagtgttttctgctggagctgcaggtgatttctctggaaagcggagatgcctctatccacgacacagtggagaatctgatcatcctggccaacaatagcctgagcagcaatggcaatgtgacagagtctggctgtaaggagtgtgaggagctggaggagaagaacatcaaggagtttctgcagagctttgtgcacatcgtgcagatgttcatcaatacaagctctggcggaggatctggaggaggcggatctggaggaggaggcagtggaggcggaggatctggcggaggatctctgcagattacatgccctcctccaatgtctgtggagcacgccgatatttgggtgaagtcctacagcctgtacagcagagagagatacatctgcaacagcggctttaagagaaaggccggcacctcttctctgacagagtgcgtgctgaataaggccacaaatgtggcccactggacaacacctagcctgaagtgcattagagatcctgccctggtccaccagaggcctgcccctccatctacagtgacaacagccggagtgacacctcagcctgaatctctgagcccttctggaaaagaacctgccgccagctctcctagctctaataataccgccgccacaacagccgccattgtgcctggatctcagctgatgcctagcaagtctcctagcacaggcacaacagagatcagcagccacgaatcttctcacggaacaccttctcagaccaccgccaagaattgggagctgacagcctctgcctctcaccagcctccaggagtgtatcctcagggccactctgatacaacagtggccatcagcacatctacagtgctgctgtgtggactgtctgccgtgtctctgctggcctgttacctgaagtctagacagacacctcctctggcctctgtggagatggaggccatggaagccctgcctgtgacatggggaacaagcagcagagatgaggacctggagaattgttctcaccacctg

SEQ ID NO: 93 - DNA, 1605 bp, Mus sp.
  misc_feature 1..1605: note = source = /note="Murine single chain IL-12 (p40-linker-p35)"
  source 1..1605: mol_type = other DNA
atgtgtcctcagaagctaaccatctcctggtttgccatcgttttgctggtgtctccactcatggccatgtgggagctggagaaagacgtttatgttgtagaggtggactggactcccgatgcccctggagaaacagtgaacctcacctgtgacacgcctgaagaagatgacatcacctggacctcagaccagagacatggagtcataggctctggaaagaccctgaccatcactgtcaaagagtttctagatgctggccagtacacctgccacaaaggaggcgagactctgagccactcacatctgctgctccacaagaaggaaaatggaatttggtccactgaaattctgaagaacttcaaaaacaagactttcctgaagtgtgaagcaccaaattacagcggccggttcacgtgctcatggctggtgcaaagaaacatggacttgaagttcaacatcaagagcagtagcagttcccctgactctcgggcagtgacatgtggaatggcgtctctgagcgccgagaaggtcacactggaccagagagactatgagaagtattcagtgtcctgccaggaggatgtcacctgcccaactgccgaggagaccctgcccattgaactggcgttggaagcacggcagcagaacaagtatgagaactacagcaccagcttcttcatcagggacatcatcaaaccagacccgcccaagaacttgcagatgaagcctttgaagaactcacaggtggaggtcagctgggagtaccctgactcctggagcactccccattcctacttctccctcaagttctttgtgagaatccagcgcaagaaagaaaagatgaaggagacagaggaggggtgtaaccagaaaggtgcgttcctcgtagagaagacatctaccgaagtccaatgcaaaggcgggaatgtctgcgtgcaagctcaggatcgctattacaattcctcatgcagcaagtgggcatgtgttccctgccgcgtccgatccggtggcggtggcggcggatctagggtcattccagtctctggacctgccaggtgtcttagccagtcccgaaacctgctgaagaccacagatgacatggtgaagacggccagagaaaaactgaaacattattcctgcactgctgaagacattgaccatgaagacatcacacgggaccaaaccagcacattgaagacctgtttaccactggaactacacaagaacgagagttgcctggctactagagagacttcttccacaacaagagggagctgcctgcccccacagaagaccagcttgatgatgaccctgtgccttggtagcatctatgaggacttgaagatgtaccagacagagttccaggccatcaacgcagcacttcagaatcacaaccatcagcagatcattctagacaagggcatgttggtggccatcgacgagctgatgcagtctctgaatcataatggcgagactctgcgccagaaacctcctgtgggagaagcagacccttacagagtgaaaatgaagctctgcatcctgcttcacgccttcagcacccgcgtcgtgaccatcaacagggtgatgggctatctgagcagcgcc

SEQ ID NO: 94 - DNA, 1596 bp, Homo sapiens
  misc_feature 1..1596: note = source = /note="Human single chain IL-12 (p40-linker-p35)"
  source 1..1596: mol_type = other DNA
atgtgtcaccagcagttggtcatctcttggttcagcctggtttttctggcatctcccctcgtggccatctgggaactgaagaaagatgtttatgtcgtagaattggattggtatcccgacgcccctggagaaatggtggtcctgacatgtgacacccctgaagaagatggtatcacctggaccttggaccagagcagtgaggtcttaggctctggcaagaccctgaccatccaagtcaaagagtttggagatgctggccagtacacctgtcacaaaggaggcgaggttctaagccattcgctcctgctgcttcacaaaaaggaagatggaatttggtccactgacattctgaaggaccagaaagaacccaagaataagacctttctaagatgcgaggccaagaattattctggacgtttcacctgctggtggctgacgacaatcagtactgatttgacattcagtgtcaaaagcagcagaggctcttctgacccccaaggggtgacgtgcggagctgctacactcagcgccgagagagtcagaggggacaacaaggagtatgagtactcagtggagtgccaggaggacagtgcctgcccagctgctgaggagagtctgcccattgaggtcatggtggatgccgttcacaagctcaagtatgaaaactacaccagcagcttcttcatcagggacatcatcaaacctgacccacccaagaacttgcagctgaagcccctgaagaacagcagacaggtggaggtcagctgggagtaccctgacacctggagtactccacattcctacttctccctgacattctgcgttcaggtccagggcaagagcaagagagaaaagaaagatagagtcttcacggacaagacctcagccacggtcatctgccgcaaaaatgccagcattagcgtgcgggcccaggaccgctactatagctcatcttggagcgaatgggcatctgtgccctgctccggtggcggtggcggcggatctagaaacctccccgtggccactccagacccaggaatgttcccatgccttcaccacagccagaacctgctgagggccgtcagcaacatgctccagaaggccagacaaactctagaattttacccttgcacttctgaagagattgatcatgaagatatcacaaaagataaaaccagcacagtggaggcctgtttaccattggaattaaccaagaatgagagttgcctaaattccagagagacctctttcataactaatgggagttgcctggcctccagaaagacctcttttatgatggccctgtgccttagtagtatttatgaagacttgaagatgtaccaggtggagttcaagaccatgaatgcaaagctgctgatggaccccaagaggcagatctttctagatcaaaacatgctggcagttattgatgagctgatgcaggccctgaatttcaacagtgagactgtgccacaaaaatcctcccttgaagaaccggatttttataaaactaaaatcaagctctgcatacttcttcatgctttcagaatcagagcagtgactattgatagagtgatgagctatctgaatgcttcc

SEQ ID NO: 95 - DNA, 6684 bp, Homo sapiens
  misc_feature 1..6684: note = source = /note="Human interleukin-2 (IL-2) gene and 5'-flanking region"
  source 1..6684: mol_type = genomic DNA
agtggtttttggagtcagtacattctcttttcaaatccttctctgccccttactggcaataagggctgagtgacctagaggcaaattacttaacttctctgagcctcagttttctaatctgcaaaataggagccatcacttcacaagtctgtaagacttatattagactaagtgcctgcctgtacactgttctctttttctctctttctatatacctgaaggcattatagtgctagatgtctgtttaaagaccagacaatattgtcttaaaaaaacaaacaaaaacacagacaataccatctttaaaaaaaaaaaaaaagtccaggtaagaaataaataaggccatagaatggaagctttacaaggactctctttgagacaggatctcctcaagtgtccccaggttaaattagaagtatatatccgtacaattgttcagccagtttgtgcactgtactgaggatgaatgaacacctatcctaaatatcctagtcttctgactaaaaacaagatcatatttcataacgattattgttacattcatagtgtcccaggtgatttagaggataaataaaaatccattaaagaggtaaagacataaaaacgagaaacatggactggtttacacataacacatacaaagtctattataaaactagcatcagtatccttgaatcgaaacctttttctgagtatttaacaatcgcaccctttaaaaaatgtacatagacattaagagacttaaacagatatataatcattttaaattaaaatagcgttaaacagtacctcaagctcaataagcattttaagtattctaatcttagtatttctctagctgacatgtaagaagcaatctatcttattgtatgcaattagctctttgtgtggataaaaaggtaaaaccattctgaaacaggaaaccaatacacttcctgtttaatcaacaaatctaaacatttattcttttcatctgtttactcttgctcttgtccaccacaatatgctattcacatgttcagtgtagttttatgacaaagaaaattttctgagttacttttgtatccccacccccttaaagaaaggaggaaaaactgtttcatacagaaggcgttaattgcatgaattagagctatcacctaagtgtgggctaatgtaacaaagagggatttcacctacatccattcagtcagtctttgggggtttaaagaaattccaaagagtcatcagaagaggaaaaatgaaggtaatgttttttcagactggtaaagtctttgaaaatatgtgtaatatgtaaaacattttgacacccccataatatttttccagaattaacagtataaattgcatctcttgttcaagagttccctatcactctttaatcactactcacagtaacctcaactcctgccacaatgtacaggatgcaactcctgtcttgcattgcactaagtcttgcacttgtcacaaacagtgcacctacttcaagttctacaaagaaaacacagctacaactggagcatttactgctggatttacagatgattttgaatggaattaatgtaagtatatttcctttcttactaaaattattacatttagtaatctagctggagatcatttcttaataacaatgcattatactttcttagaattacaagaatcccaaactcaccaggatgctcacatttaagttttacatgcccaagaaggtaagtacaatattttatgttcaatttctgttttaataaaattcaaagtaatatgaaaatttgcacagatgggactaatagcagctcatctgaggtaaagagtaactttaatttgtttttttgaaaacccaagtttgataatgaagcctctattaaaacagttttacctatatttttaatatatatttgtgtgttggtgggggtgggagaaaacataaaaataatattctctcactttatcgataagacaattctaaacaaaaatgttcatttatggtttcatttaaaaatgtaaaactctaaaatatttgattatgtcattttagtatgtaaaataccaaaatctatttccaaggagcccacttttaaaaatcttttcttgttttaggaaaggtttctaagtgagaggcagcataacactaatagcacagagtctggggccagatatctgaagtgaaatctcagctctgccatgtcctagctttcatgatctttggcaaattacctactctgtttgtgattcagtttcatgtctacttaaatgaataactgtatatacttaatatggctttgtgagaattagtaagtaaatgtaaagcactcagaaccgtgtctggcataaggtaaataccatacaagcattagctattattagtagtattaaagataaaattttcactgagaaatacaaagtaaaattttggactttatctttttaccaatagaacttgagatttataatgctatatgacttattttccaagattaaaagcttcattaggttgtttttggattcagatagagcataagcataatcatccaagctcctaggctacattaggtgtgtaaagctacctagtagctgtgccagttaagagagaatgaacaaaatctggtgccagaaagagcttgtgccagggtgaatccaagcccagaaaataataggatttaaggggacacagatgcaatcccattgactcaaattctattaattcaagacaaatctgcttctaactacccttctgaaagatgtaaaggagacagcttacagatgttactctagtttaatcagagccacataatgcaactccagcaacataaagatactagatgctgttttctgaagaaaatttctccacattgttcatgccaaaaacttaaacccgaatttgtagaatttgtagtggtgaattgaaagcgcaatagatggacatatcaggggattggtattgtcttgacctacctttcccactaaagagtgttagaaagatgagattatgtgcataatttaggggtggtagaattcatggaaatctaagtttgaaaccaaaagtaatgataaactctattcatttgttcatttaaccctcattgcacatttacaaaagattttagaaactaataaaaatatttgattccaaggatgctatgttaatgctataatgagaaagaaatgaaatctaattctggctctacctacttatgtggtcaaattctgagatttagtgtgcttatttataaagtggagatgatacttcactgcctacttcaaaagatgactgtgagaagtaaatgggcctattttggagaaaattcttttaaattgtaatataccatagaaatatgaaatattatatataatatagaatcaagaggcctgtccaaaagtcctcccaaagtattataatcttttatttcactgggacaaacatttttaaaatgcatcttaatgtagtgattgtagaaaagtaaaaatttaagacatatttaaaaatgtgtcttgctcaaggctatattgagagccactactacatgattattgttacctagtgtaaaatgttgggattgtgatagatggcatccaagagttccttctctctcaacattctgtgattcttaactcttagactatcaaatattataatcatagaatgtgatttttatgccttccacattctaatctcatctggttctaatgattttctatgcagattggaaaagtaatcagcctacatctgtaataggcatttagatgcagaaagtctaacattttgcaaagccaaattaagctaaaaccagtgagtcaactatcacttaacgctagtcataggtacttgagccctagtttttccagttttataatgtaaactctactggtccatctttacagtgacattgagaacagagagaatggtaaaaactacatactgctactccaaataaaataaattggaaattaatttctgattctgacctctatgtaaactgagctgatgataattattattctaggccacagaactgaaacatcttcagtgtctagaagaagaactcaaacctctggaggaagtgctaaatttagctcaaagcaaaaactttcacttaagacccagggacttaatcagcaatatcaacgtaatagttctggaactaaaggtaaggcattactttatttgctctcctggaaataaaaaaaaaaaagtagggggaaaagtaccacattttaaagtgacataacatttttggtatttgtaaagtacccatgcatgtaattagcctacattttaagtacactgtgaacatgaatcatttctaatgttaaatgattaactggggagtataagctactgagtttgcacctaccatctactaatggacaagcctcatcccaaactccatcacctttcatattaacacaaaactgggagtgagagagaagtgactgagttgagtttcacagaaacgcaggcaagattttattatatatttttcaagttccttcacagatcatttactggaatagccaatactgagttacctgaaaggcttttcaaatggtgtttccttatcatttgatggaaggactacccataagagatttgtcttaaaaaaaaaaactggagccattaaaatggccagtggactaaacaaacaacaatctttttagaggcaatcccactttcagaatcttaagtatttttaaatgcacaggaagcataaaatatgcaagggactcaggtgatgtaaaagagattcacttttgtctttttatatcccgtctcctaaggtataaaattcatgagttaataggtatcctaaataagcagcataagtatagtagtaaaagacattcctaaaagtaactccagttgtgtccaaatgaatcacttattagtggactgtttcagttgaattaaaaaaatacattgagatcaatgtcatctagacattgacagattcagttccttatctatggcaagagttttactctaaaataattaacatcagaaaactcattcttaactcttgatacaaatttaagacaaaaccatgcaaaaatctgaaaactgtgtttcaaaagccaaacactttttaaaataaaaaaatcccaagatatgacaatatttaaacaattatgcttaagaggatacagaacactgcaacagttttttaaaagagaatacttatttaaagggaacactctatctcacctgcttttgttcccagggtaggaatcacttcaaatttgaaaagctctcttttaaatctcactatatatcaaaatagttgcctccttagcttatcaactagaggaagcgtttaaatagctcctttcagcagagaagcctaatttctaaaaagccagtccacagaacaaaatttctaatgtttaaagcttttaaaagttggcaaattcacctgcattgatactatgatggggtagggataggtgtaagtatttatgaagatgttcattcacacaaatttacccaaacaggaagcatgtcctacctagcttactctagtgtagctcgtttcgtctttggggaaaatataaggagattcacttaagtagaaaaataggagactctaatcaagatttagaaaagaagaaagtataatgtgcatatcaattcatacatttaacttacacaaatataggtgtacattcagaggaaaagcgatcaagtttatttcacatccagcatttaatatttgtctagatctatttttatttaaatctttatttgcacccaatttagggaaaaaatttttgtgttcattgactgaattaacaaatgaggaaaatctcagcttctgtgttactatcatttggtatcataacaaaatacgcaattttggcattcattttgatcatttcaagaaaatgtgaataattaatatgtttggtaagcttgaaaataaaggcaacaggcctataagacttcaattgggaataactgtatataaggtaaactactctgtactttaaaaaattaacatttttcttttatagggatctgaaacaacattcatgtgtgaatatgctgatgagacagcaaccattgtagaatttctgaacagatggattaccttttgtcaaagcatcatctcaacactgacttgataattaagtgcttcccacttaaaacatatcaggccttctatttatttaaatatttaaattttatatttattgttgaatgtatggtttgctacctattgtaactattattcttaatcttaaaactataaatatggatcttttatgattctttttgtaagccctaggggctctaaaatggtttcacttatttatcccaaaatatttattattatgttgaatgttaaatatagtatctatgtagattggttagtaaaactatttaataaatttgataaatataaacaagcctggatatttgttattttggaaacagcacagagtaagcatttaaatatttcttagttacttgtgtgaactgtaggatggttaaaatgcttacaaaagtcactctttctctgaagaaatatgtagaacagagatgtagacttctcaaaagcccttgctttgtcctttcaagggctgatcagacccttagttctggcatctcttagcagattatattttccttcttcttaaaatgccaaacacaaacactcttgaaactcttcatagatttggtgtggc

SEQ ID NO: 96 - DNA, 1419 bp, synthetic construct
  misc_feature 1..1419: note = source = /note="Description of Artificial Sequence: Synthetic polynucleotide"
  misc_feature 1..1419: note = source = /note="CD19-specific chimeric antigen receptor (CD19-CD8a-CD28-CD3z)"
  source 1..1419: mol_type = other DNA
gacatccagatgacccagaccacctccagcctgagcgccagcctgggcgaccgggtgaccatcagctgccgggccagccaggacatcagcaagtacctgaactggtatcagcagaagcccgacggcaccgtcaagctgctgatctaccacaccagccggctgcacagcggcgtgcccagccggtttagcggcagcggctccggcaccgactacagcctgaccatctccaacctggagcaggaggacatcgccacctacttttgccagcagggcaacacactgccctacacctttggcggcggaacaaagctggagatcaccggcagcacctccggcagcggcaagcctggcagcggcgagggcagcaccaagggcgaggtgaagctgcaggagagcggccctggcctggtggcccccagccagagcctgagcgtgacctgtaccgtgtccggcgtgtccctgcccgactacggcgtgtcctggatccggcagccccctaggaagggcctggagtggctgggcgtgatctggggcagcgagaccacctactacaacagcgccctgaagagccggctgaccatcatcaaggacaacagcaagagccaggtgttcctgaagatgaacagcctgcagaccgacgacaccgccatctactactgtgccaagcactactactacggcggcagctacgccatggactactggggccagggcaccagcgtgaccgtgtccagcaagcccaccaccacccctgcccctagacctccaaccccagcccctacaatcgccagccagcccctgagcctgaggcccgaagcctgtagacctgccgctggcggagccgtgcacaccagaggcctggatttcgcctgcgacatctacatctgggcccctctggccggcacctgtggcgtgctgctgctgagcctggtcatcaccctgtactgcaaccaccggaataggagcaagcggagcagaggcggccacagcgactacatgaacatgaccccccggaggcctggccccacccggaagcactaccagccctacgcccctcccagggacttcgccgcctaccggagccgggtgaagttcagccggagcgccgacgcccctgcctaccagcagggccagaaccagctgtacaacgagctgaacctgggccggagggaggagtacgacgtgctggacaagcggagaggccgggaccctgagatgggcggcaagccccggagaaagaaccctcaggagggcctgtataacgaactgcagaaagacaagatggccgaggcctacagcgagatcggcatgaagggcgagcggcggaggggcaagggccacgacggcctgtaccagggcctgagcaccgccaccaaggatacctacgacgccctgcacatgcaggccctgccccccaga

SEQ ID NO: 97 - DNA, 1485 bp, synthetic construct
  misc_feature 1..1485: note = source = /note="Description of Artificial Sequence: Synthetic polynucleotide"
  misc_feature 1..1485: note = source = /note="CD19-specific chimeric antigen receptor (CD19-CD8a-CD28-CD3z) with Signal peptide"
  source 1..1485: mol_type = other DNA
atgctgctgctggtgaccagcctgctgctgtgtgagctgccccaccccgcctttctgctgatccccgacatccagatgacccagaccacctccagcctgagcgccagcctgggcgaccgggtgaccatcagctgccgggccagccaggacatcagcaagtacctgaactggtatcagcagaagcccgacggcaccgtcaagctgctgatctaccacaccagccggctgcacagcggcgtgcccagccggtttagcggcagcggctccggcaccgactacagcctgaccatctccaacctggagcaggaggacatcgccacctacttttgccagcagggcaacacactgccctacacctttggcggcggaacaaagctggagatcaccggcagcacctccggcagcggcaagcctggcagcggcgagggcagcaccaagggcgaggtgaagctgcaggagagcggccctggcctggtggcccccagccagagcctgagcgtgacctgtaccgtgtccggcgtgtccctgcccgactacggcgtgtcctggatccggcagccccctaggaagggcctggagtggctgggcgtgatctggggcagcgagaccacctactacaacagcgccctgaagagccggctgaccatcatcaaggacaacagcaagagccaggtgttcctgaagatgaacagcctgcagaccgacgacaccgccatctactactgtgccaagcactactactacggcggcagctacgccatggactactggggccagggcaccagcgtgaccgtgtccagcaagcccaccaccacccctgcccctagacctccaaccccagcccctacaatcgccagccagcccctgagcctgaggcccgaagcctgtagacctgccgctggcggagccgtgcacaccagaggcctggatttcgcctgcgacatctacatctgggcccctctggccggcacctgtggcgtgctgctgctgagcctggtcatcaccctgtactgcaaccaccggaataggagcaagcggagcagaggcggccacagcgactacatgaacatgaccccccggaggcctggccccacccggaagcactaccagccctacgcccctcccagggacttcgccgcctaccggagccgggtgaagttcagccggagcgccgacgcccctgcctaccagcagggccagaaccagctgtacaacgagctgaacctgggccggagggaggagtacgacgtgctggacaagcggagaggccgggaccctgagatgggcggcaagccccggagaaagaaccctcaggagggcctgtataacgaactgcagaaagacaagatggccgaggcctacagcgagatcggcatgaagggcgagcggcggaggggcaagggccacgacggcctgtaccagggcctgagcaccgccaccaaggatacctacgacgccctgcacatgcaggccctgccccccaga

SEQ ID NO: 98 - DNA, 360 bp, synthetic construct
  misc_feature 1..360: note = source = /note="Description of Artificial Sequence: Synthetic polynucleotide"
  misc_feature 1..360: note = source = /note="Anti-CD19 monoclonal antibody clone FMC63 variable heavy chain"
  source 1..360: mol_type = other DNA
gaggtgaagctgcaggagagcggccctggcctggtggcccccagccagagcctgagcgtgacctgtaccgtgtccggcgtgtccctgcccgactacggcgtgtcctggatccggcagccccctaggaagggcctggagtggctgggcgtgatctggggcagcgagaccacctactacaacagcgccctgaagagccggctgaccatcatcaaggacaacagcaagagccaggtgttcctgaagatgaacagcctgcagaccgacgacaccgccatctactactgtgccaagcactactactacggcggcagctacgccatggactactggggccagggcaccagcgtgaccgtgtccagc

SEQ ID NO: 99 - DNA, 735 bp, synthetic construct
  misc_feature 1..735: note = source = /note="Description of Artificial Sequence: Synthetic polynucleotide"
  misc_feature 1..735: note = source = /note="Anti-CD19 clone FMC63 single chain fragment variable (scFv) with Whitlow linker"
  source 1..735: mol_type = other DNA
gacatccagatgacccagaccacctccagcctgagcgccagcctgggcgaccgggtgaccatcagctgccgggccagccaggacatcagcaagtacctgaactggtatcagcagaagcccgacggcaccgtcaagctgctgatctaccacaccagccggctgcacagcggcgtgcccagccggtttagcggcagcggctccggcaccgactacagcctgaccatctccaacctggagcaggaggacatcgccacctacttttgccagcagggcaacacactgccctacacctttggcggcggaacaaagctggagatcaccggcagcacctccggcagcggcaagcctggcagcggcgagggcagcaccaagggcgaggtgaagctgcaggagagcggccctggcctggtggcccccagccagagcctgagcgtgacctgtaccgtgtccggcgtgtccctgcccgactacggcgtgtcctggatccggcagccccctaggaagggcctggagtggctgggcgtgatctggggcagcgagaccacctactacaacagcgccctgaagagccggctgaccatcatcaaggacaacagcaagagccaggtgttcctgaagatgaacagcctgcagaccgacgacaccgccatctactactgtgccaagcactactactacggcggcagctacgccatggactactggggccagggcaccagcgtgaccgtgtccagc

SEQ ID NO: 100 - DNA, 333 bp, synthetic construct
  misc_feature 1..333: note = source = /note="Description of Artificial Sequence: Synthetic polynucleotide"
  misc_feature 1..333: note = source = /note="hM195 VL"
  source 1..333: mol_type = other DNA
gacattcagatgacccagtctccgagctctctgtccgcatcagtaggagacagggtcaccatcacatgcagagccagcgaaagtgtcgacaattatggcattagctttatgaactggttccaacagaaacccgggaaggctcctaagcttctgatttacgctgcatccaaccaaggctccggggtaccctctcgcttctcaggcagtggatctgggacagacttcactctcaccatttcatctctgcagcctgatgacttcgcaacctattactgtcagcaaagtaaggaggttccgtggacgttcggtcaagggaccaaggtggagatcaaa

SEQ ID NO: 101 - DNA, 348 bp, synthetic construct
  misc_feature 1..348: note = source = /note="Description of Artificial Sequence: Synthetic polynucleotide"
  misc_feature 1..348: note = source = /note="hM195 VH"
  source 1..348: mol_type = other DNA
caggttcagctggtgcagtctggagctgaggtgaagaagcctgggagctcagtgaaggtttcctgcaaagcttctggctacaccttcactgactacaacatgcactgggtgaggcaggctcctggccaaggcctggaatggattggatatatttatccttacaatggtggtaccggctacaaccagaagttcaagagcaaggccacaattacagcagacgagagtactaacacagcctacatggaactctccagcctgaggtctgaggacactgcagtctattactgcgcaagagggcgccccgctatggactactggggccaagggactctggtcactgtctcttca

SEQ ID NO: 102 - DNA, 726 bp, synthetic construct
  misc_feature 1..726: note = source = /note="Description of Artificial Sequence: Synthetic polynucleotide"
  misc_feature 1..726: note = source = /note="hM195 scFv with linker"
  source 1..726: mol_type = other DNA
gacattcagatgacccagtctccgagctctctgtccgcatcagtaggagacagggtcaccatcacatgcagagccagcgaaagtgtcgacaattatggcattagctttatgaactggttccaacagaaacccgggaaggctcctaagcttctgatttacgctgcatccaaccaaggctccggggtaccctctcgcttctcaggcagtggatctgggacagacttcactctcaccatttcatctctgcagcctgatgacttcgcaacctattactgtcagcaaagtaaggaggttccgtggacgttcggtcaagggaccaaggtggagatcaaaggtggcggtggctcgggcggtggtgggtcgggtggcggcggatctcaggttcagctggtgcagtctggagctgaggtgaagaagcctgggagctcagtgaaggtttcctgcaaagcttctggctacaccttcactgactacaacatgcactgggtgaggcaggctcctggccaaggcctggaatggattggatatatttatccttacaatggtggtaccggctacaaccagaagttcaagagcaaggccacaattacagcagacgagagtactaacacagcctacatggaactctccagcctgaggtctgaggacactgcagtctattactgcgcaagagggcgccccgctatggactactggggccaagggactctggtcactgtctcttca

SEQ ID NO: 103 - DNA, 2773 bp, synthetic construct
  misc_feature 1..2773: note = source = /note="Description of Artificial Sequence: Synthetic polynucleotide"
  misc_feature 1..2773: note = source = /note="EGFR variant III (EGFRvIII)"
  source 1..2773: mol_type = other DNA
atgcgaccctccgggacggccggggcagcgctcctggcgctgctggctgcgctctgcccggcgagtcgggctctggaggaaaagaaaggtaattatgtggtgacagatcacggctcgtgcgtccgagcctgtggggccgacagctatgagatggaggaagacggcgtccgcaagtgtaagaagtgcgaagggccttgccgcaaagtgtgtaacggaataggtattggtgaatttaaagactcactctccataaatgctacgaatattaaacacttcaaaaactgcacctccatcagtggcgatctccacatcctgccggtggcatttaggggtgactccttcacacatactcctcctctggatccacaggaactggatattctgaaaaccgtaaaggaaatcacagggtttttgctgattcaggcttggcctgaaaacaggacggacctccatgcctttgagaacctagaaatcatacgcggcaggaccaagcaacatggtcagttttctcttgcagtcgtcagcctgaacataacatccttgggattacgctccctcaaggagataagtgatggagatgtgataatttcaggaaacaaaaatttgtgctatgcaaatacaataaactggaaaaaactgtttgggacctccggtcagaaaaccaaaattataagcaacagaggtgaaaacagctgcaaggccacaggccaggtctgccatgccttgtgctcccccgagggctgctggggcccggagcccagggactgcgtctcttgccggaatgtcagccgaggcagggaatgcgtggacaagtgcaaccttctggagggtgagccaagggagtttgtggagaactctgagtgcatacagtgccacccagagtgcctgcctcaggccatgaacatcacctgcacaggacggggaccagacaggagtcatgggagaaaacaacaccctggtctggaagtacgcagacgccggccatgtgtgccacctgtgccatccaaactgcacctacggatgcactgggccaggtcttgaaggctgtccaacgaatgggcctaagatcccgtccatcgccactgggatggtgggggccctcctcttgctgctggtggtggccctggggatcggcctcttcatgcgaaggcgccacatcgttcggaagcgcacgctgcggaggctgctgcaggagagggagcttgtggagcctcttacacccagtggagaagctcccaaccaagctctcttgaggatcttgaaggaaactgaattcaaaaagatcaaagtgctgggctccggtgcgttcggcacggtgtataagggactctggatcccagaaggtgagaaagttaaaattcccgtcgctatcaaggaattaagagaagcaacatctccgaaagccaacaaggaaatcctcgatgaagcctacgtgatggccagcgtggacaacccccacgtgtgccgcctgctgggcatctgcctcacctccaccgtgcagctcatcacgcagctcatgcccttcggctgcctcctggactatgtccgggaacacaaagacaatattggctcccagtacctgctcaactggtgtgtgcagatcgcaaagggcatgaactacttggaggaccgtcgcttggtgcaccgcgacctggcagccaggaacgtactggtgaaaacaccgcagcatgtcaagatcacagattttgggctggccaaactgctgggtgcggaagagaaagaataccatgcagaaggaggcaaagtgcctatcaagtggatggcattggaatcaattttacacagaatctatacccaccagagtgatgtctggagctacggggtgactgtttgggagttgatgacctttggatccaagccatatgacggaatccctgccagcgagatctcctccatcctggagaaaggagaacgcctccctcagccacccatatgtaccatcgatgtctacatgatcatggtcaagtgctggatgatagacgcagatagtcgcccaaagttccgtgagttgatcatcgaattctccaaaatggcccgagacccccagcgctaccttgtcattcagggggatgaaagaatgcatttgccaagtcctacagactccaacttctaccgtgccctgatggatgaagaagacatggacgacgtggtggatgccgacgagtacctcatcccacagcagggcttcttcagcagcccctccacgtcacggactcccctcctgagctctctgagtgcaaccagcaacaattccaccgtggcttgcattgatagaaatgggctgcaaagctgtcccatcaaggaagacagcttcttgcagcgatacagctcagaccccacaggcgccttgactgaggacagcatagacgacaccttcctcccagtgcctgaatacataaaccagtccgttcccaaaaggcccgctggctctgtgcagaatcctgtctatcacaatcagcctctgaaccccgcgcccagcagagacccacactaccaggacccccacagcactgcagtgggcaaccccgagtatctcaacactgtccagcccacctgtgtcaacagcacattcgacagccctgcccactgggcccagaaaggcagccaccaaattagcctggacaaccctgactaccagcaggacttctttcccaaggaagccaagccaaatggcatctttaagggctccacagctgaaaatgcagaatacctaagggtcgcgccacaaagcagtgaatttattggagcatga

SEQ ID NO: 104 - DNA, 348 bp, synthetic construct
  misc_feature 1..348: note = source = /note="Description of Artificial Sequence: Synthetic polynucleotide"
  misc_feature 1..348: note = source = /note="Anti- EGFRvIII Clone 139 VH"
  source 1..348: mol_type = other DNA
gaagtgcaggtgctggaaagcggcggaggactggtgcagcctggcggatctctgagactgagctgtgccgccagcggcttcaccttcagcagctacgccatgagctgggtgcgccaggcccctggaaaaggcctggaatgggtgtccgccatctctggctccggcggcagcaccaattacgccgatagcgtgaagggccggttcaccatcagccgggacaacagcaagaacaccctgtacctgcagatgaacagcctgagagccgaggacaccgccgtgtactactgtgccggaagctctgggtggagcgagtattggggccagggcacactcgtgaccgtgtccagc

SEQ ID NO: 105 - DNA, 321 bp, synthetic construct
  misc_feature 1..321: note = source = /note="Description of Artificial Sequence: Synthetic polynucleotide"
  misc_feature 1..321: note = source = /note="Anti- EGFRvIII Clone 139 VL"
  source 1..321: mol_type = other DNA
gacatccagatgacccagagccccagcagcctgtctgccagcgtgggcgacagagtgaccatcacctgtagagccagccagggcatccggaacaacctggcctggtatcagcagaagcccggcaaggcccccaagcggctgatctacgccgccagcaatctgcagagcggcgtgccctctagattcaccggctctggcagcggcaccgagttcaccctgatcgtgtctagcctgcagcccgaggacttcgccacctactactgcctgcagcaccacagctaccccctgacatctggcggaggcaccaaggtggaaatcaag

SEQ ID NO: 106 - DNA, 360 bp, synthetic construct
  misc_feature 1..360: note = source = /note="Description of Artificial Sequence: Synthetic polynucleotide"
  misc_feature 1..360: note = source = /note="Anti- EGFRvIII Clone MR1 VH"
  source 1..360: mol_type = other DNA
caagtgaagctgcagcagtctggcggaggcctcgtgaaacctggcgcctctctgaagctgagctgcgtgaccagcggcttcaccttcagaaagttcggcatgagctgggtgcgccagaccagcgacaagcggctggaatgggtggccagcatcagcaccggcggctacaacacctactacagcgacaacgtgaagggcagattcaccatcagcagagagaacgccaagaataccctgtacctgcagatgagcagcctgaagtccgaggacaccgccctgtactactgcaccagaggctacagcagcaccagctacgccatggactattggggccagggcaccaccgtgaccgtgtctagt

SEQ ID NO: 107 - DNA, 321 bp, synthetic construct
  misc_feature 1..321: note = source = /note="Description of Artificial Sequence: Synthetic polynucleotide"
  misc_feature 1..321: note = source = /note="Anti- EGFRvIII Clone MR1 VL"
  source 1..321: mol_type = other DNA
gacatcgagctgacacagagccctgccagcctgtctgtggccaccggcgagaaagtgaccatccggtgcatgaccagcaccgacatcgacgacgacatgaactggtatcagcagaagcccggcgagccccccaagttcctgatcagcgagggcaacacactgcggcctggcgtgccaagcagattcagcagctctggcaccggcaccgacttcgtgttcaccatcgagaacaccctgagcgaggacgtgggcgactactactgcctgcagagcttcaacgtgcccctgacctttggcgacggcaccaagctggaaatcaag

SEQ ID NO: 108 - DNA, 360 bp, synthetic construct
  misc_feature 1..360: note = source = /note="Description of Artificial Sequence: Synthetic polynucleotide"
  misc_feature 1..360: note = source = /note="Anti- EGFRvIII Clone MR1-1 VH"
  source 1..360: mol_type = other DNA
caagtgaagctgcagcagtctggcggaggcctcgtgaaacctggcgcctctctgaagctgagctgcgtgaccagcggcttcaccttcagaaagttcggcatgagctgggtgcgccagaccagcgacaagcggctggaatgggtggccagcatcagcaccggcggctacaacacctactacagcgacaacgtgaagggcagattcaccatcagcagagagaacgccaagaataccctgtacctgcagatgagcagcctgaagtccgaggacaccgccctgtactactgcaccagaggctacagcccctacagctacgccatggactattggggccagggcaccaccgtgaccgtgtctagt

SEQ ID NO: 109 - DNA, 321 bp, synthetic construct
  misc_feature 1..321: note = source = /note="Description of Artificial Sequence: Synthetic polynucleotide"
  misc_feature 1..321: note = source = /note="Anti- EGFRvIII Clone MR1-1 VL"
  source 1..321: mol_type = other DNA
gacatcgagctgacacagagccctgccagcctgtctgtggccaccggcgagaaagtgaccatccggtgcatgaccagcaccgacatcgacgacgacatgaactggtatcagcagaagcccggcgagccccccaagttcctgatcagcgagggcaacacactgcggcctggcgtgccaagcagattcagcagctctggcaccggcaccgacttcgtgttcaccatcgagaacaccctgagcgaggacgtgggcgactactactgcctgcagagctggaacgtgcccctgacctttggcgacggcaccaagctggaaatcaag

SEQ ID NO: 110 - DNA, 360 bp, synthetic construct
  misc_feature 1..360: note = source = /note="Description of Artificial Sequence: Synthetic polynucleotide"
  misc_feature 1..360: note = source = /note="Anti- EGFRvIII Clone humMR1-1 VH"
  source 1..360: mol_type = other DNA
caggtgcagctgcaggaatctggcggagggctcgtgaagcctggcggaagcctgaagctgagctgtgccgccagcggcttcaccttcagcaagttcggcatgagctgggtgcgccagacccccgacaagagactggaatgggtggccagcatcagcaccggcggctacaatacctactacagcgacaacgtgaagggccggttcaccatctcccgggacaacgccaagaacaccctgtacctgcagatgagcagcctgaagtccgaggacaccgccatgtactactgtgccagaggctacagcccctacagctacgccatggattactggggccagggcacaatggtcaccgtgtcctct

SEQ ID NO: 111 - DNA, 321 bp, synthetic construct
  misc_feature 1..321: note = source = /note="Description of Artificial Sequence: Synthetic polynucleotide"
  misc_feature 1..321: note = source = /note="Anti- EGFRvIII Clone humMR1-1 VL"
  source 1..321: mol_type = other DNA
gacatccagatgacccagagccccagcagcctgtctgccagcgtgggcgacagagtgaccatcacctgtatgaccagcaccgacatcgacgacgacatgaactggtatcagcagaagcccggcaagacccccaagctgctgatctacgagggcaacaccctgaggcctggcgtgcccagcagattttctggcagcggctccggcaccgacttcatcttcaccatcagctccctgcagcccgaggatatcgccacctactactgcctgcagagctggaacgtgcccctgacctttggcggaggcaccaaggtggaaatcaag

SEQ ID NO: 112 - DNA, 360 bp, synthetic construct
  misc_feature 1..360: note = source = /note="Description of Artificial Sequence: Synthetic polynucleotide"
  misc_feature 1..360: note = source = /note="Anti- EGFRvIII Clone humMR1-2 VH"
  source 1..360: mol_type = other DNA
caggtgcagctgcaggaatctggcggagggctcgtgaagcctggcggaagcctgaagctgagctgtgccgccagcggcttcaccttcagcaagttcggcatgagctgggtgcgccagacccccgacaagagactggaatgggtggccagcatcagcaccggcggctacaacaccttctacagcgacaacgtgaagggccggttcaccatctcccgggacaacgccaagaacaccctgtacctgcagatgagcagcctgaagtccgaggacaccgccatgtactactgtgccagaggctacagcccctacagcttcgccatggattactggggccagggcacaatggtcaccgtgtcctct

SEQ ID NO: 113 - DNA, 321 bp, synthetic construct; identical to SEQ ID NO: 111
  misc_feature 1..321: note = source = /note="Description of Artificial Sequence: Synthetic polynucleotide"
  misc_feature 1..321: note = source = /note="Anti- EGFRvIII Clone humMR1-2 VL"
  source 1..321: mol_type = other DNA

SEQ ID NO: 114 - DNA, 723 bp, synthetic construct
  misc_feature 1..723: note = source = /note="Description of Artificial Sequence: Synthetic polynucleotide"
  misc_feature 1..723: note = source = /note="Anti- EGFRvIII scFv Clone 139"
  source 1..723: mol_type = other DNA
gacatccagatgacccagagccccagcagcctgtctgccagcgtgggcgacagagtgaccatcacctgtagagccagccagggcatccggaacaacctggcctggtatcagcagaagcccggcaaggcccccaagcggctgatctacgccgccagcaatctgcagagcggcgtgccctctagattcaccggctctggcagcggcaccgagttcaccctgatcgtgtctagcctgcagcccgaggacttcgccacctactactgcctgcagcaccacagctaccccctgacatctggcggaggcaccaaggtggaaatcaagggcagcacaagcggcagcggaaaacctggatctggcgagggctctaccaagggcgaagtgcaggtgctggaaagcggcggaggactggtgcagcctggcggatctctgagactgagctgtgccgccagcggcttcaccttcagcagctacgccatgagctgggtgcgccaggcccctggaaaaggcctggaatgggtgtccgccatctctggctccggcggcagcaccaattacgccgatagcgtgaagggccggttcaccatcagccgggacaacagcaagaacaccctgtacctgcagatgaacagcctgagagccgaggacaccgccgtgtactactgtgccggaagctctgggtggagcgagtattggggccagggcacactcgtgaccgtgtccagc

SEQ ID NO: 115 - DNA, 726 bp, synthetic construct
  misc_feature 1..726: note = source = /note="Description of Artificial Sequence: Synthetic polynucleotide"
  misc_feature 1..726: note = source = /note="Anti-EGFRvIII scFv clone MR1"
  source 1..726: mol_type = other DNA
gacatcgagctgacacagagccctgccagcctgtctgtggccaccggcgagaaagtgaccatccggtgcatgaccagcaccgacatcgacgacgacatgaactggtatcagcagaagcccggcgagccccccaagttcctgatcagcgagggcaacacactgcggcctggcgtgccaagcagattcagcagctctggcaccggcaccgacttcgtgttcaccatcgagaacaccctgagcgaggacgtgggcgactactactgcctgcagagcttcaacgtgcccctgacctttggcgacggcaccaagctggaaatcaagggcggaggcggatctggcggcggaggatctgggggaggcggctctcaagtgaagctgcagcagtctggcggaggcctcgtgaaacctggcgcctctctgaagctgagctgcgtgaccagcggcttcaccttcagaaagttcggcatgagctgggtgcgccagaccagcgacaagcggctggaatgggtggccagcatcagcaccggcggctacaacacctactacagcgacaacgtgaagggcagattcaccatcagcagagagaacgccaagaataccctgtacctgcagatgagcagcctgaagtccgaggacaccgccctgtactactgcaccagaggctacagcagcaccagctacgccatggactattggggccagggcaccaccgtgaccgtgtctagt

SEQ ID NO: 116 - DNA, 726 bp, synthetic construct
  misc_feature 1..726: note = source = /note="Description of Artificial Sequence: Synthetic polynucleotide"
  misc_feature 1..726: note = source = /note="Anti EGFRvIII scFv clone MR1-1"
  source 1..726: mol_type = other DNA
gacatcgagctgacacagagccctgccagcctgtctgtggccaccggcgagaaagtgaccatccggtgcatgaccagcaccgacatcgacgacgacatgaactggtatcagcagaagcccggcgagccccccaagttcctgatcagcgagggcaacacactgcggcctggcgtgccaagcagattcagcagctctggcaccggcaccgacttcgtgttcaccatcgagaacaccctgagcgaggacgtgggcgactactactgcctgcagagctggaacgtgcccctgacctttggcgacggcaccaagctggaaatcaagggcggaggcggatctggcggcggaggatctgggggaggcggctctcaagtgaagctgcagcagtctggcggaggcctcgtgaaacctggcgcctctctgaagctgagctgcgtgaccagcggcttcaccttcagaaagttcggcatgagctgggtgcgccagaccagcgacaagcggctggaatgggtggccagcatcagcaccggcggctacaacacctactacagcgacaacgtgaagggcagattcaccatcagcagagagaacgccaagaataccctgtacctgcagatgagcagcctgaagtccgaggacaccgccctgtactactgcaccagaggctacagcccctacagctacgccatggactattggggccagggcaccaccgtgaccgtgtctagt

SEQ ID NO: 117 - DNA, 726 bp, synthetic construct
  misc_feature 1..726: note = source = /note="Description of Artificial Sequence: Synthetic polynucleotide"
  misc_feature 1..726: note = source = /note="Anti-EGFRvIII scFv clone huMR1-1"
  source 1..726: mol_type = other DNA
gacatccagatgacccagagccccagcagcctgtctgccagcgtgggcgacagagtgaccatcacctgtatgaccagcaccgacatcgacgacgacatgaactggtatcagcagaagcccggcaagacccccaagctgctgatctacgagggcaacaccctgaggcctggcgtgcccagcagattttctggcagcggctccggcaccgacttcatcttcaccatcagctccctgcagcccgaggatatcgccacctactactgcctgcagagctggaacgtgcccctgacctttggcggaggcaccaaggtggaaatcaagggcggaggcggatctggcggcggaggatctgggggaggcggctctcaggtgcagctgcaggaatctggcggagggctcgtgaagcctggcggaagcctgaagctgagctgtgccgccagcggcttcaccttcagcaagttcggcatgagctgggtgcgccagacccccgacaagagactggaatgggtggccagcatcagcaccggcggctacaatacctactacagcgacaacgtgaagggccggttcaccatctcccgggacaacgccaagaacaccctgtacctgcagatgagcagcctgaagtccgaggacaccgccatgtactactgtgccagaggctacagcccctacagctacgccatggattactggggccagggcacaatggtcaccgtgtcctct

SEQ ID NO: 118 - DNA, 726 bp, synthetic construct
  misc_feature 1..726: note = source = /note="Description of Artificial Sequence: Synthetic polynucleotide"
  misc_feature 1..726: note = source = /note="Anti-EGFRvIII scFv clone huMR1-2"
  source 1..726: mol_type = other DNA
gacatccagatgacccagagccccagcagcctgtctgccagcgtgggcgacagagtgaccatcacctgtatgaccagcaccgacatcgacgacgacatgaactggtatcagcagaagcccggcaagacccccaagctgctgatctacgagggcaacaccctgaggcctggcgtgcccagcagattttctggcagcggctccggcaccgacttcatcttcaccatcagctccctgcagcccgaggatatcgccacctactactgcctgcagagctggaacgtgcccctgacctttggcggaggcaccaaggtggaaatcaagggcggaggcggatctggcggcggaggatctgggggaggcggctctcaggtgcagctgcaggaatctggcggagggctcgtgaagcctggcggaagcctgaagctgagctgtgccgccagcggcttcaccttcagcaagttcggcatgagctgggtgcgccagacccccgacaagagactggaatgggtggccagcatcagcaccggcggctacaacaccttctacagcgacaacgtgaagggccggttcaccatctcccgggacaacgccaagaacaccctgtacctgcagatgagcagcctgaagtccgaggacaccgccatgtactactgtgccagaggctacagcccctacagcttcgccatggattactggggccagggcacaatggtcaccgtgtcctct

SEQ ID NO: 119 - DNA, 1410 bp, synthetic construct
  misc_feature 1..1410: note = source = /note="Description of Artificial Sequence: Synthetic polynucleotide"
  misc_feature 1..1410: note = source = /note="EGFRvIII CAR (clone 139 scFv.CD8alpha hinge &TM.4-1BB.CD3-zeta)"
  source 1..1410: mol_type = other DNA
gacatccagatgacccagagccccagcagcctgtctgccagcgtgggcgacagagtgaccatcacctgtagagccagccagggcatccggaacaacctggcctggtatcagcagaagcccggcaaggcccccaagcggctgatctacgccgccagcaatctgcagagcggcgtgccctctagattcaccggctctggcagcggcaccgagttcaccctgatcgtgtctagcctgcagcccgaggacttcgccacctactactgcctgcagcaccacagctaccccctgacatctggcggaggcaccaaggtggaaatcaagggcagcacaagcggcagcggaaaacctggatctggcgagggctctaccaagggcgaagtgcaggtgctggaaagcggcggaggactggtgcagcctggcggatctctgagactgagctgtgccgccagcggcttcaccttcagcagctacgccatgagctgggtgcgccaggcccctggaaaaggcctggaatgggtgtccgccatctctggctccggcggcagcaccaattacgccgatagcgtgaagggccggttcaccatcagccgggacaacagcaagaacaccctgtacctgcagatgaacagcctgagagccgaggacaccgccgtgtactactgtgccggaagctctgggtggagcgagtattggggccagggcacactcgtgaccgtgtccagcaagcccaccaccacccctgcccctagacctccaaccccagcccctacaatcgccagccagcccctgagcctgaggcccgaagcctgtagacctgccgctggcggagccgtgcacaccagaggcctggatttcgcctgcgacatctacatctgggcccctctggccggcacctgtggcgtgctgctgctgagcctggtcatcaccctgtactgcaaccaccggaataagagaggccggaagaaactgctgtacatcttcaagcagcccttcatgcggcccgtgcagaccacccaggaagaggacggctgcagctgccggttccccgaggaagaggaaggcggctgcgaactgcgggtgaagttcagccggagcgccgacgcccctgcctaccagcagggccagaaccagctgtacaacgagctgaacctgggccggagggaggagtacgacgtgctggacaagcggagaggccgggaccctgagatgggcggcaagccccggagaaagaaccctcaggagggcctgtataacgaactgcagaaagacaagatggccgaggcctacagcgagatcggcatgaagggcgagcggcggaggggcaagggccacgacggcctgtaccagggcctgagcaccgccaccaaggatacctacgacgccctgcacatgcaggccctgccccccaga

SEQ ID NO: 120 - DNA, 1413 bp, synthetic construct
  misc_feature 1..1413: note = source = /note="Description of Artificial Sequence: Synthetic polynucleotide"
  misc_feature 1..1413: note = source = /note="EGFRvIII CAR (MR1 scFv.CD8alpha hinge &TM.4-1BB.CD3-zeta)"
  source 1..1413: mol_type = other DNA
gacatcgagctgacacagagccctgccagcctgtctgtggccaccggcgagaaagtgaccatccggtgcatgaccagcaccgacatcgacgacgacatgaactggtatcagcagaagcccggcgagccccccaagttcctgatcagcgagggcaacacactgcggcctggcgtgccaagcagattcagcagctctggcaccggcaccgacttcgtgttcaccatcgagaacaccctgagcgaggacgtgggcgactactactgcctgcagagcttcaacgtgcccctgacctttggcgacggcaccaagctggaaatcaagggcggaggcggatctggcggcggaggatctgggggaggcggctctcaagtgaagctgcagcagtctggcggaggcctcgtgaaacctggcgcctctctgaagctgagctgcgtgaccagcggcttcaccttcagaaagttcggcatgagctgggtgcgccagaccagcgacaagcggctggaatgggtggccagcatcagcaccggcggctacaacacctactacagcgacaacgtgaagggcagattcaccatcagcagagagaacgccaagaataccctgtacctgcagatgagcagcctgaagtccgaggacaccgccctgtactactgcaccagaggctacagcagcaccagctacgccatggactattggggccagggcaccaccgtgaccgtgtctagtaagcccaccaccacccctgcccctagacctccaaccccagcccctacaatcgccagccagcccctgagcctgaggcccgaagcctgtagacctgccgctggcggagccgtgcacaccagaggcctggatttcgcctgcgacatctacatctgggcccctctggccggcacctgtggcgtgctgctgctgagcctggtcatcaccctgtactgcaaccaccggaataagagaggccggaagaaactgctgtacatcttcaagcagcccttcatgcggcccgtgcagaccacccaggaagaggacggctgcagctgccggttccccgaggaagaggaaggcggctgcgaactgcgggtgaagttcagccggagcgccgacgcccctgcctaccagcagggccagaaccagctgtacaacgagctgaacctgggccggagggaggagtacgacgtgctggacaagcggagaggccgggaccctgagatgggcggcaagccccggagaaagaaccctcaggagggcctgtataacgaactgcagaaagacaagatggccgaggcctacagcgagatcggcatgaagggcgagcggcggaggggcaagggccacgacggcctgtaccagggcctgagcaccgccaccaaggatacctacgacgccctgcacatgcaggccctgccccccaga

SEQ ID NO: 121 - DNA, 1413 bp, synthetic construct
  misc_feature 1..1413: note = source = /note="Description of Artificial Sequence: Synthetic polynucleotide"
  misc_feature 1..1413: note = source = /note="EGFRvIII CAR (MR1-1 scFv.CD8alpha hinge &TM.4-1BB.CD3-zeta)"
  source 1..1413: mol_type = other DNA
gacatcgagctgacacagagccctgccagcctgtctgtggccaccggcgagaaagtgaccatccggtgcatgaccagcaccgacatcgacgacgacatgaactggtatcagcagaagcccggcgagccccccaagttcctgatcagcgagggcaacacactgcggcctggcgtgccaagcagattcagcagctctggcaccggcaccgacttcgtgttcaccatcgagaacaccctgagcgaggacgtgggcgactactactgcctgcagagctggaacgtgcccctgacctttggcgacggcaccaagctggaaatcaagggcggaggcggatctggcggcggaggatctgggggaggcggctctcaagtgaagctgcagcagtctggcggaggcctcgtgaaacctggcgcctctctgaagctgagctgcgtgaccagcggcttcaccttcagaaagttcggcatgagctgggtgcgccagaccagcgacaagcggctggaatgggtggccagcatcagcaccggcggctacaacacctactacagcgacaacgtgaagggcagattcaccatcagcagagagaacgccaagaataccctgtacctgcagatgagcagcctgaagtccgaggacaccgccctgtactactgcaccagaggctacagcccctacagctacgccatggactattggggccagggcaccaccgtgaccgtgtctagtaagcccaccaccacccctgcccctagacctccaaccccagcccctacaatcgccagccagcccctgagcctgaggcccgaagcctgtagacctgccgctggcggagccgtgcacaccagaggcctggatttcgcctgcgacatctacatctgggcccctctggccggcacctgtggcgtgctgctgctgagcctggtcatcaccctgtactgcaaccaccggaataagagaggccggaagaaactgctgtacatcttcaagcagcccttcatgcggcccgtgcagaccacccaggaagaggacggctgcagctgccggttccccgaggaagaggaaggcggctgcgaactgcgggtgaagttcagccggagcgccgacgcccctgcctaccagcagggccagaaccagctgtacaacgagctgaacctgggccggagggaggagtacgacgtgctggacaagcggagaggccgggaccctgagatgggcggcaagccccggagaaagaaccctcaggagggcctgtataacgaactgcagaaagacaagatggccgaggcctacagcgagatcggcatgaagggcgagcggcggaggggcaagggccacgacggcctgtaccagggcctgagcaccgccaccaaggatacctacgacgccctgcacatgcaggccctgccccccaga

SEQ ID NO: 122 - DNA, 1413 bp, synthetic construct
  misc_feature 1..1413: note = source = /note="Description of Artificial Sequence: Synthetic polynucleotide"
  misc_feature 1..1413: note = source = /note="EGFRvIII CAR (humMR1-1 scFv.CD8alpha hinge &TM.4-1BB.CD3-zeta)"
  source 1..1413: mol_type = other DNA
gacatccagatgacccagagccccagcagcctgtctgccagcgtgggcgacagagtgaccatcacctgtatgaccagcaccgacatcgacgacgacatgaactggtatcagcagaagcccggcaagacccccaagctgctgatctacgagggcaacaccctgaggcctggcgtgcccagcagattttctggcagcggctccggcaccgacttcatcttcaccatcagctccctgcagcccgaggatatcgccacctactactgcctgcagagctggaacgtgcccctgacctttggcggaggcaccaaggtggaaatcaagggcggaggcggatctggcggcggaggatctgggggaggcggctctcaggtgcagctgcaggaatctggcggagggctcgtgaagcctggcggaagcctgaagctgagctgtgccgccagcggcttcaccttcagcaagttcggcatgagctgggtgcgccagacccccgacaagagactggaatgggtggccagcatcagcaccggcggctacaatacctactacagcgacaacgtgaagggccggttcaccatctcccgggacaacgccaagaacaccctgtacctgcagatgagcagcctgaagtccgaggacaccgccatgtactactgtgccagaggctacagcccctacagctacgccatggattactggggccagggcacaatggtcaccgtgtcctctaagcccaccaccacccctgcccctagacctccaaccccagcccctacaatcgccagccagcccctgagcctgaggcccgaagcctgtagacctgccgctggcggagccgtgcacaccagaggcctggatttcgcctgcgacatctacatctgggcccctctggccggcacctgtggcgtgctgctgctgagcctggtcatcaccctgtactgcaaccaccggaataagagaggccggaagaaactgctgtacatcttcaagcagcccttcatgcggcccgtgcagaccacccaggaagaggacggctgcagctgccggttccccgaggaagaggaaggcggctgcgaactgcgggtgaagttcagccggagcgccgacgcccctgcctaccagcagggccagaaccagctgtacaacgagctgaacctgggccggagggaggagtacgacgtgctggacaagcggagaggccgggaccctgagatgggcggcaagccccggagaaagaaccctcaggagggcctgtataacgaactgcagaaagacaagatggccgaggcctacagcgagatcggcatgaagggcgagcggcggaggggcaagggccacgacggcctgtaccagggcctgagcaccgccaccaaggatacctacgacgccctgcacatgcaggccctgccccccaga

SEQ ID NO: 123 - DNA, 1413 bp, synthetic construct
  misc_feature 1..1413: note = source = /note="Description of Artificial Sequence: Synthetic polynucleotide"
  misc_feature 1..1413: note = source = /note="EGFRvIII CAR (humMR1-2 scFv.CD8alpha hinge &TM.4-1BB.CD3-zeta)"
  source 1..1413: mol_type = other DNA
gacatccagatgacccagagccccagcagcctgtctgccagcgtgggcgacagagtgaccatcacctgtatgaccagcaccgacatcgacgacgacatgaactggtatcagcagaagcccggcaagacccccaagctgctgatctacgagggcaacaccctgaggcctggcgtgcccagcagattttctggcagcggctccggcaccgacttcatcttcaccatcagctccctgcagcccgaggatatcgccacctactactgcctgcagagctggaacgtgcccctgacctttggcggaggcaccaaggtggaaatcaagggcggaggcggatctggcggcggaggatctgggggaggcggctctcaggtgcagctgcaggaatctggcggagggctcgtgaagcctggcggaagcctgaagctgagctgtgccgccagcggcttcaccttcagcaagttcggcatgagctgggtgcgccagacccccgacaagagactggaatgggtggccagcatcagcaccggcggctacaacaccttctacagcgacaacgtgaagggccggttcaccatctcccgggacaacgccaagaacaccctgtacctgcagatgagcagcctgaagtccgaggacaccgccatgtactactgtgccagaggctacagcccctacagcttcgccatggattactggggccagggcacaatggtcaccgtgtcctctaagcccaccaccacccctgcccctagacctccaaccccagcccctacaatcgccagccagcccctgagcctgaggcccgaagcctgtagacctgccgctggcggagccgtgcacaccagaggcctggatttcgcctgcgacatctacatctgggcccctctggccggcacctgtggcgtgctgctgctgagcctggtcatcaccctgtactgcaaccaccggaataagagaggccggaagaaactgctgtacatcttcaagcagcccttcatgcggcccgtgcagaccacccaggaagaggacggctgcagctgccggttccccgaggaagaggaaggcggctgcgaactgcgggtgaagttcagccggagcgccgacgcccctgcctaccagcagggccagaaccagctgtacaacgagctgaacctgggccggagggaggagtacgacgtgctggacaagcggagaggccgggaccctgagatgggcggcaagccccggagaaagaaccctcaggagggcctgtataacgaactgcagaaagacaagatggccgaggcctacagcgagatcggcatgaagggcgagcggcggaggggcaagggccacgacggcctgtaccagggcctgagcaccgccaccaaggatacctacgacgccctgcacatgcaggccctgccccccaga

SEQ ID NO: 124 - DNA, 1554 bp, synthetic construct
  misc_feature 1..1554: note = source = /note="Description of Artificial Sequence: Synthetic polynucleotide"
  misc_feature 1..1554: note = source = /note="EGFRvIII CAR (MR1-1 scFv.CD8alpha 2x hinge &TM.4-1BB.CD3-zeta)"
  source 1..1554: mol_type = other DNA
gacatcgagctgacacagagccctgccagcctgtctgtggccaccggcgagaaagtgaccatccggtgcatgaccagcaccgacatcgacgacgacatgaactggtatcagcagaagcccggcgagccccccaagttcctgatcagcgagggcaacacactgcggcctggcgtgccaagcagattcagcagctctggcaccggcaccgacttcgtgttcaccatcgagaacaccctgagcgaggacgtgggcgactactactgcctgcagagctggaacgtgcccctgacctttggcgacggcaccaagctggaaatcaagggcggaggcggatctggcggcggaggatctgggggaggcggctctcaagtgaagctgcagcagtctggcggaggcctcgtgaaacctggcgcctctctgaagctgagctgcgtgaccagcggcttcaccttcagaaagttcggcatgagctgggtgcgccagaccagcgacaagcggctggaatgggtggccagcatcagcaccggcggctacaacacctactacagcgacaacgtgaagggcagattcaccatcagcagagagaacgccaagaataccctgtacctgcagatgagcagcctgaagtccgaggacaccgccctgtactactgcaccagaggctacagcccctacagctacgccatggactattggggccagggcaccaccgtgaccgtgtctagtaaacctactacaactcctgccccccggcctcctacaccagctcctactatcgcctcccagccactcagtctcagacccgaggcttctaggccagcggccggaggcgcggtccacacccgcgggctggactttgcatccgataagcccaccaccacccctgcccctagacctccaaccccagcccctacaatcgccagccagcccctgagcctgaggcccgaagcctgtagacctgccgctggcggagccgtgcacaccagaggcctggatttcgcctgcgacatctacatctgggcccctctggccggcacctgtggcgtgctgctgctgagcctggtcatcaccctgtactgcaaccaccggaataagagaggccggaagaaactgctgtacatcttcaagcagcccttcatgcggcccgtgcagaccacccaggaagaggacggctgcagctgccggttccccgaggaagaggaaggcggctgcgaactgcgggtgaagttcagccggagcgccgacgcccctgcctaccagcagggccagaaccagctgtacaacgagctgaacctgggccggagggaggagtacgacgtgctggacaagcggagaggccgggaccctgagatgggcggcaagccccggagaaagaaccctcaggagggcctgtataacgaactgcagaaagacaagatggccgaggcctacagcgagatcggcatgaagggcgagcggcggaggggcaagggccacgacggcctgtaccagggcctgagcaccgccaccaaggatacctacgacgccctgcacatgcaggccctgccccccaga

SEQ ID NO: 125 - DNA, 1695 bp, synthetic construct
  misc_feature 1..1695: note = source = /note="Description of Artificial Sequence: Synthetic polynucleotide"
  misc_feature 1..1695: note = source = /note="EGFRvIII CAR (MR1-1 scFv.CD8alpha 3x hinge &TM.4-1BB.CD3-zeta)"
  source 1..1695: mol_type = other DNA
gacatcgagctgacacagagccctgccagcctgtctgtggccaccggcgagaaagtgaccatccggtgcatgaccagcaccgacatcgacgacgacatgaactggtatcagcagaagcccggcgagccccccaagttcctgatcagcgagggcaacacactgcggcctggcgtgccaagcagattcagcagctctggcaccggcaccgacttcgtgttcaccatcgagaacaccctgagcgaggacgtgggcgactactactgcctgcagagctggaacgtgcccctgacctttggcgacggcaccaagctggaaatcaagggcggaggcggatctggcggcggaggatctgggggaggcggctctcaagtgaagctgcagcagtctggcggaggcctcgtgaaacctggcgcctctctgaagctgagctgcgtgaccagcggcttcaccttcagaaagttcggcatgagctgggtgcgccagaccagcgacaagcggctggaatgggtggccagcatcagcaccggcggctacaacacctactacagcgacaacgtgaagggcagattcaccatcagcagagagaacgccaagaataccctgtacctgcagatgagcagcctgaagtccgaggacaccgccctgtactactgcaccagaggctacagcccctacagctacgccatggactattggggccagggcaccaccgtgaccgtgtctagtaagcctaccaccacccccgcacctcgtcctccaacccctgcacctacgattgccagtcagcctctttcactgcggcctgaggccagcagaccagctgccggcggtgccgtccatacaagaggactggacttcgcgtccgataaacctactaccactccagccccaaggcccccaaccccagcaccgactatcgcatcacagcctttgtcactgcgtcctgaagccagccggccagctgcagggggggccgtccacacaaggggactcgactttgcgagtgataagcccaccaccacccctgcccctagacctccaaccccagcccctacaatcgccagccagcccctgagcctgaggcccgaagcctgtagacctgccgctggcggagccgtgcacaccagaggcctggatttcgcctgcgacatctacatctgggcccctctggccggcacctgtggcgtgctgctgctgagcctggtcatcaccctgtactgcaaccaccggaataagagaggccggaagaaactgctgtacatcttcaagcagcccttcatgcggcccgtgcagaccacccaggaagaggacggctgcagctgccggttccccgaggaagaggaaggcggctgcgaactgcgggtgaagttcagccggagcgccgacgcccctgcctaccagcagggccagaaccagctgtacaacgagctgaacctgggccggagggaggagtacgacgtgctggacaagcggagaggccgggaccctgagatgggcggcaagccccggagaaagaaccctcaggagggcctgtataacgaactgcagaaagacaagatggccgaggcctacagcgagatcggcatgaagggcgagcggcggaggggcaagggccacgacggcctgtaccagggcctgagcaccgccaccaaggatacctacgacgccctgcacatgcaggccctgccccccaga

SEQ ID NO: 126 - DNA, 1836 bp, synthetic construct
  misc_feature 1..1836: note = source = /note="Description of Artificial Sequence: Synthetic polynucleotide"
  misc_feature 1..1836: note = source = /note="EGFRvIII CAR (MR1-1 scFv.CD8alpha 4x hinge &TM.4-1BB.CD3-zeta)"
  source 1..1836: mol_type = other DNA
gacatcgagctgacacagagccctgccagcctgtctgtggccaccggcgagaaagtgaccatccggtgcatgaccagcaccgacatcgacgacgacatgaactggtatcagcagaagcccggcgagccccccaagttcctgatcagcgagggcaacacactgcggcctggcgtgccaagcagattcagcagctctggcaccggcaccgacttcgtgttcaccatcgagaacaccctgagcgaggacgtgggcgactactactgcctgcagagctggaacgtgcccctgacctttggcgacggcaccaagctggaaatcaagggcggaggcggatctggcggcggaggatctgggggaggcggctctcaagtgaagctgcagcagtctggcggaggcctcgtgaaacctggcgcctctctgaagctgagctgcgtgaccagcggcttcaccttcagaaagttcggcatgagctgggtgcgccagaccagcgacaagcggctggaatgggtggccagcatcagcaccggcggctacaacacctactacagcgacaacgtgaagggcagattcaccatcagcagagagaacgccaagaataccctgtacctgcagatgagcagcctgaagtccgaggacaccgccctgtactactgcaccagaggctacagcccctacagctacgccatggactattggggccagggcaccaccgtgaccgtgtctagtaagcctaccaccacccccgcacctcgtcctccaacccctgcacctacgattgccagtcagcctctttcactgcggcctgaggccagcagaccagctgccggcggtgccgtccatacaagaggactggacttcgcgtccgataaacctactaccactccagccccaaggcccccaaccccagcaccgactatcgcatcacagcctttgtcactgcgtcctgaagccagccggccagctgcagggggggccgtccacacaaggggactcgactttgcgagtgataaacctactacaactcctgccccccggcctcctacaccagctcctactatcgcctcccagccactcagtctcagacccgaggcttctaggccagcggccggaggcgcggtccacacccgcgggctggactttgcatccgataagcccaccaccacccctgcccctagacctccaaccccagcccctacaatcgccagccagcccctgagcctgaggcccgaagcctgtagacctgccgctggcggagccgtgcacaccagaggcctggatttcgcctgcgacatctacatctgggcccctctggccggcacctgtggcgtgctgctgctgagcctggtcatcaccctgtactgcaaccaccggaataagagaggccggaagaaactgctgtacatcttcaagcagcccttcatgcggcccgtgcagaccacccaggaagaggacggctgcagctgccggttccccgaggaagaggaaggcggctgcgaactgcgggtgaagttcagccggagcgccgacgcccctgcctaccagcagggccagaaccagctgtacaacgagctgaacctgggccggagggaggagtacgacgtgctggacaagcggagaggccgggaccctgagatgggcggcaagccccggagaaagaaccctcaggagggcctgtataacgaactgcagaaagacaagatggccgaggcctacagcgagatcggcatgaagggcgagcggcggaggggcaagggccacgacggcctgtaccagggcctgagcaccgccaccaaggatacctacgacgccctgcacatgcaggccctgccccccaga

SEQ ID NO: 127 - DNA, 1695 bp, synthetic construct
  misc_feature 1..1695: note = source = /note="Description of Artificial Sequence: Synthetic polynucleotide"
  misc_feature 1..1695: note = source = /note="EGFRvIII CAR (huMR1-1 scFv.CD8alpha 3x hinge & TM.4-1BB.CD3-zeta)"
  source 1..1695: mol_type = other DNA
gacatccagatgacccagagccccagcagcctgtctgccagcgtgggcgacagagtgaccatcacctgtatgaccagcaccgacatcgacgacgacatgaactggtatcagcagaagcccggcaagacccccaagctgctgatctacgagggcaacaccctgaggcctggcgtgcccagcagattttctggcagcggctccggcaccgacttcatcttcaccatcagctccctgcagcccgaggatatcgccacctactactgcctgcagagctggaacgtgcccctgacctttggcggaggcaccaaggtggaaatcaagggcggaggcggatctggcggcggaggatctgggggaggcggctctcaggtgcagctgcaggaatctggcggagggctcgtgaagcctggcggaagcctgaagctgagctgtgccgccagcggcttcaccttcagcaagttcggcatgagctgggtgcgccagacccccgacaagagactggaatgggtggccagcatcagcaccggcggctacaatacctactacagcgacaacgtgaagggccggttcaccatctcccgggacaacgccaagaacaccctgtacctgcagatgagcagcctgaagtccgaggacaccgccatgtactactgtgccagaggctacagcccctacagctacgccatggattactggggccagggcacaatggtcaccgtgtcctctaagcctaccaccacccccgcacctcgtcctccaacccctgcacctacgattgccagtcagcctctttcactgcggcctgaggccagcagaccagctgccggcggtgccgtccatacaagaggactggacttcgcgtccgataaacctactaccactccagccccaaggcccccaaccccagcaccgactatcgcatcacagcctttgtcactgcgtcctgaagccagccggccagctgcagggggggccgtccacacaaggggactcgactttgcgagtgataagcccaccaccacccctgcccctagacctccaaccccagcccctacaatcgccagccagcccctgagcctgaggcccgaagcctgtagacctgccgctggcggagccgtgcacaccagaggcctggatttcgcctgcgacatctacatctgggcccctctggccggcacctgtggcgtgctgctgctgagcctggtcatcaccctgtactgcaaccaccggaataagagaggccggaagaaactgctgtacatcttcaagcagcccttcatgcggcccgtgcagaccacccaggaagaggacggctgcagctgccggttccccgaggaagaggaaggcggctgcgaactgcgggtgaagttcagccggagcgccgacgcccctgcctaccagcagggccagaaccagctgtacaacgagctgaacctgggccggagggaggagtacgacgtgctggacaagcggagaggccgggaccctgagatgggcggcaagccccggagaaagaaccctcaggagggcctgtataacgaactgcagaaagacaagatggccgaggcctacagcgagatcggcatgaagggcgagcggcggaggggcaagggccacgacggcctgtaccagggcctgagcaccgccaccaaggatacctacgacgccctgcacatgcaggccctgccccccaga

SEQ ID NO: 128 - DNA, 1836 bp, synthetic construct
  misc_feature 1..1836: note = source = /note="Description of Artificial Sequence: Synthetic polynucleotide"
  misc_feature 1..1836: note = source = /note="EGFRvIII CAR (huMR1-1 scFv.CD8alpha 4x hinge & TM.4-1BB.CD3-zeta)"
  source 1..1836: mol_type = other DNA
gacatccagatgacccagagccccagcagcctgtctgccagcgtgggcgacagagtgaccatcacctgtatgaccagcaccgacatcgacgacgacatgaactggtatcagcagaagcccggcaagacccccaagctgctgatctacgagggcaacaccctgaggcctggcgtgcccagcagattttctggcagcggctccggcaccgacttcatcttcaccatcagctccctgcagcccgaggatatcgccacctactactgcctgcagagctggaacgtgcccctgacctttggcggaggcaccaaggtggaaatcaagggcggaggcggatctggcggcggaggatctgggggaggcggctctcaggtgcagctgcaggaatctggcggagggctcgtgaagcctggcggaagcctgaagctgagctgtgccgccagcggcttcaccttcagcaagttcggcatgagctgggtgcgccagacccccgacaagagactggaatgggtggccagcatcagcaccggcggctacaatacctactacagcgacaacgtgaagggccggttcaccatctcccgggacaacgccaagaacaccctgtacctgcagatgagcagcctgaagtccgaggacaccgccatgtactactgtgccagaggctacagcccctacagctacgccatggattactggggccagggcacaatggtcaccgtgtcctctaagcctaccaccacccccgcacctcgtcctccaacccctgcacctacgattgccagtcagcctctttcactgcggcctgaggccagcagaccagctgccggcggtgccgtccatacaagaggactggacttcgcgtccgataaacctactaccactccagccccaaggcccccaaccccagcaccgactatcgcatcacagcctttgtcactgcgtcctgaagccagccggccagctgcagggggggccgtccacacaaggggactcgactttgcgagtgataaacctactacaactcctgccccccggcctcctacaccagctcctactatcgcctcccagccactcagtctcagacccgaggcttctaggccagcggccggaggcgcggtccacacccgcgggctggactttgcatccgataagcccaccaccacccctgcccctagacctccaaccccagcccctacaatcgccagccagcccctgagcctgaggcccgaagcctgtagacctgccgctggcggagccgtgcacaccagaggcctggatttcgcctgcgacatctacatctgggcccctctggccggcacctgtggcgtgctgctgctgagcctggtcatcaccctgtactgcaaccaccggaataagagaggccggaagaaactgctgtacatcttcaagcagcccttcatgcggcccgtgcagaccacccaggaagaggacggctgcagctgccggttccccgaggaagaggaaggcggctgcgaactgcgggtgaagttcagccggagcgccgacgcccctgcctaccagcagggccagaaccagctgtacaacgagctgaacctgggccggagggaggagtacgacgtgctggacaagcggagaggccgggaccctgagatgggcggcaagccccggagaaagaaccctcaggagggcctgtataacgaactgcagaaagacaagatggccgaggcctacagcgagatcggcatgaagggcgagcggcggaggggcaagggccacgacggcctgtaccagggcctgagcaccgccaccaaggatacctacgacgccctgcacatgcaggccctgccccccaga

SEQ ID NO: 129 - DNA, 1695 bp, synthetic construct
  misc_feature 1..1695: note = source = /note="Description of Artificial Sequence: Synthetic polynucleotide"
  misc_feature 1..1695: note = source = /note="EGFRvIII CAR (huMR1-2 scFv.CD8alpha 3x hinge & TM.4-1BB.CD3-zeta)"
  source 1..1695: mol_type = other DNA
gacatccagatgacccagagccccagcagcctgtctgccagcgtgggcgacagagtgaccatcacctgtatgaccagcaccgacatcgacgacgacatgaactggtatcagcagaagcccggcaagacccccaagctgctgatctacgagggcaacaccctgaggcctggcgtgcccagcagattttctggcagcggctccggcaccgacttcatcttcaccatcagctccctgcagcccgaggatatcgccacctactactgcctgcagagctggaacgtgcccctgacctttggcggaggcaccaaggtggaaatcaagggcggaggcggatctggcggcggaggatctgggggaggcggctctcaggtgcagctgcaggaatctggcggagggctcgtgaagcctggcggaagcctgaagctgagctgtgccgccagcggcttcaccttcagcaagttcggcatgagctgggtgcgccagacccccgacaagagactggaatgggtggccagcatcagcaccggcggctacaacaccttctacagcgacaacgtgaagggccggttcaccatctcccgggacaacgccaagaacaccctgtacctgcagatgagcagcctgaagtccgaggacaccgccatgtactactgtgccagaggctacagcccctacagcttcgccatggattactggggccagggcacaatggtcaccgtgtcctctaagcctaccaccacccccgcacctcgtcctccaacccctgcacctacgattgccagtcagcctctttcactgcggcctgaggccagcagaccagctgccggcggtgccgtccatacaagaggactggacttcgcgtccgataaacctactaccactccagccccaaggcccccaaccccagcaccgactatcgcatcacagcctttgtcactgcgtcctgaagccagccggccagctgcagggggggccgtccacacaaggggactcgactttgcgagtgataagcccaccaccacccctgcccctagacctccaaccccagcccctacaatcgccagccagcccctgagcctgaggcccgaagcctgtagacctgccgctggcggagccgtgcacaccagaggcctggatttcgcctgcgacatctacatctgggcccctctggccggcacctgtggcgtgctgctgctgagcctggtcatcaccctgtactgcaaccaccggaataagagaggccggaagaaactgctgtacatcttcaagcagcccttcatgcggcccgtgcagaccacccaggaagaggacggctgcagctgccggttccccgaggaagaggaaggcggctgcgaactgcgggtgaagttcagccggagcgccgacgcccctgcctaccagcagggccagaaccagctgtacaacgagctgaacctgggccggagggaggagtacgacgtgctggacaagcggagaggccgggaccctgagatgggcggcaagccccggagaaagaaccctcaggagggcctgtataacgaactgcagaaagacaagatggccgaggcctacagcgagatcggcatgaagggcgagcggcggaggggcaagggccacgacggcctgtaccagggcctgagcaccgccaccaaggatacctacgacgccctgcacatgcaggccctgccccccaga

SEQ ID NO: 130 - DNA, 1836 bp, synthetic construct
  misc_feature 1..1836: note = source = /note="Description of Artificial Sequence: Synthetic polynucleotide"
  misc_feature 1..1836: note = source = /note="EGFRvIII CAR (huMR1-2 scFv.CD8alpha 4x hinge & TM.4-1BB.CD3-zeta"
  source 1..1836: mol_type = other DNA
gacatccagatgacccagagccccagcagcctgtctgccagcgtgggcgacagagtgaccatcacctgtatgaccagcaccgacatcgacgacgacatgaactggtatcagcagaagcccggcaagacccccaagctgctgatctacgagggcaacaccctgaggcctggcgtgcccagcagattttctggcagcggctccggcaccgacttcatcttcaccatcagctccctgcagcccgaggatatcgccacctactactgcctgcagagctggaacgtgcccctgacctttggcggaggcaccaaggtggaaatcaagggcggaggcggatctggcggcggaggatctgggggaggcggctctcaggtgcagctgcaggaatctggcggagggctcgtgaagcctggcggaagcctgaagctgagctgtgccgccagcggcttcaccttcagcaagttcggcatgagctgggtgcgccagacccccgacaagagactggaatgggtggccagcatcagcaccggcggctacaacaccttctacagcgacaacgtgaagggccggttcaccatctcccgggacaacgccaagaacaccctgtacctgcagatgagcagcctgaagtccgaggacaccgccatgtactactgtgccagaggctacagcccctacagcttcgccatggattactggggccagggcacaatggtcaccgtgtcctctaagcctaccaccacccccgcacctcgtcctccaacccctgcacctacgattgccagtcagcctctttcactgcggcctgaggccagcagaccagctgccggcggtgccgtccatacaagaggactggacttcgcgtccgataaacctactaccactccagccccaaggcccccaaccccagcaccgactatcgcatcacagcctttgtcactgcgtcctgaagccagccggccagctgcagggggggccgtccacacaaggggactcgactttgcgagtgataaacctactacaactcctgccccccggcctcctacaccagctcctactatcgcctcccagccactcagtctcagacccgaggcttctaggccagcggccggaggcgcggtccacacccgcgggctggactttgcatccgataagcccaccaccacccctgcccctagacctccaaccccagcccctacaatcgccagccagcccctgagcctgaggcccgaagcctgtagacctgccgctggcggagccgtgcacaccagaggcctggatttcgcctgcgacatctacatctgggcccctctggccggcacctgtggcgtgctgctgctgagcctggtcatcaccctgtactgcaaccaccggaataagagaggccggaagaaactgctgtacatcttcaagcagcccttcatgcggcccgtgcagaccacccaggaagaggacggctgcagctgccggttccccgaggaagaggaaggcggctgcgaactgcgggtgaagttcagccggagcgccgacgcccctgcctaccagcagggccagaaccagctgtacaacgagctgaacctgggccggagggaggagtacgacgtgctggacaagcggagaggccgggaccctgagatgggcggcaagccccggagaaagaaccctcaggagggcctgtataacgaactgcagaaagacaagatggccgaggcctacagcgagatcggcatgaagggcgagcggcggaggggcaagggccacgacggcctgtaccagggcctgagcaccgccaccaaggatacctacgacgccctgcacatgcaggccctgccccccaga

SEQ ID NO: 131 - DNA, 3224 bp, synthetic construct
  misc_feature 1..3224: note = source = /note="Description of Artificial Sequence: Synthetic polynucleotide"
  misc_feature 1..3224: note = source = /note="XON-64"
  source 1..3224: mol_type = other DNA
gtggaatgtgtgtcagttagggtgtggaaagtccccaggctccccagcaggcagaagtatgcaaagcatcgagcggccgcaataaaatatctttattttcattacatctgtgtgttggttttttgtgtgaatcgtaactaacatacgctctccatcaaaacaaaacgaaacaaaacaaactagcaaaataggctgtccccagtgcaagtgcaggtgccagaacatttctctatcgaaggatctgcgatcgctccggtgcccgtcagtgggcagagcgcacatcgcccacagtccccgagaagttggggggaggggtcggcaattgaaccggtgcctagagaaggtggcgcggggtaaactgggaaagtgatgtcgtgtactggctccgcctttttcccgagggtgggggagaaccgtatataagtgcagtagtcgccgtgaacgttctttttcgcaacgggtttgccgccagaacacagctgaagcttcgaggggctcgcatctctccttcacgcgcccgccgccctacctgaggccgccatccacgccggttgagtcgcgttctgccgcctcccgcctgtggtgcctcctgaactgcgtccgccgtctaggtaagtttaaagctcaggtcgagaccgggcctttgtccggcgctcccttggagcctacctagactcagccggctctccacgctttgcctgaccctgcttgctcaactctacgtctttgtttcgttttctgttctgcgccgttacagatccaagctgtgaccggcgcctacctgagatcaccggcgaaggaggcctatcatgaagatctatcgattgtacagctagccgccaccatgctgctgctggtgaccagcctgctgctgtgtgagctgccccaccccgcctttctgctgatccccgacatccagatgacccagagccccagcagcctgtctgccagcgtgggcgacagagtgaccatcacctgtatgaccagcaccgacatcgacgacgacatgaactggtatcagcagaagcccggcaagacccccaagctgctgatctacgagggcaacaccctgaggcctggcgtgcccagcagattttctggcagcggctccggcaccgacttcatcttcaccatcagctccctgcagcccgaggatatcgccacctactactgcctgcagagctggaacgtgcccctgacctttggcggaggcaccaaggtggaaatcaagggcggaggcggatctggcggcggaggatctgggggaggcggctctcaggtgcagctgcaggaatctggcggagggctcgtgaagcctggcggaagcctgaagctgagctgtgccgccagcggcttcaccttcagcaagttcggcatgagctgggtgcgccagacccccgacaagagactggaatgggtggccagcatcagcaccggcggctacaatacctactacagcgacaacgtgaagggccggttcaccatctcccgggacaacgccaagaacaccctgtacctgcagatgagcagcctgaagtccgaggacaccgccatgtactactgtgccagaggctacagcccctacagctacgccatggattactggggccagggcacaatggtcaccgtgtcctctaagcctaccaccacccccgcacctcgtcctccaacccctgcacctacgattgccagtcagcctctttcactgcggcctgaggccagcagaccagctgccggcggtgccgtccatacaagaggactggacttcgcgtccgataaacctactaccactccagccccaaggcccccaaccccagcaccgactatcgcatcacagcctttgtcactgcgtcctgaagccagccggccagctgcagggggggccgtccacacaaggggactcgactttgcgagtgataagcccaccaccacccctgcccctagacctccaaccccagcccctacaatcgccagccagcccctgagcctgaggcccgaagcctgtagacctgccgctggcggagccgtgcacaccagaggcctggatttcgcctgcgacatctacatctgggcccctctggccggcacctgtggcgtgctgctgctgagcctggtcatcaccctgtactgcaaccaccggaataagagaggccggaagaaactgctgtacatcttcaagcagcccttcatgcggcccgtgcagaccacccaggaagaggacggctgcagctgccggttccccgaggaagaggaaggcggctgcgaactgcgggtgaagttcagccggagcgccgacgcccctgcctaccagcagggccagaaccagctgtacaacgagctgaacctgggccggagggaggagtacgacgtgctggacaagcggagaggccgggaccctgagatgggcggcaagccccggagaaagaaccctcaggagggcctgtataacgaactgcagaaagacaagatggccgaggcctacagcgagatcggcatgaagggcgagcggcggaggggcaagggccacgacggcctgtaccagggcctgagcaccgccaccaaggatacctacgacgccctgcacatgcaggccctgccccccagatgagatatcactagtctcgagtcgatcatgctcatagtggcaagagagagccgtacgtgatcagcgggatctgctgtgccttctagttgccagccatctgttgtttgcccctcccccgtgccttccttgaccctggaaggtgccactcccactgtcctttcctaataaaatgaggaaattgcatcgcattgtctgagtaggtgtcattctattctggggggtggggtggggcaggacagcaagggggaggattgggaagacaatagcaggcatgctggggatgcggtgggctctatgggtacccaggtgctgaagaattgacccggttcctcctgggccagaaagaagcaggcacatccccttctctgtgacacaccctgtccacgcccctggttcttagttccagccccactcataggacactcatagctcaggagggctccgccttcaatcccacccgctaaagtacttggagcggtctctccctccctcatcagcccaccaaaccaaacctagcctccaagagtgggaagaaattaaagcaagataggctattaagtgcagagggagagaaaatgcctccaacatgtgaggaagtaatgagagaaatcatagaatt

SEQ ID NO: 132 - DNA, 3319 bp, synthetic construct
  misc_feature 1..3319: note = source = /note="Description of Artificial Sequence: Synthetic polynucleotide"
  misc_feature 1..3319: note = source = /note="XON-30"
  source 1..3319: mol_type = other DNA
gtggaatgtgtgtcagttagggtgtggaaagtccccaggctccccagcaggcagaagtatgcaaagcatcgagcggccgcaataaaatatctttattttcattacatctgtgtgttggttttttgtgtgaatcgtaactaacatacgctctccatcaaaacaaaacgaaacaaaacaaactagcaaaataggctgtccccagtgcaagtgcaggtgccagaacatttctctatcgaaggatctgcgatcgctccggtgcccgtcagtgggcagagcgcacatcgcccacagtccccgagaagttggggggaggggtcggcaattgaaccggtgcctagagaaggtggcgcggggtaaactgggaaagtgatgtcgtgtactggctccgcctttttcccgagggtgggggagaaccgtatataagtgcagtagtcgccgtgaacgttctttttcgcaacgggtttgccgccagaacacagctgaagcttcgaggggctcgcatctctccttcacgcgcccgccgccctacctgaggccgccatccacgccggttgagtcgcgttctgccgcctcccgcctgtggtgcctcctgaactgcgtccgccgtctaggtaagtttaaagctcaggtcgagaccgggcctttgtccggcgctcccttggagcctacctagactcagccggctctccacgctttgcctgaccctgcttgctcaactctacgtctttgtttcgttttctgttctgcgccgttacagatccaagctgtgaccggcgcctacctgagatcaccggcgaaggaggcctatcatgaagatctatcgattgtacagctagccgccaccatgctgctgctggtgaccagcctgctgctgtgtgagctgccccaccccgcctttctgctgatccccgacatccagatgacccagagccccagcagcctgtctgccagcgtgggcgacagagtgaccatcacctgtatgaccagcaccgacatcgacgacgacatgaactggtatcagcagaagcccggcaagacccccaagctgctgatctacgagggcaacaccctgaggcctggcgtgcccagcagattttctggcagcggctccggcaccgacttcatcttcaccatcagctccctgcagcccgaggatatcgccacctactactgcctgcagagctggaacgtgcccctgacctttggcggaggcaccaaggtggaaatcaagggcggaggcggatctggcggcggaggatctgggggaggcggctctcaggtgcagctgcaggaatctggcggagggctcgtgaagcctggcggaagcctgaagctgagctgtgccgccagcggcttcaccttcagcaagttcggcatgagctgggtgcgccagacccccgacaagagactggaatgggtggccagcatcagcaccggcggctacaatacctactacagcgacaacgtgaagggccggttcaccatctcccgggacaacgccaagaacaccctgtacctgcagatgagcagcctgaagtccgaggacaccgccatgtactactgtgccagaggctacagcccctacagctacgccatggattactggggccagggcacaatggtcaccgtgtcctctaagcctaccaccacccccgcacctcgtcctccaacccctgcacctacgattgccagtcagcctctttcactgcggcctgaggccagcagaccagctgccggcggtgccgtccatacaagaggactggacttcgcgtccgataaacctactaccactccagccccaaggcccccaaccccagcaccgactatcgcatcacagcctttgtcactgcgtcctgaagccagccggccagctgcagggggggccgtccacacaaggggactcgactttgcgagtgataagcccaccaccacccctgcccctagacctccaaccccagcccctacaatcgccagccagcccctgagcctgaggcccgaagcctgtagacctgccgctggcggagccgtgcacaccagaggcctggatttcgcctgcgacatctacatctgggcccctctggccggcacctgtggcgtgctgctgctgagcctggtcatcaccctgtactgcaaccaccggaataagagaggccggaagaaactgctgtacatcttcaagcagcccttcatgcggcccgtgcagaccacccaggaagaggacggctgcagctgccggttccccgaggaagaggaaggcggctgcgaactgcgggtgaagttcagccggagcgccgacgcccctgcctaccagcagggccagaaccagctgtacaacgagctgaacctgggccggagggaggagtacgacgtgctggacaagcggagaggccgggaccctgagatgggcggcaagccccggagaaagaaccctcaggagggcctgtataacgaactgcagaaagacaagatggccgaggcctacagcgagatcggcatgaagggcgagcggcggaggggcaagggccacgacggcctgtaccagggcctgagcaccgccaccaaggatacctacgacgccctgcacatgcaggccctgccccccagaagggccaagaggagtggcagcggcgagggcagaggaagtcttctaacatgcggtgacgtggaggagaatcccggccctatgaggctccctgctcagctcctggggctgctaatgctctgggtcccaggatccagtgggcgcaaagtgtgtaacggaataggtattggtgaatttaaagactcactctccataaatgctacgaatattaaacacttcaaaaactgcacctccatcagtggcgatctccacatcctgccggtggcatttaggggtgactccttcacacatactcctcctctggatccacaggaactggatattctgaaaaccgtaaaggaaatcacagggtttttgctgattcaggcttggcctgaaaacaggacggacctccatgcctttgagaacctagaaatcatacgcggcaggaccaagcaacatggtcagttttctcttgcagtcgtcagcctgaacataacatccttgggattacgctccctcaaggagataagtgatggagatgtgataatttcaggaaacaaaaatttgtgctatgcaaatacaataaactggaaaaaactgtttgggacctccggtcagaaaaccaaaattataagcaacagaggtgaaaacagctgcaaggccacaggccaggtctgccatgccttgtgctcccccgagggctgctggggcccggagcccagggactgcgtctct

SEQ ID NO: 133 - DNA, 4763 bp, synthetic construct
  misc_feature 1..4763: note = source = /note="Description of Artificial Sequence: Synthetic polynucleotide"
  misc_feature 1..4763: note = source = /note="XON-59"
  source 1..4763: mol_type = other DNA
gagcgtgcgtgaggctccggtgcccgtcagtgggcagagcgcacatcgcccacagtccccgagaagttggggggagggggtcggcgattgaaccggtgcctagagaaggtggcgcggggtaaactgggaaagtgatgtcgtgtactggctccgcctttttcccgagggtgggggagaaccgtatataagtgcagtagtcgccgtgaacgttctttttcgcaacgggtttgccgccagaacacagcagccgctaaatccaaggtaaggtcagaagagctagcgccaccatgctgctgctggtgaccagcctgctgctgtgtgagctgccccaccccgcctttctgctgatccccgacatccagatgacccagagccccagcagcctgtctgccagcgtgggcgacagagtgaccatcacctgtatgaccagcaccgacatcgacgacgacatgaactggtatcagcagaagcccggcaagacccccaagctgctgatctacgagggcaacaccctgaggcctggcgtgcccagcagattttctggcagcggctccggcaccgacttcatcttcaccatcagctccctgcagcccgaggatatcgccacctactactgcctgcagagctggaacgtgcccctgacctttggcggaggcaccaaggtggaaatcaagggcggaggcggatctggcggcggaggatctgggggaggcggctctcaggtgcagctgcaggaatctggcggagggctcgtgaagcctggcggaagcctgaagctgagctgtgccgccagcggcttcaccttcagcaagttcggcatgagctgggtgcgccagacccccgacaagagactggaatgggtggccagcatcagcaccggcggctacaatacctactacagcgacaacgtgaagggccggttcaccatctcccgggacaacgccaagaacaccctgtacctgcagatgagcagcctgaagtccgaggacaccgccatgtactactgtgccagaggctacagcccctacagctacgccatggattactggggccagggcacaatggtcaccgtgtcctctaagcctaccaccacccccgcacctcgtcctccaacccctgcacctacgattgccagtcagcctctttcactgcggcctgaggccagcagaccagctgccggcggtgccgtccatacaagaggactggacttcgcgtccgataaacctactaccactccagccccaaggcccccaaccccagcaccgactatcgcatcacagcctttgtcactgcgtcctgaagccagccggccagctgcagggggggccgtccacacaaggggactcgactttgcgagtgataagcccaccaccacccctgcccctagacctccaaccccagcccctacaatcgccagccagcccctgagcctgaggcccgaagcctgtagacctgccgctggcggagccgtgcacaccagaggcctggatttcgcctgcgacatctacatctgggcccctctggccggcacctgtggcgtgctgctgctgagcctggtcatcaccctgtactgcaaccaccggaataagagaggccggaagaaactgctgtacatcttcaagcagcccttcatgcggcccgtgcagaccacccaggaagaggacggctgcagctgccggttccccgaggaagaggaaggcggctgcgaactgcgggtgaagttcagccggagcgccgacgcccctgcctaccagcagggccagaaccagctgtacaacgagctgaacctgggccggagggaggagtacgacgtgctggacaagcggagaggccgggaccctgagatgggcggcaagccccggagaaagaaccctcaggagggcctgtataacgaactgcagaaagacaagatggccgaggcctacagcgagatcggcatgaagggcgagcggcggaggggcaagggccacgacggcctgtaccagggcctgagcaccgccaccaaggatacctacgacgccctgcacatgcaggccctgccccccagaagagctaagaggggaagcggagagggcagaggaagtctgctaacatgcggtgacgtcgaggagaatcctggacctggccccaagaagaaaaggaaggtggccccccccaccgacgtgagcctgggcgacgagctgcacctggacggcgaggacgtggccatggcccacgccgacgccctggacgacttcgacctggacatgctgggcgacggcgacagccccggccccggcttcaccccccacgacagcgccccctacggcgccctggacatggccgacttcgagttcgagcagatgttcaccgacgccctgggcatcgacgagtacggcggcgaattcgagatgcccgtggacaggattctggaggccgaactcgccgtggagcagaaaagcgaccagggcgtggagggccccggcggaaccggcggcagcggcagcagccccaacgaccccgtgaccaacatctgccaggccgccgacaagcagctgttcaccctggtggagtgggccaagaggattccccacttcagcagcctgcccctggacgaccaggtgatcctgctgagggccggatggaacgagctgctgatcgccagcttcagccacaggagcatcgacgtgagggacggcatcctgctggccaccggcctgcacgtccataggaacagcgcccacagcgccggagtgggcgccatcttcgacagggtgctgaccgagctggtgagcaagatgagggacatgaggatggacaagaccgagctgggctgcctgagggccatcatcctgttcaaccccgaggtgaggggcctgaaaagcgcccaggaggtggagctgctgagggagaaggtgtacgccgccctggaggagtacaccaggaccacccaccccgacgagcccggcagattcgccaagctgctgctgaggctgcccagcctgaggagcatcggcctgaagtgcctggagcacctgttcttcttcaggctgatcggcgacgtgcccatcgacaccttcctgatggagatgctggagagccccagcgacagcagagctaagaggggaagcggagagggcagaggaagtctgctaacatgcggtgacgtcgaggagaatcctggacctaagctgctgagcagcatcgagcaggcttgcgacatctgcaggctgaagaagctgaagtgcagcaaggagaagcccaagtgcgccaagtgcctgaagaacaactgggagtgcagatacagccccaagaccaagaggagccccctgaccagggcccacctgaccgaggtggagagcaggctggagaggctggagcagctgttcctgctgatcttccccagggaggacctggacatgatcctgaagatggacagcctgcaagacatcaaggccctgctgaccggcctgttcgtgcaggacaacgtgaacaaggacgccgtgaccgacaggctggccagcgtggagaccgacatgcccctgaccctgaggcagcacaggatcagcgccaccagcagcagcgaggagagcagcaacaagggccagaggcagctgaccgtgagccccgagtttcccgggatcaggcccgagtgcgtggtgcccgagacccagtgcgccatgaaaaggaaggagaagaaggcccagaaggagaaggacaagctgcccgtgagcaccaccaccgtcgatgaccacatgccccccatcatgcagtgcgagccccccccccccgaggccgccaggattcacgaggtcgtgcccaggttcctgagcgacaagctgctggtgaccaacaggcagaagaacatcccccagctgaccgccaaccagcagttcctgatcgccaggctgatctggtatcaggacggctacgagcagcccagcgacgaggacctgaaaaggatcacccagacctggcagcaggccgacgacgagaacgaggagagcgacacccccttcaggcagatcaccgagatgaccatcctgaccgtgcagctgatcgtggagttcgccaagggcctgcccggattcgccaagatcagccagcccgaccagatcaccctgctgaaggcttgcagcagcgaggtgatgatgctgagggtggccaggaggtacgacgccgccagcgacagcatcctgttcgccaacaaccaggcttacaccagggacaactacaggaaggctggcatggccgaggtgatcgaggacctcctgcacttctgcagatgtatgtacagcatggccctggacaacatccactacgccctgctgaccgccgtggtgatcttcagcgacaggcccggcctggagcagccccagctggtggaggagatccagaggtactacctgaacaccctgaggatctacatcctgaaccagctgagcggcagcgccaggagcagcgtgatctacggcaagatcctgagcatcctgagcgagctgaggaccctgggaatgcagaacagcaatatgtgtatcagcctgaagctgaagaacaggaagctgccccccttcctggaggagatttgggacgtggccgacatgagccacacccagcccccccccatcctggagagccccaccaacctgtgaaacttgtttattgcagcttataatggttacaaataaagcaatagcatcacaaatttcacaaataaagcatttttttcactgcattctagttgtggtttgtccaaactcatcaatgtatcttatcatgtctgg

SEQ ID NO: 134 - DNA, 4785 bp, synthetic construct
  misc_feature 1..4785: note = source = /note="Description of Artificial Sequence: Synthetic polynucleotide"
  misc_feature 1..4785: note = source = /note="XON-60"
  source 1..4785: mol_type = other DNA
gagcgtgcgtgaggctccggtgcccgtcagtgggcagagcgcacatcgcccacagtccccgagaagttggggggagggggtcggcgattgaaccggtgcctagagaaggtggcgcggggtaaactgggaaagtgatgtcgtgtactggctccgcctttttcccgagggtgggggagaaccgtatataagtgcagtagtcgccgtgaacgttctttttcgcaacgggtttgccgccagaacacagcagccgctaaatccaaggtaaggtcagaagagctagcgccaccatgctgctgctggtgaccagcctgctgctgtgtgagctgccccaccccgcctttctgctgatccccgacatccagatgacccagagccccagcagcctgtctgccagcgtgggcgacagagtgaccatcacctgtatgaccagcaccgacatcgacgacgacatgaactggtatcagcagaagcccggcaagacccccaagctgctgatctacgagggcaacaccctgaggcctggcgtgcccagcagattttctggcagcggctccggcaccgacttcatcttcaccatcagctccctgcagcccgaggatatcgccacctactactgcctgcagagctggaacgtgcccctgacctttggcggaggcaccaaggtggaaatcaagggcggaggcggatctggcggcggaggatctgggggaggcggctctcaggtgcagctgcaggaatctggcggagggctcgtgaagcctggcggaagcctgaagctgagctgtgccgccagcggcttcaccttcagcaagttcggcatgagctgggtgcgccagacccccgacaagagactggaatgggtggccagcatcagcaccggcggctacaatacctactacagcgacaacgtgaagggccggttcaccatctcccgggacaacgccaagaacaccctgtacctgcagatgagcagcctgaagtccgaggacaccgccatgtactactgtgccagaggctacagcccctacagctacgccatggattactggggccagggcacaatggtcaccgtgtcctctaagcctaccaccacccccgcacctcgtcctccaacccctgcacctacgattgccagtcagcctctttcactgcggcctgaggccagcagaccagctgccggcggtgccgtccatacaagaggactggacttcgcgtccgataaacctactaccactccagccccaaggcccccaaccccagcaccgactatcgcatcacagcctttgtcactgcgtcctgaagccagccggccagctgcagggggggccgtccacacaaggggactcgactttgcgagtgataagcccaccaccacccctgcccctagacctccaaccccagcccctacaatcgccagccagcccctgagcctgaggcccgaagcctgtagacctgccgctggcggagccgtgcacaccagaggcctggatttcgcctgcgacatctacatctgggcccctctggccggcacctgtggcgtgctgctgctgagcctggtcatcaccctgtactgcaaccaccggaataagagaggccggaagaaactgctgtacatcttcaagcagcccttcatgcggcccgtgcagaccacccaggaagaggacggctgcagctgccggttccccgaggaagaggaaggcggctgcgaactgcgggtgaagttcagccggagcgccgacgcccctgcctaccagcagggccagaaccagctgtacaacgagctgaacctgggccggagggaggagtacgacgtgctggacaagcggagaggccgggaccctgagatgggcggcaagccccggagaaagaaccctcaggagggcctgtataacgaactgcagaaagacaagatggccgaggcctacagcgagatcggcatgaagggcgagcggcggaggggcaagggccacgacggcctgtaccagggcctgagcaccgccaccaaggatacctacgacgccctgcacatgcaggccctgccccccagaagagctaagaggggaagcggagagggcagaggaagtctgctaacatgcggtgacgtcgaggagaatcctggacctggccccaagaagaaaaggaaggtggccccccccaccgacgtgagcctgggcgacgagctgcacctggacggcgaggacgtggccatggcccacgccgacgccctggacgacttcgacctggacatgctgggcgacggcgacagccccggccccggcttcaccccccacgacagcgccccctacggcgccctggacatggccgacttcgagttcgagcagatgttcaccgacgccctgggcatcgacgagtacggcggcgaattcgagatgcccgtggacaggattctggaggccgaactcgccgtggagcagaaaagcgaccagggcgtggagggccccggcggaaccggcggcagcggcagcagccccaacgaccccgtgaccaacatctgccaggccgccgacaagcagctgttcaccctggtggagtgggccaagaggattccccacttcagcagcctgcccctggacgaccaggtgatcctgctgagggccggatggaacgagctgctgatcgccagcttcagccacaggagcatcgacgtgagggacggcatcctgctggccaccggcctgcacgtccataggaacagcgcccacagcgccggagtgggcgccatcttcgacagggtgctgaccgagctggtgagcaagatgagggacatgaggatggacaagaccgagctgggctgcctgagggccatcatcctgttcaaccccgaggtgaggggcctgaaaagcgcccaggaggtggagctgctgagggagaaggtgtacgccgccctggaggagtacaccaggaccacccaccccgacgagcccggcagattcgccaagctgctgctgaggctgcccagcctgaggagcatcggcctgaagtgcctggagcacctgttcttcttcaggctgatcggcgacgtgcccatcgacaccttcctgatggagatgctggagagccccagcgacagctgagcatgcactagttttataatttcttcttccagaatttctgacattttataatttcttcttccagaagactcacaacctccatatggccaccatgaagctgctgagcagcatcgagcaggcttgcgacatctgcaggctgaagaagctgaagtgcagcaaggagaagcccaagtgcgccaagtgcctgaagaacaactgggagtgcagatacagccccaagaccaagaggagccccctgaccagggcccacctgaccgaggtggagagcaggctggagaggctggagcagctgttcctgctgatcttccccagggaggacctggacatgatcctgaagatggacagcctgcaagacatcaaggccctgctgaccggcctgttcgtgcaggacaacgtgaacaaggacgccgtgaccgacaggctggccagcgtggagaccgacatgcccctgaccctgaggcagcacaggatcagcgccaccagcagcagcgaggagagcagcaacaagggccagaggcagctgaccgtgagccccgagtttcccgggatcaggcccgagtgcgtggtgcccgagacccagtgcgccatgaaaaggaaggagaagaaggcccagaaggagaaggacaagctgcccgtgagcaccaccaccgtcgatgaccacatgccccccatcatgcagtgcgagccccccccccccgaggccgccaggattcacgaggtcgtgcccaggttcctgagcgacaagctgctggtgaccaacaggcagaagaacatcccccagctgaccgccaaccagcagttcctgatcgccaggctgatctggtatcaggacggctacgagcagcccagcgacgaggacctgaaaaggatcacccagacctggcagcaggccgacgacgagaacgaggagagcgacacccccttcaggcagatcaccgagatgaccatcctgaccgtgcagctgatcgtggagttcgccaagggcctgcccggattcgccaagatcagccagcccgaccagatcaccctgctgaaggcttgcagcagcgaggtgatgatgctgagggtggccaggaggtacgacgccgccagcgacagcatcctgttcgccaacaaccaggcttacaccagggacaactacaggaaggctggcatggccgaggtgatcgaggacctcctgcacttctgcagatgtatgtacagcatggccctggacaacatccactacgccctgctgaccgccgtggtgatcttcagcgacaggcccggcctggagcagccccagctggtggaggagatccagaggtactacctgaacaccctgaggatctacatcctgaaccagctgagcggcagcgccaggagcagcgtgatctacggcaagatcctgagcatcctgagcgagctgaggaccctgggaatgcagaacagcaatatgtgtatcagcctgaagctgaagaacaggaagctgccccccttcctggaggagatttgggacgtggccgacatgagccacacccagcccccccccatcctggagagccccaccaacctgtgaaacttgtttattgcagcttataatggttacaaataaagcaatagcatcacaaatttcacaaataaagcatttttttcactgcattctagttgtggtttgtccaaactcatcaatgtatcttatcatgtctgg

SEQ ID NO: 135 - DNA, 2009 bp, synthetic construct
  misc_feature 1..2009: note = source = /note="Description of Artificial Sequence: Synthetic polynucleotide"
  misc_feature 1..2009: note = source = /note="XON-61"
  source 1..2009: mol_type = other DNA
attgttcggagcagtgcggcgcgtttagcggagtactgtcctccgatattaatcggggcagactattccggggtttaccggcgcactctcgcccgaacttcaccggcggtctttcgtccgtgctttatcggggcggatcactccgaaccccgggaggtctatataagcagagctcgtttagtgaaccctcattctggagacggatcccgagccgagtgttttgacctccatagaacagccgctaaatccaaggtaaggtcagaagagctagcgccaccatgtgtcaccagcagttggtcatctcttggttcagcctggtttttctggcatctcccctcgtggccatctgggaactgaagaaagatgtttatgtcgtagaattggattggtatcccgacgcccctggagaaatggtggtcctgacatgtgacacccctgaagaagatggtatcacctggaccttggaccagagcagtgaggtcttaggctctggcaagaccctgaccatccaagtcaaagagtttggagatgctggccagtacacctgtcacaaaggaggcgaggttctaagccattcgctcctgctgcttcacaaaaaggaagatggaatttggtccactgacattctgaaggaccagaaagaacccaagaataagacctttctaagatgcgaggccaagaattattctggacgtttcacctgctggtggctgacgacaatcagtactgatttgacattcagtgtcaaaagcagcagaggctcttctgacccccaaggggtgacgtgcggagctgctacactcagcgccgagagagtcagaggggacaacaaggagtatgagtactcagtggagtgccaggaggacagtgcctgcccagctgctgaggagagtctgcccattgaggtcatggtggatgccgttcacaagctcaagtatgaaaactacaccagcagcttcttcatcagggacatcatcaaacctgacccacccaagaacttgcagctgaagcccctgaagaacagcagacaggtggaggtcagctgggagtaccctgacacctggagtactccacattcctacttctccctgacattctgcgttcaggtccagggcaagagcaagagagaaaagaaagatagagtcttcacggacaagacctcagccacggtcatctgccgcaaaaatgccagcattagcgtgcgggcccaggaccgctactatagctcatcttggagcgaatgggcatctgtgccctgctccggtggcggtggcggcggatctagaaacctccccgtggccactccagacccaggaatgttcccatgccttcaccacagccagaacctgctgagggccgtcagcaacatgctccagaaggccagacaaactctagaattttacccttgcacttctgaagagattgatcatgaagatatcacaaaagataaaaccagcacagtggaggcctgtttaccattggaattaaccaagaatgagagttgcctaaattccagagagacctctttcataactaatgggagttgcctggcctccagaaagacctcttttatgatggccctgtgccttagtagtatttatgaagacttgaagatgtaccaggtggagttcaagaccatgaatgcaaagctgctgatggaccccaagaggcagatctttctagatcaaaacatgctggcagttattgatgagctgatgcaggccctgaatttcaacagtgagactgtgccacaaaaatcctcccttgaagaaccggatttttataaaactaaaatcaagctctgcatacttcttcatgctttcagaatcagagcagtgactattgatagagtgatgagctatctgaatgcttcctaaaacttgtttattgcagcttataatggttacaaataaagcaatagcatcacaaatttcacaaataaagcatttttttcactgcattctagttgtggtttgtccaaactcatcaatgtatcttatcatgtctgg

SEQ ID NO: 136 - DNA, 2873 bp, synthetic construct
  misc_feature 1..2873: note = source = /note="Description of Artificial Sequence: Synthetic polynucleotide"
  misc_feature 1..2873: note = source = /note="XON-62"
  source 1..2873: mol_type = other DNA
attgttcggagcagtgcggcgcgtttagcggagtactgtcctccgatattaatcggggcagactattccggggtttaccggcgcactctcgcccgaacttcaccggcggtctttcgtccgtgctttatcggggcggatcactccgaaccccgggaggtctatataagcagagctcgtttagtgaaccctcattctggagacggatcccgagccgagtgttttgacctccatagaacagccgctaaatccaaggtaaggtcagaagagctagcgccaccatgtgtcaccagcagttggtcatctcttggttcagcctggtttttctggcatctcccctcgtggccatctgggaactgaagaaagatgtttatgtcgtagaattggattggtatcccgacgcccctggagaaatggtggtcctgacatgtgacacccctgaagaagatggtatcacctggaccttggaccagagcagtgaggtcttaggctctggcaagaccctgaccatccaagtcaaagagtttggagatgctggccagtacacctgtcacaaaggaggcgaggttctaagccattcgctcctgctgcttcacaaaaaggaagatggaatttggtccactgacattctgaaggaccagaaagaacccaagaataagacctttctaagatgcgaggccaagaattattctggacgtttcacctgctggtggctgacgacaatcagtactgatttgacattcagtgtcaaaagcagcagaggctcttctgacccccaaggggtgacgtgcggagctgctacactcagcgccgagagagtcagaggggacaacaaggagtatgagtactcagtggagtgccaggaggacagtgcctgcccagctgctgaggagagtctgcccattgaggtcatggtggatgccgttcacaagctcaagtatgaaaactacaccagcagcttcttcatcagggacatcatcaaacctgacccacccaagaacttgcagctgaagcccctgaagaacagcagacaggtggaggtcagctgggagtaccctgacacctggagtactccacattcctacttctccctgacattctgcgttcaggtccagggcaagagcaagagagaaaagaaagatagagtcttcacggacaagacctcagccacggtcatctgccgcaaaaatgccagcattagcgtgcgggcccaggaccgctactatagctcatcttggagcgaatgggcatctgtgccctgctccggtggcggtggcggcggatctagaaacctccccgtggccactccagacccaggaatgttcccatgccttcaccacagccagaacctgctgagggccgtcagcaacatgctccagaaggccagacaaactctagaattttacccttgcacttctgaagagattgatcatgaagatatcacaaaagataaaaccagcacagtggaggcctgtttaccattggaattaaccaagaatgagagttgcctaaattccagagagacctctttcataactaatgggagttgcctggcctccagaaagacctcttttatgatggccctgtgccttagtagtatttatgaagacttgaagatgtaccaggtggagttcaagaccatgaatgcaaagctgctgatggaccccaagaggcagatctttctagatcaaaacatgctggcagttattgatgagctgatgcaggccctgaatttcaacagtgagactgtgccacaaaaatcctcccttgaagaaccggatttttataaaactaaaatcaagctctgcatacttcttcatgctttcagaatcagagcagtgactattgatagagtgatgagctatctgaatgcttccagagctaagaggggaagcggagagggcagaggaagtctgctaacatgcggtgacgtcgaggagaatcctggacctaggctccctgctcagctcctggggctgctaatgctctgggtcccaggatccagtgggcgcaaagtgtgtaacggaataggtattggtgaatttaaagactcactctccataaatgctacgaatattaaacacttcaaaaactgcacctccatcagtggcgatctccacatcctgccggtggcatttaggggtgactccttcacacatactcctcctctggatccacaggaactggatattctgaaaaccgtaaaggaaatcacagggtttttgctgattcaggcttggcctgaaaacaggacggacctccatgcctttgagaacctagaaatcatacgcggcaggaccaagcaacatggtcagttttctcttgcagtcgtcagcctgaacataacatccttgggattacgctccctcaaggagataagtgatggagatgtgataatttcaggaaacaaaaatttgtgctatgcaaatacaataaactggaaaaaactgtttgggacctccggtcagaaaaccaaaattataagcaacagaggtgaaaacagctgcaaggccacaggccaggtctgccatgccttgtgctcccccgagggctgctggggcccggagcccagggactgcgtctctggtggcggtggctcgggcggtggtgggtcgggtggcggcggatctggtggcggtggctcgttttgggtgctggtggtggttggtggagtcctggcttgctatagcttgctagtaacagtggcctttattattttctgggtgaggagtaagaggagctaaaacttgtttattgcagcttataatggttacaaataaagcaatagcatcacaaatttcacaaataaagcatttttttcactgcattctagttgtggtttgtccaaactcatcaatgtatcttatcatgtctgg

SEQ ID NO: 137 - DNA, 3532 bp, synthetic construct
  misc_feature 1..3532: note = source = /note="Description of Artificial Sequence: Synthetic polynucleotide"
  misc_feature 1..3532: note = source = /note="FLC-2B12/13-2"
  source 1..3532: mol_type = other DNA
attgttcggagcagtgcggcgcgtttagcggagtactgtcctccgatattaatcggggcagactattccggggtttaccggcgcactctcgcccgaacttcaccggcggtctttcgtccgtgctttatcggggcggatcactccgaaccccgggaggtctatataagcagagctcgtttagtgaaccctcattctggagacggatcccgagccgagtgttttgacctccatagaacagccgctaaatccaaggtaaggtcagaagagctagcgccaccatggattggacctggattctgtttctggtggccgctgccacaagagtgcacagcaactgggtgaatgtgatcagcgacctgaagaagatcgaggatctgatccagagcatgcacattgatgccaccctgtacacagaatctgatgtgcaccctagctgtaaagtgaccgccatgaagtgttttctgctggagctgcaggtgatttctctggaaagcggagatgcctctatccacgacacagtggagaatctgatcatcctggccaacaatagcctgagcagcaatggcaatgtgacagagtctggctgtaaggagtgtgaggagctggaggagaagaacatcaaggagtttctgcagagctttgtgcacatcgtgcagatgttcatcaatacaagctctggcggaggatctggaggaggcggatctggaggaggaggcagtggaggcggaggatctggcggaggatctctgcagattacatgccctcctccaatgtctgtggagcacgccgatatttgggtgaagtcctacagcctgtacagcagagagagatacatctgcaacagcggctttaagagaaaggccggcacctcttctctgacagagtgcgtgctgaataaggccacaaatgtggcccactggacaacacctagcctgaagtgcattagagatcctgccctggtccaccagaggcctgcccctccatctacagtgacaacagccggagtgacacctcagcctgaatctctgagcccttctggaaaagaacctgccgccagctctcctagctctaataataccgccgccacaacagccgccattgtgcctggatctcagctgatgcctagcaagtctcctagcacaggcacaacagagatcagcagccacgaatcttctcacggaacaccttctcagaccaccgccaagaattgggagctgacagcctctgcctctcaccagcctccaggagtgtatcctcagggccactctgatacaacagtggccatcagcacatctacagtgctgctgtgtggactgtctgccgtgtctctgctggcctgttacctgaagtctagacagacacctcctctggcctctgtggagatggaggccatggaagccctgcctgtgacatggggaacaagcagcagagatgaggacctggagaattgttctcaccacctgtgaaacttgtttattgcagcttataatggttacaaataaagcaatagcatcacaaatttcacaaataaagcatttttttcactgcattctagttgtggtttgtccaaactcatcaatgtatcttatcatgtctgggagcgtgcgtgaggctccggtgcccgtcagtgggcagagcgcacatcgcccacagtccccgagaagttggggggagggggtcggcgattgaaccggtgcctagagaaggtggcgcggggtaaactgggaaagtgatgtcgtgtactggctccgcctttttcccgagggtgggggagaaccgtatataagtgcagtagtcgccgtgaacgttctttttcgcaacgggtttgccgccagaacacagcagccgctaaatccaaggtaaggtcagaagagctagcgccaccatgaagctgctgagcagcatcgagcaggcttgcgacatctgcaggctgaagaagctgaagtgcagcaaggagaagcccaagtgcgccaagtgcctgaagaacaactgggagtgcagatacagccccaagaccaagaggagccccctgaccagggcccacctgaccgaggtggagagcaggctggagaggctggagcagctgttcctgctgatcttccccagggaggacctggacatgatcctgaagatggacagcctgcaagacatcaaggccctgctgaccggcctgttcgtgcaggacaacgtgaacaaggacgccgtgaccgacaggctggccagcgtggagaccgacatgcccctgaccctgaggcagcacaggatcagcgccaccagcagcagcgaggagagcagcaacaagggccagaggcagctgaccgtgagccccgagtttcccgggatcaggcccgagtgcgtggtgcccgagacccagtgcgccatgaaaaggaaggagaagaaggcccagaaggagaaggacaagctgcccgtgagcaccaccaccgtcgatgaccacatgccccccatcatgcagtgcgagccccccccccccgaggccgccaggattcacgaggtcgtgcccaggttcctgagcgacaagctgctggtgaccaacaggcagaagaacatcccccagctgaccgccaaccagcagttcctgatcgccaggctgatctggtatcaggacggctacgagcagcccagcgacgaggacctgaaaaggatcacccagacctggcagcaggccgacgacgagaacgaggagagcgacacccccttcaggcagatcaccgagatgaccatcctgaccgtgcagctgatcgtggagttcgccaagggcctgcccggattcgccaagatcagccagcccgaccagatcaccctgctgaaggcttgcagcagcgaggtgatgatgctgagggtggccaggaggtacgacgccgccagcgacagcatcctgttcgccaacaaccaggcttacaccagggacaactacaggaaggctggcatggccgaggtgatcgaggacctcctgcacttctgcagatgtatgtacagcatggccctggacaacatccactacgccctgctgaccgccgtggtgatcttcagcgacaggcccggcctggagcagccccagctggtggaggagatccagaggtactacctgaacaccctgaggatctacatcctgaaccagctgagcggcagcgccaggagcagcgtgatctacggcaagatcctgagcatcctgagcgagctgaggaccctgggaatgcagaacagcaatatgtgtatcagcctgaagctgaagaacaggaagctgccccccttcctggaggagatttgggacgtggccgacatgagccacacccagcccccccccatcctggagagccccaccaacctgtgatgatgggtggcatccctgtgacccctccccagtgcctctcctggccctggaagttgccactccagtgcccaccagccttgtcctaataaaattaagttgcatcattttgtctgactaggtgtccttctataatattatggggtggaggggggtggtatggagcaaggggcaagttgggaa

SEQ ID NO: 138 - DNA, 4423 bp, synthetic construct
  misc_feature 1..4423: note = source = /note="Description of Artificial Sequence: Synthetic polynucleotide"
  misc_feature 1..4423: note = source = /note="XON-02"
  source 1..4423: mol_type = other DNA
attgttcggagcagtgcggcgcgtttagcggagtactgtcctccgatattaatcggggcagactattccggggtttaccggcgcactctcgcccgaacttcaccggcggtctttcgtccgtgctttatcggggcggatcactccgaaccccgggaggtctatataagcagagctcgtttagtgaaccctcattctggagacggatcccgagccgagtgttttgacctccatagaacagccgctaaatccaaggtaaggtcagaagagctagcgccaccatggattggacctggattctgtttctggtggccgctgccacaagagtgcacagcaactgggtgaatgtgatcagcgacctgaagaagatcgaggatctgatccagagcatgcacattgatgccaccctgtacacagaatctgatgtgcaccctagctgtaaagtgaccgccatgaagtgttttctgctggagctgcaggtgatttctctggaaagcggagatgcctctatccacgacacagtggagaatctgatcatcctggccaacaatagcctgagcagcaatggcaatgtgacagagtctggctgtaaggagtgtgaggagctggaggagaagaacatcaaggagtttctgcagagctttgtgcacatcgtgcagatgttcatcaatacaagctctggcggaggatctggaggaggcggatctggaggaggaggcagtggaggcggaggatctggcggaggatctctgcagattacatgccctcctccaatgtctgtggagcacgccgatatttgggtgaagtcctacagcctgtacagcagagagagatacatctgcaacagcggctttaagagaaaggccggcacctcttctctgacagagtgcgtgctgaataaggccacaaatgtggcccactggacaacacctagcctgaagtgcattagagatcctgccctggtccaccagaggcctgcccctccatctacagtgacaacagccggagtgacacctcagcctgaatctctgagcccttctggaaaagaacctgccgccagctctcctagctctaataataccgccgccacaacagccgccattgtgcctggatctcagctgatgcctagcaagtctcctagcacaggcacaacagagatcagcagccacgaatcttctcacggaacaccttctcagaccaccgccaagaattgggagctgacagcctctgcctctcaccagcctccaggagtgtatcctcagggccactctgatacaacagtggccatcagcacatctacagtgctgctgtgtggactgtctgccgtgtctctgctggcctgttacctgaagtctagacagacacctcctctggcctctgtggagatggaggccatggaagccctgcctgtgacatggggaacaagcagcagagatgaggacctggagaattgttctcaccacctgtgaaacttgtttattgcagcttataatggttacaaataaagcaatagcatcacaaatttcacaaataaagcatttttttcactgcattctagttgtggtttgtccaaactcatcaatgtatcttatcatgtctgggagcgtgcgtgaggctccggtgcccgtcagtgggcagagcgcacatcgcccacagtccccgagaagttggggggagggggtcggcgattgaaccggtgcctagagaaggtggcgcggggtaaactgggaaagtgatgtcgtgtactggctccgcctttttcccgagggtgggggagaaccgtatataagtgcagtagtcgccgtgaacgttctttttcgcaacgggtttgccgccagaacacagcagccgctaaatccaaggtaaggtcagaagagctagcgccaccatgctgctgctggtgaccagcctgctgctgtgtgagctgccccaccccgcctttctgctgatccccgacatccagatgacccagaccacctccagcctgagcgccagcctgggcgaccgggtgaccatcagctgccgggccagccaggacatcagcaagtacctgaactggtatcagcagaagcccgacggcaccgtcaagctgctgatctaccacaccagccggctgcacagcggcgtgcccagccggtttagcggcagcggctccggcaccgactacagcctgaccatctccaacctggagcaggaggacatcgccacctacttttgccagcagggcaacacactgccctacacctttggcggcggaacaaagctggagatcaccggcagcacctccggcagcggcaagcctggcagcggcgagggcagcaccaagggcgaggtgaagctgcaggagagcggccctggcctggtggcccccagccagagcctgagcgtgacctgtaccgtgtccggcgtgtccctgcccgactacggcgtgtcctggatccggcagccccctaggaagggcctggagtggctgggcgtgatctggggcagcgagaccacctactacaacagcgccctgaagagccggctgaccatcatcaaggacaacagcaagagccaggtgttcctgaagatgaacagcctgcagaccgacgacaccgccatctactactgtgccaagcactactactacggcggcagctacgccatggactactggggccagggcaccagcgtgaccgtgtccagcaagcccaccaccacccctgcccctagacctccaaccccagcccctacaatcgccagccagcccctgagcctgaggcccgaagcctgtagacctgccgctggcggagccgtgcacaccagaggcctggatttcgcctgcgacatctacatctgggcccctctggccggcacctgtggcgtgctgctgctgagcctggtcatcaccctgtactgcaaccaccggaataggagcaagcggagcagaggcggccacagcgactacatgaacatgaccccccggaggcctggccccacccggaagcactaccagccctacgcccctcccagggacttcgccgcctaccggagccgggtgaagttcagccggagcgccgacgcccctgcctaccagcagggccagaaccagctgtacaacgagctgaacctgggccggagggaggagtacgacgtgctggacaagcggagaggccgggaccctgagatgggcggcaagccccggagaaagaaccctcaggagggcctgtataacgaactgcagaaagacaagatggccgaggcctacagcgagatcggcatgaagggcgagcggcggaggggcaagggccacgacggcctgtaccagggcctgagcaccgccaccaaggatacctacgacgccctgcacatgcaggccctgccccccagaagggccaagaggagtggcagcggcgagggcagaggaagtcttctaacatgcggtgacgtggaggagaatcccggccctatgaggctccctgctcagctcctggggctgctaatgctctgggtcccaggatccagtgggcgcaaagtgtgtaacggaataggtattggtgaatttaaagactcactctccataaatgctacgaatattaaacacttcaaaaactgcacctccatcagtggcgatctccacatcctgccggtggcatttaggggtgactccttcacacatactcctcctctggatccacaggaactggatattctgaaaaccgtaaaggaaatcacagggtttttgctgattcaggcttggcctgaaaacaggacggacctccatgcctttgagaacctagaaatcatacgcggcaggaccaagcaacatggtcagttttctcttgcagtcgtcagcctgaacataacatccttgggattacgctccctcaaggagataagtgatggagatgtgataatttcaggaaacaaaaatttgtgctatgcaaatacaataaactggaaaaaactgtttgggacctccggtcagaaaaccaaaattataagcaacagaggtgaaaacagctgcaaggccacaggccaggtctgccatgccttgtgctcccccgagggctgctggggcccggagcccagggactgcgtctctggtggcggtggctcgggcggtggtgggtcgggtggcggcggatctggtggcggtggctcgttttgggtgctggtggtggttggtggagtcctggcttgctatagcttgctagtaacagtggcctttattattttctgggtgaggagtaagaggagctaatgatgggtggcatccctgtgacccctccccagtgcctctcctggccctggaagttgccactccagtgcccaccagccttgtcctaataaaattaagttgcatcattttgtctgactaggtgtccttctataatattatggggtggaggggggtggtatggagcaaggggcaagttgggaa

SEQ ID NO: 139 - DNA, 4423 bp, synthetic construct
  misc_feature 1..4423: note = source = /note="Description of Artificial Sequence: Synthetic polynucleotide"
  misc_feature 1..4423: note = source = /note="XON-02(h)"
  source 1..4423: mol_type = other DNA
gagcgtgcgtgaggctccggtgcccgtcagtgggcagagcgcacatcgcccacagtccccgagaagttggggggagggggtcggcgattgaaccggtgcctagagaaggtggcgcggggtaaactgggaaagtgatgtcgtgtactggctccgcctttttcccgagggtgggggagaaccgtatataagtgcagtagtcgccgtgaacgttctttttcgcaacgggtttgccgccagaacacagcagccgctaaatccaaggtaaggtcagaagagctagcgccaccatgctgctgctggtgaccagcctgctgctgtgtgagctgccccaccccgcctttctgctgatccccgacatccagatgacccagaccacctccagcctgagcgccagcctgggcgaccgggtgaccatcagctgccgggccagccaggacatcagcaagtacctgaactggtatcagcagaagcccgacggcaccgtcaagctgctgatctaccacaccagccggctgcacagcggcgtgcccagccggtttagcggcagcggctccggcaccgactacagcctgaccatctccaacctggagcaggaggacatcgccacctacttttgccagcagggcaacacactgccctacacctttggcggcggaacaaagctggagatcaccggcagcacctccggcagcggcaagcctggcagcggcgagggcagcaccaagggcgaggtgaagctgcaggagagcggccctggcctggtggcccccagccagagcctgagcgtgacctgtaccgtgtccggcgtgtccctgcccgactacggcgtgtcctggatccggcagccccctaggaagggcctggagtggctgggcgtgatctggggcagcgagaccacctactacaacagcgccctgaagagccggctgaccatcatcaaggacaacagcaagagccaggtgttcctgaagatgaacagcctgcagaccgacgacaccgccatctactactgtgccaagcactactactacggcggcagctacgccatggactactggggccagggcaccagcgtgaccgtgtccagcaagcccaccaccacccctgcccctagacctccaaccccagcccctacaatcgccagccagcccctgagcctgaggcccgaagcctgtagacctgccgctggcggagccgtgcacaccagaggcctggatttcgcctgcgacatctacatctgggcccctctggccggcacctgtggcgtgctgctgctgagcctggtcatcaccctgtactgcaaccaccggaataggagcaagcggagcagaggcggccacagcgactacatgaacatgaccccccggaggcctggccccacccggaagcactaccagccctacgcccctcccagggacttcgccgcctaccggagccgggtgaagttcagccggagcgccgacgcccctgcctaccagcagggccagaaccagctgtacaacgagctgaacctgggccggagggaggagtacgacgtgctggacaagcggagaggccgggaccctgagatgggcggcaagccccggagaaagaaccctcaggagggcctgtataacgaactgcagaaagacaagatggccgaggcctacagcgagatcggcatgaagggcgagcggcggaggggcaagggccacgacggcctgtaccagggcctgagcaccgccaccaaggatacctacgacgccctgcacatgcaggccctgccccccagaagggccaagaggagtggcagcggcgagggcagaggaagtcttctaacatgcggtgacgtggaggagaatcccggccctatgaggctccctgctcagctcctggggctgctaatgctctgggtcccaggatccagtgggcgcaaagtgtgtaacggaataggtattggtgaatttaaagactcactctccataaatgctacgaatattaaacacttcaaaaactgcacctccatcagtggcgatctccacatcctgccggtggcatttaggggtgactccttcacacatactcctcctctggatccacaggaactggatattctgaaaaccgtaaaggaaatcacagggtttttgctgattcaggcttggcctgaaaacaggacggacctccatgcctttgagaacctagaaatcatacgcggcaggaccaagcaacatggtcagttttctcttgcagtcgtcagcctgaacataacatccttgggattacgctccctcaaggagataagtgatggagatgtgataatttcaggaaacaaaaatttgtgctatgcaaatacaataaactggaaaaaactgtttgggacctccggtcagaaaaccaaaattataagcaacagaggtgaaaacagctgcaaggccacaggccaggtctgccatgccttgtgctcccccgagggctgctggggcccggagcccagggactgcgtctctggtggcggtggctcgggcggtggtgggtcgggtggcggcggatctggtggcggtggctcgttttgggtgctggtggtggttggtggagtcctggcttgctatagcttgctagtaacagtggcctttattattttctgggtgaggagtaagaggagctaatgatgggtggcatccctgtgacccctccccagtgcctctcctggccctggaagttgccactccagtgcccaccagccttgtcctaataaaattaagttgcatcattttgtctgactaggtgtccttctataatattatggggtggaggggggtggtatggagcaaggggcaagttgggaaattgttcggagcagtgcggcgcgtttagcggagtactgtcctccgatattaatcggggcagactattccggggtttaccggcgcactctcgcccgaacttcaccggcggtctttcgtccgtgctttatcggggcggatcactccgaaccccgggaggtctatataagcagagctcgtttagtgaaccctcattctggagacggatcccgagccgagtgttttgacctccatagaacagccgctaaatccaaggtaaggtcagaagagctagcgccaccatggattggacctggattctgtttctggtggccgctgccacaagagtgcacagcaactgggtgaatgtgatcagcgacctgaagaagatcgaggatctgatccagagcatgcacattgatgccaccctgtacacagaatctgatgtgcaccctagctgtaaagtgaccgccatgaagtgttttctgctggagctgcaggtgatttctctggaaagcggagatgcctctatccacgacacagtggagaatctgatcatcctggccaacaatagcctgagcagcaatggcaatgtgacagagtctggctgtaaggagtgtgaggagctggaggagaagaacatcaaggagtttctgcagagctttgtgcacatcgtgcagatgttcatcaatacaagctctggcggaggatctggaggaggcggatctggaggaggaggcagtggaggcggaggatctggcggaggatctctgcagattacatgccctcctccaatgtctgtggagcacgccgatatttgggtgaagtcctacagcctgtacagcagagagagatacatctgcaacagcggctttaagagaaaggccggcacctcttctctgacagagtgcgtgctgaataaggccacaaatgtggcccactggacaacacctagcctgaagtgcattagagatcctgccctggtccaccagaggcctgcccctccatctacagtgacaacagccggagtgacacctcagcctgaatctctgagcccttctggaaaagaacctgccgccagctctcctagctctaataataccgccgccacaacagccgccattgtgcctggatctcagctgatgcctagcaagtctcctagcacaggcacaacagagatcagcagccacgaatcttctcacggaacaccttctcagaccaccgccaagaattgggagctgacagcctctgcctctcaccagcctccaggagtgtatcctcagggccactctgatacaacagtggccatcagcacatctacagtgctgctgtgtggactgtctgccgtgtctctgctggcctgttacctgaagtctagacagacacctcctctggcctctgtggagatggaggccatggaagccctgcctgtgacatggggaacaagcagcagagatgaggacctggagaattgttctcaccacctgtgaaacttgtttattgcagcttataatggttacaaataaagcaatagcatcacaaatttcacaaataaagcatttttttcactgcattctagttgtggtttgtccaaactcatcaatgtatcttatcatgtctgg

SEQ ID NO: 140 - DNA, 4487 bp, synthetic construct
  misc_feature 1..4487: note = source = /note="Description of Artificial Sequence: Synthetic polynucleotide"
  misc_feature 1..4487: note = source = /note="FLC-2B8-1"
  source 1..4487: mol_type = other DNA
gagcgtgcgtgaggctccggtgcccgtcagtgggcagagcgcacatcgcccacagtccccgagaagttggggggagggggtcggcgattgaaccggtgcctagagaaggtggcgcggggtaaactgggaaagtgatgtcgtgtactggctccgcctttttcccgagggtgggggagaaccgtatataagtgcagtagtcgccgtgaacgttctttttcgcaacgggtttgccgccagaacacagcagccgctaaatccaaggtaaggtcagaagagctagcgccaccatgctgctgctggtgaccagcctgctgctgtgtgagctgccccaccccgcctttctgctgatccccgacatccagatgacccagaccacctccagcctgagcgccagcctgggcgaccgggtgaccatcagctgccgggccagccaggacatcagcaagtacctgaactggtatcagcagaagcccgacggcaccgtcaagctgctgatctaccacaccagccggctgcacagcggcgtgcccagccggtttagcggcagcggctccggcaccgactacagcctgaccatctccaacctggagcaggaggacatcgccacctacttttgccagcagggcaacacactgccctacacctttggcggcggaacaaagctggagatcaccggcagcacctccggcagcggcaagcctggcagcggcgagggcagcaccaagggcgaggtgaagctgcaggagagcggccctggcctggtggcccccagccagagcctgagcgtgacctgtaccgtgtccggcgtgtccctgcccgactacggcgtgtcctggatccggcagccccctaggaagggcctggagtggctgggcgtgatctggggcagcgagaccacctactacaacagcgccctgaagagccggctgaccatcatcaaggacaacagcaagagccaggtgttcctgaagatgaacagcctgcagaccgacgacaccgccatctactactgtgccaagcactactactacggcggcagctacgccatggactactggggccagggcaccagcgtgaccgtgtccagcaagcccaccaccacccctgcccctagacctccaaccccagcccctacaatcgccagccagcccctgagcctgaggcccgaagcctgtagacctgccgctggcggagccgtgcacaccagaggcctggatttcgcctgcgacatctacatctgggcccctctggccggcacctgtggcgtgctgctgctgagcctggtcatcaccctgtactgcaaccaccggaataggagcaagcggagcagaggcggccacagcgactacatgaacatgaccccccggaggcctggccccacccggaagcactaccagccctacgcccctcccagggacttcgccgcctaccggagccgggtgaagttcagccggagcgccgacgcccctgcctaccagcagggccagaaccagctgtacaacgagctgaacctgggccggagggaggagtacgacgtgctggacaagcggagaggccgggaccctgagatgggcggcaagccccggagaaagaaccctcaggagggcctgtataacgaactgcagaaagacaagatggccgaggcctacagcgagatcggcatgaagggcgagcggcggaggggcaagggccacgacggcctgtaccagggcctgagcaccgccaccaaggatacctacgacgccctgcacatgcaggccctgccccccagaagagctaagaggggaagcggagagggcagaggaagtctgctaacatgcggtgacgtcgaggagaatcctggacctggccccaagaagaaaaggaaggtggccccccccaccgacgtgagcctgggcgacgagctgcacctggacggcgaggacgtggccatggcccacgccgacgccctggacgacttcgacctggacatgctgggcgacggcgacagccccggccccggcttcaccccccacgacagcgccccctacggcgccctggacatggccgacttcgagttcgagcagatgttcaccgacgccctgggcatcgacgagtacggcggcgaattcgagatgcccgtggacaggattctggaggccgaactcgccgtggagcagaaaagcgaccagggcgtggagggccccggcggaaccggcggcagcggcagcagccccaacgaccccgtgaccaacatctgccaggccgccgacaagcagctgttcaccctggtggagtgggccaagaggattccccacttcagcagcctgcccctggacgaccaggtgatcctgctgagggccggatggaacgagctgctgatcgccagcttcagccacaggagcatcgacgtgagggacggcatcctgctggccaccggcctgcacgtccataggaacagcgcccacagcgccggagtgggcgccatcttcgacagggtgctgaccgagctggtgagcaagatgagggacatgaggatggacaagaccgagctgggctgcctgagggccatcatcctgttcaaccccgaggtgaggggcctgaaaagcgcccaggaggtggagctgctgagggagaaggtgtacgccgccctggaggagtacaccaggaccacccaccccgacgagcccggcagattcgccaagctgctgctgaggctgcccagcctgaggagcatcggcctgaagtgcctggagcacctgttcttcttcaggctgatcggcgacgtgcccatcgacaccttcctgatggagatgctggagagccccagcgacagcagagctaagaggggaagcggagagggcagaggaagtctgctaacatgcggtgacgtcgaggagaatcctggacctaagctgctgagcagcatcgagcaggcttgcgacatctgcaggctgaagaagctgaagtgcagcaaggagaagcccaagtgcgccaagtgcctgaagaacaactgggagtgcagatacagccccaagaccaagaggagccccctgaccagggcccacctgaccgaggtggagagcaggctggagaggctggagcagctgttcctgctgatcttccccagggaggacctggacatgatcctgaagatggacagcctgcaagacatcaaggccctgctgaccggcctgttcgtgcaggacaacgtgaacaaggacgccgtgaccgacaggctggccagcgtggagaccgacatgcccctgaccctgaggcagcacaggatcagcgccaccagcagcagcgaggagagcagcaacaagggccagaggcagctgaccgtgagccccgagtttcccgggatcaggcccgagtgcgtggtgcccgagacccagtgcgccatgaaaaggaaggagaagaaggcccagaaggagaaggacaagctgcccgtgagcaccaccaccgtcgatgaccacatgccccccatcatgcagtgcgagccccccccccccgaggccgccaggattcacgaggtcgtgcccaggttcctgagcgacaagctgctggtgaccaacaggcagaagaacatcccccagctgaccgccaaccagcagttcctgatcgccaggctgatctggtatcaggacggctacgagcagcccagcgacgaggacctgaaaaggatcacccagacctggcagcaggccgacgacgagaacgaggagagcgacacccccttcaggcagatcaccgagatgaccatcctgaccgtgcagctgatcgtggagttcgccaagggcctgcccggattcgccaagatcagccagcccgaccagatcaccctgctgaaggcttgcagcagcgaggtgatgatgctgagggtggccaggaggtacgacgccgccagcgacagcatcctgttcgccaacaaccaggcttacaccagggacaactacaggaaggctggcatggccgaggtgatcgaggacctcctgcacttctgcagatgtatgtacagcatggccctggacaacatccactacgccctgctgaccgccgtggtgatcttcagcgacaggcccggcctggagcagccccagctggtggaggagatccagaggtactacctgaacaccctgaggatctacatcctgaaccagctgagcggcagcgccaggagcagcgtgatctacggcaagatcctgagcatcctgagcgagctgaggaccctgggaatgcagaacagcaatatgtgtatcagcctgaagctgaagaacaggaagctgccccccttcctggaggagatttgggacgtggccgacatgagccacacccagcccccccccatcctggagagccccaccaacctgtgaaacttgtttattgcagcttataatggttacaaataaagcaatagcatcacaaatttcacaaataaagcatttttttcactgcattctagttgtggtttgtccaaactcatcaatgtatcttatcatgtctgg

SEQ ID NO: 141 - DNA, 4509 bp, synthetic construct
  misc_feature 1..4509: note = source = /note="Description of Artificial Sequence: Synthetic polynucleotide"
  misc_feature 1..4509: note = source = /note="FLC-2A3-1"
  source 1..4509: mol_type = other DNA
gagcgtgcgtgaggctccggtgcccgtcagtgggcagagcgcacatcgcccacagtccccgagaagttggggggagggggtcggcgattgaaccggtgcctagagaaggtggcgcggggtaaactgggaaagtgatgtcgtgtactggctccgcctttttcccgagggtgggggagaaccgtatataagtgcagtagtcgccgtgaacgttctttttcgcaacgggtttgccgccagaacacagcagccgctaaatccaaggtaaggtcagaagagctagcgccaccatgctgctgctggtgaccagcctgctgctgtgtgagctgccccaccccgcctttctgctgatccccgacatccagatgacccagaccacctccagcctgagcgccagcctgggcgaccgggtgaccatcagctgccgggccagccaggacatcagcaagtacctgaactggtatcagcagaagcccgacggcaccgtcaagctgctgatctaccacaccagccggctgcacagcggcgtgcccagccggtttagcggcagcggctccggcaccgactacagcctgaccatctccaacctggagcaggaggacatcgccacctacttttgccagcagggcaacacactgccctacacctttggcggcggaacaaagctggagatcaccggcagcacctccggcagcggcaagcctggcagcggcgagggcagcaccaagggcgaggtgaagctgcaggagagcggccctggcctggtggcccccagccagagcctgagcgtgacctgtaccgtgtccggcgtgtccctgcccgactacggcgtgtcctggatccggcagccccctaggaagggcctggagtggctgggcgtgatctggggcagcgagaccacctactacaacagcgccctgaagagccggctgaccatcatcaaggacaacagcaagagccaggtgttcctgaagatgaacagcctgcagaccgacgacaccgccatctactactgtgccaagcactactactacggcggcagctacgccatggactactggggccagggcaccagcgtgaccgtgtccagcaagcccaccaccacccctgcccctagacctccaaccccagcccctacaatcgccagccagcccctgagcctgaggcccgaagcctgtagacctgccgctggcggagccgtgcacaccagaggcctggatttcgcctgcgacatctacatctgggcccctctggccggcacctgtggcgtgctgctgctgagcctggtcatcaccctgtactgcaaccaccggaataggagcaagcggagcagaggcggccacagcgactacatgaacatgaccccccggaggcctggccccacccggaagcactaccagccctacgcccctcccagggacttcgccgcctaccggagccgggtgaagttcagccggagcgccgacgcccctgcctaccagcagggccagaaccagctgtacaacgagctgaacctgggccggagggaggagtacgacgtgctggacaagcggagaggccgggaccctgagatgggcggcaagccccggagaaagaaccctcaggagggcctgtataacgaactgcagaaagacaagatggccgaggcctacagcgagatcggcatgaagggcgagcggcggaggggcaagggccacgacggcctgtaccagggcctgagcaccgccaccaaggatacctacgacgccctgcacatgcaggccctgccccccagaagagctaagaggggaagcggagagggcagaggaagtctgctaacatgcggtgacgtcgaggagaatcctggacctggccccaagaagaaaaggaaggtggccccccccaccgacgtgagcctgggcgacgagctgcacctggacggcgaggacgtggccatggcccacgccgacgccctggacgacttcgacctggacatgctgggcgacggcgacagccccggccccggcttcaccccccacgacagcgccccctacggcgccctggacatggccgacttcgagttcgagcagatgttcaccgacgccctgggcatcgacgagtacggcggcgaattcgagatgcccgtggacaggattctggaggccgaactcgccgtggagcagaaaagcgaccagggcgtggagggccccggcggaaccggcggcagcggcagcagccccaacgaccccgtgaccaacatctgccaggccgccgacaagcagctgttcaccctggtggagtgggccaagaggattccccacttcagcagcctgcccctggacgaccaggtgatcctgctgagggccggatggaacgagctgctgatcgccagcttcagccacaggagcatcgacgtgagggacggcatcctgctggccaccggcctgcacgtccataggaacagcgcccacagcgccggagtgggcgccatcttcgacagggtgctgaccgagctggtgagcaagatgagggacatgaggatggacaagaccgagctgggctgcctgagggccatcatcctgttcaaccccgaggtgaggggcctgaaaagcgcccaggaggtggagctgctgagggagaaggtgtacgccgccctggaggagtacaccaggaccacccaccccgacgagcccggcagattcgccaagctgctgctgaggctgcccagcctgaggagcatcggcctgaagtgcctggagcacctgttcttcttcaggctgatcggcgacgtgcccatcgacaccttcctgatggagatgctggagagccccagcgacagctgagcatgcactagttttataatttcttcttccagaatttctgacattttataatttcttcttccagaagactcacaacctccatatggccaccatgaagctgctgagcagcatcgagcaggcttgcgacatctgcaggctgaagaagctgaagtgcagcaaggagaagcccaagtgcgccaagtgcctgaagaacaactgggagtgcagatacagccccaagaccaagaggagccccctgaccagggcccacctgaccgaggtggagagcaggctggagaggctggagcagctgttcctgctgatcttccccagggaggacctggacatgatcctgaagatggacagcctgcaagacatcaaggccctgctgaccggcctgttcgtgcaggacaacgtgaacaaggacgccgtgaccgacaggctggccagcgtggagaccgacatgcccctgaccctgaggcagcacaggatcagcgccaccagcagcagcgaggagagcagcaacaagggccagaggcagctgaccgtgagccccgagtttcccgggatcaggcccgagtgcgtggtgcccgagacccagtgcgccatgaaaaggaaggagaagaaggcccagaaggagaaggacaagctgcccgtgagcaccaccaccgtcgatgaccacatgccccccatcatgcagtgcgagccccccccccccgaggccgccaggattcacgaggtcgtgcccaggttcctgagcgacaagctgctggtgaccaacaggcagaagaacatcccccagctgaccgccaaccagcagttcctgatcgccaggctgatctggtatcaggacggctacgagcagcccagcgacgaggacctgaaaaggatcacccagacctggcagcaggccgacgacgagaacgaggagagcgacacccccttcaggcagatcaccgagatgaccatcctgaccgtgcagctgatcgtggagttcgccaagggcctgcccggattcgccaagatcagccagcccgaccagatcaccctgctgaaggcttgcagcagcgaggtgatgatgctgagggtggccaggaggtacgacgccgccagcgacagcatcctgttcgccaacaaccaggcttacaccagggacaactacaggaaggctggcatggccgaggtgatcgaggacctcctgcacttctgcagatgtatgtacagcatggccctggacaacatccactacgccctgctgaccgccgtggtgatcttcagcgacaggcccggcctggagcagccccagctggtggaggagatccagaggtactacctgaacaccctgaggatctacatcctgaaccagctgagcggcagcgccaggagcagcgtgatctacggcaagatcctgagcatcctgagcgagctgaggaccctgggaatgcagaacagcaatatgtgtatcagcctgaagctgaagaacaggaagctgccccccttcctggaggagatttgggacgtggccgacatgagccacacccagcccccccccatcctggagagccccaccaacctgtgaaacttgtttattgcagcttataatggttacaaataaagcaatagcatcacaaatttcacaaataaagcatttttttcactgcattctagttgtggtttgtccaaactcatcaatgtatcttatcatgtctgg

SEQ ID NO: 142 - DNA, 3155 bp, synthetic construct
  misc_feature 1..3155: note = source = /note="Description of Artificial Sequence: Synthetic polynucleotide"
  misc_feature 1..3155: note = source = /note="FLC-2A7-1"
  source 1..3155: mol_type = other DNA
attgttcggagcagtgcggcgcgtttagcggagtactgtcctccgatattaatcggggcagactattccggggtttaccggcgcactctcgcccgaacttcaccggcggtctttcgtccgtgctttatcggggcggatcactccgaaccccgggaggtctatataagcagagctcgtttagtgaaccctcattctggagacggatcccgagccgagtgttttgacctccatagaacagccgctaaatccaaggtaaggtcagaagagctagcgccaccatgctgctgctggtgaccagcctgctgctgtgtgagctgccccaccccgcctttctgctgatccccgacatccagatgacccagaccacctccagcctgagcgccagcctgggcgaccgggtgaccatcagctgccgggccagccaggacatcagcaagtacctgaactggtatcagcagaagcccgacggcaccgtcaagctgctgatctaccacaccagccggctgcacagcggcgtgcccagccggtttagcggcagcggctccggcaccgactacagcctgaccatctccaacctggagcaggaggacatcgccacctacttttgccagcagggcaacacactgccctacacctttggcggcggaacaaagctggagatcaccggcagcacctccggcagcggcaagcctggcagcggcgagggcagcaccaagggcgaggtgaagctgcaggagagcggccctggcctggtggcccccagccagagcctgagcgtgacctgtaccgtgtccggcgtgtccctgcccgactacggcgtgtcctggatccggcagccccctaggaagggcctggagtggctgggcgtgatctggggcagcgagaccacctactacaacagcgccctgaagagccggctgaccatcatcaaggacaacagcaagagccaggtgttcctgaagatgaacagcctgcagaccgacgacaccgccatctactactgtgccaagcactactactacggcggcagctacgccatggactactggggccagggcaccagcgtgaccgtgtccagcaagcccaccaccacccctgcccctagacctccaaccccagcccctacaatcgccagccagcccctgagcctgaggcccgaagcctgtagacctgccgctggcggagccgtgcacaccagaggcctggatttcgcctgcgacatctacatctgggcccctctggccggcacctgtggcgtgctgctgctgagcctggtcatcaccctgtactgcaaccaccggaataggagcaagcggagcagaggcggccacagcgactacatgaacatgaccccccggaggcctggccccacccggaagcactaccagccctacgcccctcccagggacttcgccgcctaccggagccgggtgaagttcagccggagcgccgacgcccctgcctaccagcagggccagaaccagctgtacaacgagctgaacctgggccggagggaggagtacgacgtgctggacaagcggagaggccgggaccctgagatgggcggcaagccccggagaaagaaccctcaggagggcctgtataacgaactgcagaaagacaagatggccgaggcctacagcgagatcggcatgaagggcgagcggcggaggggcaagggccacgacggcctgtaccagggcctgagcaccgccaccaaggatacctacgacgccctgcacatgcaggccctgccccccagaagagctaagaggggaagcggagagggcagaggaagtctgctaacatgcggtgacgtcgaggagaatcctggacctgattggacctggattctgtttctggtggccgctgccacaagagtgcacagcaactgggtgaatgtgatcagcgacctgaagaagatcgaggatctgatccagagcatgcacattgatgccaccctgtacacagaatctgatgtgcaccctagctgtaaagtgaccgccatgaagtgttttctgctggagctgcaggtgatttctctggaaagcggagatgcctctatccacgacacagtggagaatctgatcatcctggccaacaatagcctgagcagcaatggcaatgtgacagagtctggctgtaaggagtgtgaggagctggaggagaagaacatcaaggagtttctgcagagctttgtgcacatcgtgcagatgttcatcaatacaagctctggcggaggatctggaggaggcggatctggaggaggaggcagtggaggcggaggatctggcggaggatctctgcagattacatgccctcctccaatgtctgtggagcacgccgatatttgggtgaagtcctacagcctgtacagcagagagagatacatctgcaacagcggctttaagagaaaggccggcacctcttctctgacagagtgcgtgctgaataaggccacaaatgtggcccactggacaacacctagcctgaagtgcattagagatcctgccctggtccaccagaggcctgcccctccatctacagtgacaacagccggagtgacacctcagcctgaatctctgagcccttctggaaaagaacctgccgccagctctcctagctctaataataccgccgccacaacagccgccattgtgcctggatctcagctgatgcctagcaagtctcctagcacaggcacaacagagatcagcagccacgaatcttctcacggaacaccttctcagaccaccgccaagaattgggagctgacagcctctgcctctcaccagcctccaggagtgtatcctcagggccactctgatacaacagtggccatcagcacatctacagtgctgctgtgtggactgtctgccgtgtctctgctggcctgttacctgaagtctagacagacacctcctctggcctctgtggagatggaggccatggaagccctgcctgtgacatggggaacaagcagcagagatgaggacctggagaattgttctcaccacctgtgaaacttgtttattgcagcttataatggttacaaataaagcaatagcatcacaaatttcacaaataaagcatttttttcactgcattctagttgtggtttgtccaaactcatcaatgtatcttatcatgtctgg

SEQ ID NO: 143 - DNA, 3476 bp, synthetic construct
  misc_feature 1..3476: note = source = /note="Description of Artificial Sequence: Synthetic polynucleotide"
  misc_feature 1..3476: note = source = /note="FLC-2A5-2"
  source 1..3476: mol_type = other DNA
attgttcggagcagtgcggcgcgtttagcggagtactgtcctccgatattaatcggggcagactattccggggtttaccggcgcactctcgcccgaacttcaccggcggtctttcgtccgtgctttatcggggcggatcactccgaaccccgggaggtctatataagcagagctcgtttagtgaaccctcattctggagacggatcccgagccgagtgttttgacctccatagaacagccgctaaatccaaggtaaggtcagaagagctagcgccaccatggattggacctggattctgtttctggtggccgctgccacaagagtgcacagcaactgggtgaatgtgatcagcgacctgaagaagatcgaggatctgatccagagcatgcacattgatgccaccctgtacacagaatctgatgtgcaccctagctgtaaagtgaccgccatgaagtgttttctgctggagctgcaggtgatttctctggaaagcggagatgcctctatccacgacacagtggagaatctgatcatcctggccaacaatagcctgagcagcaatggcaatgtgacagagtctggctgtaaggagtgtgaggagctggaggagaagaacatcaaggagtttctgcagagctttgtgcacatcgtgcagatgttcatcaatacaagctctggcggaggatctggaggaggcggatctggaggaggaggcagtggaggcggaggatctggcggaggatctctgcagattacatgccctcctccaatgtctgtggagcacgccgatatttgggtgaagtcctacagcctgtacagcagagagagatacatctgcaacagcggctttaagagaaaggccggcacctcttctctgacagagtgcgtgctgaataaggccacaaatgtggcccactggacaacacctagcctgaagtgcattagagatcctgccctggtccaccagaggcctgcccctccatctacagtgacaacagccggagtgacacctcagcctgaatctctgagcccttctggaaaagaacctgccgccagctctcctagctctaataataccgccgccacaacagccgccattgtgcctggatctcagctgatgcctagcaagtctcctagcacaggcacaacagagatcagcagccacgaatcttctcacggaacaccttctcagaccaccgccaagaattgggagctgacagcctctgcctctcaccagcctccaggagtgtatcctcagggccactctgatacaacagtggccatcagcacatctacagtgctgctgtgtggactgtctgccgtgtctctgctggcctgttacctgaagtctagacagacacctcctctggcctctgtggagatggaggccatggaagccctgcctgtgacatggggaacaagcagcagagatgaggacctggagaattgttctcaccacctgtgaatcgattaatctagcggccctagacgagcagacatgataagatacattgatgagtttggacaaaccacaactagaatgcagtgaaaaaaatgctttatttgtgaaatttgtgatgctattgctttatttgtaaccattataagctgcaataaacaagttaacaacaacaattgcattcattttatgtttcaggttcagggggagatgtgggaggttttttaaagcaagtaaaacctctacaaatgtggtaaaatccgataagcgtacctagaggccgcctagagattcgtgggggactcgaggataggcggcggttgggtgtgcgacatgtccgccacatcccagatctcctcgaggaaaggcggcagctttctgttcttgagcttgagggagatgcacatgttggagttttgcatgccgagcgtgcgtagctcagagaggattgagaggatcttgccgtatatgacggacgaacgcgccgacccgctcagctggttcaggatatagatgcggagcgtattcaggtagtaccgctggatctcttccaccagttgcggctgctccaaccctggccggtcagaaaagatgacgacagccgtgagcagcgcgtaatggatgttgtccaacgccatagagtacatgcaccggcagaagtgcagtagatcctcgatgacctcggccatgccagccttgcggtagttgtcgcgagtgtacgcttggttgttcgcgaacagaatactgtctgaggccgcatcgtatcgtcgcgcgactcggagcatcattacctcacttgagcaagccttaagcagcgtaatttgatcaggctgcgagatcttggcgaaccctggcaatcccttcgcgaactccacgataagttggaccgtgaggatagtcatctctgtgatctggcggaagggagtgtccgactcttcgttttcatcgtccgcttgctgccacgtctgcgtaatcctcttcaaatcttcatcagaaggctgctcgtacccgtcctggtaccagatgagcctggcgataaggaactgctggttggctgtcaactgggggatgtttttctgccggtttgtcaccaacagcttgtcggagagaaaccttgggaccacttcgtgaatccttgctgcttcaggaggtggaggttcacactgcataatgggcggcatgtggtcgtccaccgtcgtcgtgctgacaggcagtttgtccttctccttctgtgctttcttctctttccgcttcatggcgcactgagtctcgggtactacgcactcaggccgcccgggaaactcggggctcacggtcagctgcctctggcccttgttgctgctctcctcgctgctgctggtggcgctgatcctgtgctgcctcagggtcaggggcatgtcggtctccacgctggccagcctgtcggtcacggcgtccttgttcacgttgtcctgcacgaacaggccggtcagcagggccttgatgtcttgcaggctgtccatcttcaggatcatgtccaggtcctccctggggaagatcagcaggaacagctgctccagcctctccagcctgctctccacctcggtcaggtgggccctggtcagggggctcctcttggtcttggggctgtatctgcactcccagttgttcttcaggcacttggcgcacttgggcttctccttgctgcacttcagcttcttcagcctgcagatgtcgcaagcctgctcgatgctgctcagcagcttcatggtggcccgaaaagcacacaatgcctgtgttctggcggcaaacccgttgcgaaaaagaacgttcacggcgactactgcacttatatacggttctcccccaccctcgggaaaaaggcggagccagtacacgacatcactttcccagtttaccccgcgccaccttctctaggcaccggttcaatcgccgaccccctccccccaacttctcggggactgtgggcgatgtgcgctctgcccactgacgggcaccggagcctcacgcacgctc

SEQ ID NO: 144 - DNA, 3503 bp, synthetic construct
  misc_feature 1..3503: note = source = /note="Description of Artificial Sequence: Synthetic polynucleotide"
  misc_feature 1..3503: note = source = /note="FLC-2A6-1"
  source 1..3503: mol_type = other DNA
gagcgtgcgtgaggctccggtgcccgtcagtgggcagagcgcacatcgcccacagtccccgagaagttggggggagggggtcggcgattgaaccggtgcctagagaaggtggcgcggggtaaactgggaaagtgatgtcgtgtactggctccgcctttttcccgagggtgggggagaaccgtatataagtgcagtagtcgccgtgaacgttctttttcgcaacgggtttgccgccagaacacagcagccgctaaatccaaggtaaggtcagaagagctagcgccaccatgctgctgctggtgaccagcctgctgctgtgtgagctgccccaccccgcctttctgctgatccccgacatccagatgacccagaccacctccagcctgagcgccagcctgggcgaccgggtgaccatcagctgccgggccagccaggacatcagcaagtacctgaactggtatcagcagaagcccgacggcaccgtcaagctgctgatctaccacaccagccggctgcacagcggcgtgcccagccggtttagcggcagcggctccggcaccgactacagcctgaccatctccaacctggagcaggaggacatcgccacctacttttgccagcagggcaacacactgccctacacctttggcggcggaacaaagctggagatcaccggcagcacctccggcagcggcaagcctggcagcggcgagggcagcaccaagggcgaggtgaagctgcaggagagcggccctggcctggtggcccccagccagagcctgagcgtgacctgtaccgtgtccggcgtgtccctgcccgactacggcgtgtcctggatccggcagccccctaggaagggcctggagtggctgggcgtgatctggggcagcgagaccacctactacaacagcgccctgaagagccggctgaccatcatcaaggacaacagcaagagccaggtgttcctgaagatgaacagcctgcagaccgacgacaccgccatctactactgtgccaagcactactactacggcggcagctacgccatggactactggggccagggcaccagcgtgaccgtgtccagcaagcccaccaccacccctgcccctagacctccaaccccagcccctacaatcgccagccagcccctgagcctgaggcccgaagcctgtagacctgccgctggcggagccgtgcacaccagaggcctggatttcgcctgcgacatctacatctgggcccctctggccggcacctgtggcgtgctgctgctgagcctggtcatcaccctgtactgcaaccaccggaataggagcaagcggagcagaggcggccacagcgactacatgaacatgaccccccggaggcctggccccacccggaagcactaccagccctacgcccctcccagggacttcgccgcctaccggagccgggtgaagttcagccggagcgccgacgcccctgcctaccagcagggccagaaccagctgtacaacgagctgaacctgggccggagggaggagtacgacgtgctggacaagcggagaggccgggaccctgagatgggcggcaagccccggagaaagaaccctcaggagggcctgtataacgaactgcagaaagacaagatggccgaggcctacagcgagatcggcatgaagggcgagcggcggaggggcaagggccacgacggcctgtaccagggcctgagcaccgccaccaaggatacctacgacgccctgcacatgcaggccctgccccccagatgaatcgattaatctagcggccctagacgagcagacatgataagatacattgatgagtttggacaaaccacaactagaatgcagtgaaaaaaatgctttatttgtgaaatttgtgatgctattgctttatttgtaaccattataagctgcaataaacaagttaacaacaacaattgcattcattttatgtttcaggttcagggggagatgtgggaggttttttaaagcaagtaaaacctctacaaatgtggtaaaatccgataagcgtacctagaggctcacaggtggtgagaacaattctccaggtcctcatctctgctgcttgttccccatgtcacaggcagggcttccatggcctccatctccacagaggccagaggaggtgtctgtctagacttcaggtaacaggccagcagagacacggcagacagtccacacagcagcactgtagatgtgctgatggccactgttgtatcagagtggccctgaggatacactcctggaggctggtgagaggcagaggctgtcagctcccaattcttggcggtggtctgagaaggtgttccgtgagaagattcgtggctgctgatctctgttgtgcctgtgctaggagacttgctaggcatcagctgagatccaggcacaatggcggctgttgtggcggcggtattattagagctaggagagctggcggcaggttcttttccagaagggctcagagattcaggctgaggtgtcactccggctgttgtcactgtagatggaggggcaggcctctggtggaccagggcaggatctctaatgcacttcaggctaggtgttgtccagtgggccacatttgtggccttattcagcacgcactctgtcagagaagaggtgccggcctttctcttaaagccgctgttgcagatgtatctctctctgctgtacaggctgtaggacttcacccaaatatcggcgtgctccacagacattggaggagggcatgtaatctgcagagatcctccgccagatcctccgcctccactgcctcctcctccagatccgcctcctccagatcctccgccagagcttgtattgatgaacatctgcacgatgtgcacaaagctctgcagaaactccttgatgttcttctcctccagctcctcacactccttacagccagactctgtcacattgccattgctgctcaggctattgttggccaggatgatcagattctccactgtgtcgtggatagaggcatctccgctttccagagaaatcacctgcagctccagcagaaaacacttcatggcggtcactttacagctagggtgcacatcagattctgtgtacagggtggcatcaatgtgcatgctctggatcagatcctcgatcttcttcaggtcgctgatcacattcacccagttgctgtgcactcttgtggcagcggccaccagaaacagaatccaggtccaatccatggtggcgctagcccgaaaagcacacaatgcttctatggaggtcaaaacactcggctcgggatccgtctccagaatgagggttcactaaacgagctctgcttatatagacctcccggggttcggagtgatccgccccgataaagcacggacgaaagaccgccggtgaagttcgggcgagagtgcgccggtaaaccccggaatagtctgccccgattaatatcggaggacagtactccgctaaacgcgccgcactgctccgaacaat

SEQ ID NO: 145 - DNA, 4079 bp, synthetic construct
  misc_feature 1..4079: note = source = /note="Description of Artificial Sequence: Synthetic polynucleotide"
  misc_feature 1..4079: note = source = /note="XON-00(h)"
  source 1..4079: mol_type = other DNA
gagcgtgcgtgaggctccggtgcccgtcagtgggcagagcgcacatcgcccacagtccccgagaagttggggggagggggtcggcgattgaaccggtgcctagagaaggtggcgcggggtaaactgggaaagtgatgtcgtgtactggctccgcctttttcccgagggtgggggagaaccgtatataagtgcagtagtcgccgtgaacgttctttttcgcaacgggtttgccgccagaacacagcagccgctaaatccaaggtaaggtcagaagagctagcgccaccatgctgctgctggtgaccagcctgctgctgtgtgagctgccccaccccgcctttctgctgatccccgacatccagatgacccagaccacctccagcctgagcgccagcctgggcgaccgggtgaccatcagctgccgggccagccaggacatcagcaagtacctgaactggtatcagcagaagcccgacggcaccgtcaagctgctgatctaccacaccagccggctgcacagcggcgtgcccagccggtttagcggcagcggctccggcaccgactacagcctgaccatctccaacctggagcaggaggacatcgccacctacttttgccagcagggcaacacactgccctacacctttggcggcggaacaaagctggagatcaccggcagcacctccggcagcggcaagcctggcagcggcgagggcagcaccaagggcgaggtgaagctgcaggagagcggccctggcctggtggcccccagccagagcctgagcgtgacctgtaccgtgtccggcgtgtccctgcccgactacggcgtgtcctggatccggcagccccctaggaagggcctggagtggctgggcgtgatctggggcagcgagaccacctactacaacagcgccctgaagagccggctgaccatcatcaaggacaacagcaagagccaggtgttcctgaagatgaacagcctgcagaccgacgacaccgccatctactactgtgccaagcactactactacggcggcagctacgccatggactactggggccagggcaccagcgtgaccgtgtccagcaagcccaccaccacccctgcccctagacctccaaccccagcccctacaatcgccagccagcccctgagcctgaggcccgaagcctgtagacctgccgctggcggagccgtgcacaccagaggcctggatttcgcctgcgacatctacatctgggcccctctggccggcacctgtggcgtgctgctgctgagcctggtcatcaccctgtactgcaaccaccggaataggagcaagcggagcagaggcggccacagcgactacatgaacatgaccccccggaggcctggccccacccggaagcactaccagccctacgcccctcccagggacttcgccgcctaccggagccgggtgaagttcagccggagcgccgacgcccctgcctaccagcagggccagaaccagctgtacaacgagctgaacctgggccggagggaggagtacgacgtgctggacaagcggagaggccgggaccctgagatgggcggcaagccccggagaaagaaccctcaggagggcctgtataacgaactgcagaaagacaagatggccgaggcctacagcgagatcggcatgaagggcgagcggcggaggggcaagggccacgacggcctgtaccagggcctgagcaccgccaccaaggatacctacgacgccctgcacatgcaggccctgccccccagaagagctaagaggggaagcggagagggcagaggaagtctgctaacatgcggtgacgtcgaggagaatcctggacctatgcttctcctggtgacaagccttctgctctgtgagttaccacacccagcattcctcctgatcccacgcaaagtgtgtaacggaataggtattggtgaatttaaagactcactctccataaatgctacgaatattaaacacttcaaaaactgcacctccatcagtggcgatctccacatcctgccggtggcatttaggggtgactccttcacacatactcctcctctggatccacaggaactggatattctgaaaaccgtaaaggaaatcacagggtttttgctgattcaggcttggcctgaaaacaggacggacctccatgcctttgagaacctagaaatcatacgcggcaggaccaagcaacatggtcagttttctcttgcagtcgtcagcctgaacataacatccttgggattacgctccctcaaggagataagtgatggagatgtgataatttcaggaaacaaaaatttgtgctatgcaaatacaataaactggaaaaaactgtttgggacctccggtcagaaaaccaaaattataagcaacagaggtgaaaacagctgcaaggccacaggccaggtctgccatgccttgtgctcccccgagggctgctggggcccggagcccagggactgcgtctcttgccggaatgtcagccgaggcagggaatgcgtggacaagtgcaaccttctggagggtgagccaagggagtttgtggagaactctgagtgcatacagtgccacccagagtgcctgcctcaggccatgaacatcacctgcacaggacggggaccagacaactgtatccagtgtgcccactacattgacggcccccactgcgtcaagacctgcccggcaggagtcatgggagaaaacaacaccctggtctggaagtacgcagacgccggccatgtgtgccacctgtgccatccaaactgcacctacggatgcactgggccaggtcttgaaggctgtccaacgaatgggcctaagatcccgtccatcgccactgggatggtgggggccctcctcttgctgctggtggtggccctggggatcggcctcttcatggagggcagaggaagtctgctaacatgcggtgacgtcgaggagaatcctggacctatgggccccaagaagaaaaggaaggtggccccccccaccgacgtgagcctgggcgacgagctgcacctggacggcgaggacgtggccatggcccacgccgacgccctggacgacttcgacctggacatgctgggcgacggcgacagccccggccccggcttcaccccccacgacagcgccccctacggcgccctggacatggccgacttcgagttcgagcagatgttcaccgacgccctgggcatcgacgagtacggcggcgaattcgagatgcccgtggacaggattctggaggccgaactcgccgtggagcagaaaagcgaccagggcgtggagggccccggcggaaccggcggcagcggcagcagccccaacgaccccgtgaccaacatctgccaggccgccgacaagcagctgttcaccctggtggagtgggccaagaggattccccacttcagcagcctgcccctggacgaccaggtgatcctgctgagggccggatggaacgagctgctgatcgccagcttcagccacaggagcatcgacgtgagggacggcatcctgctggccaccggcctgcacgtccataggaacagcgcccacagcgccggagtgggcgccatcttcgacagggtgctgaccgagctggtgagcaagatgagggacatgaggatggacaagaccgagctgggctgcctgagggccatcatcctgttcaaccccgaggtgaggggcctgaaaagcgcccaggaggtggagctgctgagggagaaggtgtacgccgccctggaggagtacaccaggaccacccaccccgacgagcccggcagattcgccaagctgctgctgaggctgcccagcctgaggagcatcggcctgaagtgcctggagcacctgttcttcttcaggctgatcggcgacgtgcccatcgacaccttcctgatggagatgctggagagccccagcgacagctgaaacttgtttattgcagcttataatggttacaaataaagcaatagcatcacaaatttcacaaataaagcatttttttcactgcattctagttgtggtttgtccaaactcatcaatgtatcttatcatgtctgg

SEQ ID NO: 146 - protein, 18 aa, synthetic construct
  REGION 1..18: note = source = /note="Description of Artificial Sequence: Synthetic peptide"
  REGION 1..18: note = source = /note="Whitlow Linker"
GSTSGSGKPGSGEGSTKG

SEQ ID NO: 147 - protein, 26 aa, synthetic construct
  REGION 1..26: note = source = /note="Description of Artificial Sequence: Synthetic peptide"
  REGION 1..26: note = source = /note="Linker"
SGGGSGGGGSGGGGSGGGGSGGGSLQ

SEQ ID NO: 148 - skipped

SEQ ID NO: 149 - protein, 4 aa, synthetic construct
  REGION 1..4: note = source = /note="Description of Artificial Sequence: Synthetic peptide"
  REGION 1..4: note = source = /note="SGSG linker"
SGSG

SEQ ID NO: 150 - protein, 15 aa, synthetic construct
  REGION 1..15: note = source = /note="Description of Artificial Sequence: Synthetic peptide"
  REGION 1..15: note = source = /note="(G4S)3 linker"
GGGGSGGGGSGGGGS

SEQ ID NO: 151 - protein, 4 aa, synthetic construct
  REGION 1..4: note = source = /note="Description of Artificial Sequence: Synthetic peptide"
  REGION 1..4: note = source = /note="Furin cleavage site/ Furinlink1"
RAKR

SEQ ID NO: 152 - protein, 28 aa, Foot-and-mouth disease virus
  REGION 1..28: note = source = /note="Fmdv"
RAKRAPVKQTLNFDLLKLAGDVESNPGP

SEQ ID NO: 153 - protein, 18 aa, Thosea asigna virus
  REGION 1..18: note = source = /note="Thosea asigna virus 2A region (T2A)"
EGRGSLLTCGDVEENPGP

SEQ ID NO: 154 - protein, 25 aa, synthetic construct
  REGION 1..25: note = source = /note="Description of Artificial Sequence: Synthetic peptide"
  REGION 1..25: note = source = /note="Furin-GSG-T2A"
RAKRGSGEGRGSLLTCGDVEENPGP

SEQ ID NO: 155 - protein, 26 aa, synthetic construct
  REGION 1..26: note = source = /note="Description of Artificial Sequence: Synthetic peptide"
  REGION 1..26: note = source = /note="Furin-SGSG-T2A"
RAKRSGSGEGRGSLLTCGDVEENPGP

SEQ ID NO: 156 - protein, 19 aa, Porcine teschovirus
  REGION 1..19: note = source = /note="Porcine teschovirus-1 2A region (P2A)"
ATNFSLLKQAGDVEENPGP

SEQ ID NO: 157 - protein, 22 aa, synthetic construct
  REGION 1..22: note = source = /note="Description of Artificial Sequence: Synthetic peptide"
  REGION 1..22: note = source = /note="GSG-P2A"
GSGATNFSLLKQAGDVEENPGP

SEQ ID NO: 158 - protein, 20 aa, Equine rhinitis A virus
  REGION 1..20: note = source = /note="Equine rhinitis A virus 2A region (E2A)"
QCTNYALLKLAGDVESNPGP

SEQ ID NO: 159 - protein, 22 aa, Foot-and-mouth disease virus
  REGION 1..22: note = source = /note="Foot-and-mouth disease virus 2A region (F2A)"
VKQTLNFDLLKLAGDVESNPGP

SEQ ID NO: 160 - protein, 31 aa, synthetic construct
  REGION 1..31: note = source = /note="Description of Artificial Sequence: Synthetic polypeptide"
  REGION 1..31: note = source = /note="FP2A"
RAKRAPVKQGSGATNFSLLKQAGDVEENPGP

SEQ ID NO: 161 - protein, 8 aa, synthetic construct
  REGION 1..8: note = source = /note="Description of Artificial Sequence: Synthetic peptide"
  REGION 1..8: note = source = /note="Linker-GSG"
APVKQGSG

SEQ ID NO: 162 - protein, 5 aa, synthetic construct
  REGION 1..5: note = source = /note="Description of Artificial Sequence: Synthetic peptide"
  REGION 1..5: note = source = /note="Linker"
APVKQ

SEQ ID NO: 163 - protein, 22 aa, synthetic construct
  REGION 1..22: note = source = /note="Description of Artificial Sequence: Synthetic peptide"
  REGION 1..22: note = source = /note="GM-CSFR-alpha signal peptide"
MLLLVTSLLLCELPHPAFLLIP

SEQ ID NO: 164 - protein, 20 aa, synthetic construct
  REGION 1..20: note = source = /note="Description of Artificial Sequence: Synthetic peptide"
  REGION 1..20: note = source = /note="Ig Kappa signal peptide"
MRLPAQLLGLLMLWVPGSSG

SEQ ID NO: 165 - protein, 18 aa, synthetic construct
  REGION 1..18: note = source = /note="Description of Artificial Sequence: Synthetic peptide"
  REGION 1..18: note = source = /note="IgE signal peptide"
MDWTWILFLVAAATRVHS

SEQ ID NO: 166 - protein, 21 aa, synthetic construct
  REGION 1..21: note = source = /note="Description of Artificial Sequence: Synthetic peptide"
  REGION 1..21: note = source = /note="CD8-alpha signal peptide"
MALPVTALLLPLALLLHAARP

SEQ ID NO: 167 - protein, 21 aa, synthetic construct
  REGION 1..21: note = source = /note="Description of Artificial Sequence: Synthetic peptide"
  REGION 1..21: note = source = /note="TVB2(T21A)signal peptide"
MGTSLLCWMALCLLGADHADA

SEQ ID NO: 168 - protein, 24 aa, Homo sapiens
  REGION 1..24: note = source = /note="CD52 signal peptide"
MKRFLFLLLTISLLVMVQIQTGLS

SEQ ID NO: 169 - protein, 28 aa, synthetic construct
  REGION 1..28: note = source = /note="Description of Artificial Sequence: Synthetic peptide"
  REGION 1..28: note = source = /note="Low-affinity nerve growth factor receptor (LNGFR, TNFRSF16) signal peptide"
MGAGATGRAMDGPRLLLLLLLGVSLGGA

SEQ ID NO: 170 - protein, 47 aa, synthetic construct
  REGION 1..47: note = source = /note="Description of Artificial Sequence: Synthetic polypeptide"
  REGION 1..47: note = source = /note="CD8-alpha hinge region"
KPTTTPAPRPPTPAPTIASQPLSLRPEACRPAAGGAVHTRGLDFACD

SEQ ID NO: 171 - protein, 94 aa, synthetic construct
  REGION 1..94: note = source = /note="Description of Artificial Sequence: Synthetic polypeptide"
  REGION 1..94: note = source = /note="CD8 alpha 2x"
KPTTTPAPRPPTPAPTIASQPLSLRPEASRPAAGGAVHTRGLDFASDKPTTTPAPRPPTPAPTIASQPLSLRPEACRPAAGGAVHTRGLDFACD

SEQ ID NO: 172 - protein, 141 aa, synthetic construct
  REGION 1..141: note = source = /note="Description of Artificial Sequence: Synthetic polypeptide"
  REGION 1..141: note = source = /note="CD8 alpha 3x"
KPTTTPAPRPPTPAPTIASQPLSLRPEASRPAAGGAVHTRGLDFASDKPTTTPAPRPPTPAPTIASQPLSLRPEASRPAAGGAVHTRGLDFASDKPTTTPAPRPPTPAPTIASQPLSLRPEACRPAAGGAVHTRGLDFACD

SEQ ID NO: 173 - protein, 188 aa, synthetic construct
  REGION 1..188: note = source = /note="Description of Artificial Sequence: Synthetic polypeptide"
  REGION 1..188: note = source = /note="CD8 alpha 4x"
KPTTTPAPRPPTPAPTIASQPLSLRPEASRPAAGGAVHTRGLDFASDKPTTTPAPRPPTPAPTIASQPLSLRPEASRPAAGGAVHTRGLDFASDKPTTTPAPRPPTPAPTIASQPLSLRPEASRPAAGGAVHTRGLDFASDKPTTTPAPRPPTPAPTIASQPLSLRPEACRPAAGGAVHTRGLDFACD

SEQ ID NO: 174 - protein, 28 aa, synthetic construct
  REGION 1..28: note = source = /note="Description of Artificial Sequence: Synthetic peptide"
  REGION 1..28: note = source = /note="CD8-alpha TM domain"
IYIWAPLAGTCGVLLLSLVITLYCNHRN

SEQ ID NO: 175 - protein, 27 aa, synthetic construct
  REGION 1..27: note = source = /note="Description of Artificial Sequence: Synthetic peptide"
  REGION 1..27: note = source = /note="CD28 TM domain"
FWVLVVVGGVLACYSLLVTVAFIIFWV

SEQ ID NO: 176 - protein, 41 aa, synthetic construct
  REGION 1..41: note = source = /note="Description of Artificial Sequence: Synthetic polypeptide"
  REGION 1..41: note = source = /note="CD28 signaling domain"
RSKRSRGGHSDYMNMTPRRPGPTRKHYQPYAPPRDFAAYRS

SEQ ID NO: 177 - protein, 112 aa, synthetic construct
  REGION 1..112: note = source = /note="Description of Artificial Sequence: Synthetic polypeptide"
  REGION 1..112: note = source = /note="CD3 zeta signaling domain"
RVKFSRSADAPAYQQGQNQLYNELNLGRREEYDVLDKRRGRDPEMGGKPRRKNPQEGLYNELQKDKMAEAYSEIGMKGERRRGKGHDGLYQGLSTATKDTYDALHMQALPPR

SEQ ID NO: 178 - protein, 42 aa, synthetic construct
  REGION 1..42: note = source = /note="Description of Artificial Sequence: Synthetic polypeptide"
  REGION 1..42: note = source = /note="4-1BB signaling domain"
KRGRKKLLYIFKQPFMRPVQTTQEEDGCSCRFPEEEEGGCEL

SEQ ID NO: 179 - protein, 24 aa, synthetic construct
  REGION 1..24: note = source = /note="Description of Artificial Sequence: Synthetic peptide"
  REGION 1..24: note = source = /note="DNAX-activation protein 10 (DAP 10) Signaling Domain"
LCARPRRSPAQEDGKVYINMPGRG

SEQ ID NO: 180 - protein, 52 aa, synthetic construct
  REGION 1..52: note = source = /note="Description of Artificial Sequence: Synthetic polypeptide"
  REGION 1..52: note = source = /note="DNAX-activation protein 12 (DAP12) Signaling Domain"
YFLGRLVPRGRGAAEAATRKQRITETESPYQELQGQRSDVYSDLNTQRPYYK

SEQ ID NO: 181 - protein, 86 aa, synthetic construct
  REGION 1..86: note = source = /note="Description of Artificial Sequence: Synthetic polypeptide"
  REGION 1..86: note = source = /note="VP16 activation domain"
GPKKKRKVAPPTDVSLGDELHLDGEDVAMAHADALDDFDLDMLGDGDSPGPGFTPHDSAPYGALDMADFEFEQMFTDALGIDEYGG

SEQ ID NO: 182 - protein, 235 aa, synthetic construct
  REGION 1..235: note = source = /note="Description of Artificial Sequence: Synthetic polypeptide"
  REGION 1..235: note = source = /note="Retinoid x receptor (RxR)"
EMPVDRILEAELAVEQKSDQGVEGPGGTGGSGSSPNDPVTNICQAADKQLFTLVEWAKRIPHFSSLPLDDQVILLRAGWNELLIASFSHRSIDVRDGILLATGLHVHRNSAHSAGVGAIFDRVLTELVSKMRDMRMDKTELGCLRAIILFNPEVRGLKSAQEVELLREKVYAALEEYTRTTHPDEPGRFAKLLLRLPSLRSIGLKCLEHLFFFRLIGDVPIDTFLMEMLESPSDS

SEQ ID NO: 183 - protein, 323 aa, synthetic construct
  REGION 1..323: note = source = /note="Description of Artificial Sequence: Synthetic polypeptide"
  REGION 1..323: note = source = /note="VP16-linker-RxR"
GPKKKRKVAPPTDVSLGDELHLDGEDVAMAHADALDDFDLDMLGDGDSPGPGFTPHDSAPYGALDMADFEFEQMFTDALGIDEYGGEFEMPVDRILEAELAVEQKSDQGVEGPGGTGGSGSSPNDPVTNICQAADKQLFTLVEWAKRIPHFSSLPLDDQVILLRAGWNELLIASFSHRSIDVRDGILLATGLHVHRNSAHSAGVGAIFDRVLTELVSKMRDMRMDKTELGCLRAIILFNPEVRGLKSAQEVELLREKVYAALEEYTRTTHPDEPGRFAKLLLRLPSLRSIGLKCLEHLFFFRLIGDVPIDTFLMEMLESPSDS

SEQ ID NO: 184 - protein, 150 aa, synthetic construct
  REGION 1..150: note = source = /note="Description of Artificial Sequence: Synthetic polypeptide"
  REGION 1..150: note = source = /note="GAL4 DNA Binding Domain"
MKLLSSIEQACDICRLKKLKCSKEKPKCAKCLKNNWECRYSPKTKRSPLTRAHLTEVESRLERLEQLFLLIFPREDLDMILKMDSLQDIKALLTGLFVQDNVNKDAVTDRLASVETDMPLTLRQHRISATSSSEESSNKGQRQLTVSPEF

SEQ ID NO: 185 - protein, 336 aa, synthetic construct
  REGION 1..336: note = source = /note="Description of Artificial Sequence: Synthetic polypeptide"
  REGION 1..336: note = source = /note="Ecdysone Receptor Ligand Binding Domain - VY variant (EcR)"
IRPECVVPETQCAMKRKEKKAQKEKDKLPVSTTTVDDHMPPIMQCEPPPPEAARIHEVVPRFLSDKLLVTNRQKNIPQLTANQQFLIARLIWYQDGYEQPSDEDLKRITQTWQQADDENEESDTPFRQITEMTILTVQLIVEFAKGLPGFAKISQPDQITLLKACSSEVMMLRVARRYDAASDSILFANNQAYTRDNYRKAGMAEVIEDLLHFCRCMYSMALDNIHYALLTAVVIFSDRPGLEQPQLVEEIQRYYLNTLRIYILNQLSGSARSSVIYGKILSILSELRTLGMQNSNMCISLKLKNRKLPPFLEEIWDVADMSHTQPPPILESPTNL

SEQ ID NO: 186 - protein, 335 aa, synthetic construct
  REGION 1..335: note = source = /note="Description of Artificial Sequence: Synthetic polypeptide"
  REGION 1..335: note = source = /note="Ecdysone Receptor Ligand Binding Domain - VY variant (EcR)"
RPECVVPETQCAMKRKEKKAQKEKDKLPVSTTTVDDHMPPIMQCEPPPPEAARIHEVVPRFLSDKLLVTNRQKNIPQLTANQQFLIARLIWYQDGYEQPSDEDLKRITQTWQQADDENEESDTPFRQITEMTILTVQLIVEFAKGLPGFAKISQPDQITLLKACSSEVMMLRVARRYDAASDSILFANNQAYTRDNYRKAGMAEVIEDLLHFCRCMYSMALDNIHYALLTAVVIFSDRPGLEQPQLVEEIQRYYLNTLRIYILNQLSGSARSSVIYGKILSILSELRTLGMQNSNMCISLKLKNRKLPPFLEEIWDVADMSHTQPPPILESPTNL

SEQ ID NO: 187 - protein, 488 aa, synthetic construct
  REGION 1..488: note = source = /note="Description of Artificial Sequence: Synthetic polypeptide"
  REGION 1..488: note = source = /note="GAL4-Linker-EcR"
MKLLSSIEQACDICRLKKLKCSKEKPKCAKCLKNNWECRYSPKTKRSPLTRAHLTEVESRLERLEQLFLLIFPREDLDMILKMDSLQDIKALLTGLFVQDNVNKDAVTDRLASVETDMPLTLRQHRISATSSSEESSNKGQRQLTVSPEFPGIRPECVVPETQCAMKRKEKKAQKEKDKLPVSTTTVDDHMPPIMQCEPPPPEAARIHEVVPRFLSDKLLVTNRQKNIPQLTANQQFLIARLIWYQDGYEQPSDEDLKRITQTWQQADDENEESDTPFRQITEMTILTVQLIVEFAKGLPGFAKISQPDQITLLKACSSEVMMLRVARRYDAASDSILFANNQAYTRDNYRKAGMAEVIEDLLHFCRCMYSMALDNIHYALLTAVVIFSDRPGLEQPQLVEEIQRYYLNTLRIYILNQLSGSARSSVIYGKILSILSELRTLGMQNSNMCISLKLKNRKLPPFLEEIWDVADMSHTQPPPILESPTNL

SEQ ID NO: 188 - protein, 487 aa, synthetic construct
  REGION 1..487: note = source = /note="Description of Artificial Sequence: Synthetic polypeptide"
  REGION 1..487: note = source = /note="GAL4-Linker-EcR"
MKLLSSIEQACDICRLKKLKCSKEKPKCAKCLKNNWECRYSPKTKRSPLTRAHLTEVESRLERLEQLFLLIFPREDLDMILKMDSLQDIKALLTGLFVQDNVNKDAVTDRLASVETDMPLTLRQHRISATSSSEESSNKGQRQLTVSPEFPGRPECVVPETQCAMKRKEKKAQKEKDKLPVSTTTVDDHMPPIMQCEPPPPEAARIHEVVPRFLSDKLLVTNRQKNIPQLTANQQFLIARLIWYQDGYEQPSDEDLKRITQTWQQADDENEESDTPFRQITEMTILTVQLIVEFAKGLPGFAKISQPDQITLLKACSSEVMMLRVARRYDAASDSILFANNQAYTRDNYRKAGMAEVIEDLLHFCRCMYSMALDNIHYALLTAVVIFSDRPGLEQPQLVEEIQRYYLNTLRIYILNQLSGSARSSVIYGKILSILSELRTLGMQNSNMCISLKLKNRKLPPFLEEIWDVADMSHTQPPPILESPTNL

SEQ ID NO: 189 - protein, 335 aa, synthetic construct
  REGION 1..335: note = source = /note="Description of Artificial Sequence: Synthetic polypeptide"
  REGION 1..335: note = source = /note="Truncated EGFR (huEGFRt) (Her1t)"
RKVCNGIGIGEFKDSLSINATNIKHFKNCTSISGDLHILPVAFRGDSFTHTPPLDPQELDILKTVKEITGFLLIQAWPENRTDLHAFENLEIIRGRTKQHGQFSLAVVSLNITSLGLRSLKEISDGDVIISGNKNLCYANTINWKKLFGTSGQKTKIISNRGENSCKATGQVCHALCSPEGCWGPEPRDCVSCRNVSRGRECVDKCNLLEGEPREFVENSECIQCHPECLPQAMNITCTGRGPDNCIQCAHYIDGPHCVKTCPAGVMGENNTLVWKYADAGHVCHLCHPNCTYGCTGPGLEGCPTNGPKIPSIATGMVGALLLLLVVALGIGLFM

SEQ ID NO: 190 - protein, 244 aa, synthetic construct
  REGION 1..244: note = source = /note="Description of Artificial Sequence: Synthetic polypeptide"
  REGION 1..244: note = source = /note="EGFR truncated design 1 (Her1 truncated design 1) (HER1t1)"
RKVCNGIGIGEFKDSLSINATNIKHFKNCTSISGDLHILPVAFRGDSFTHTPPLDPQELDILKTVKEITGFLLIQAWPENRTDLHAFENLEIIRGRTKQHGQFSLAVVSLNITSLGLRSLKEISDGDVIISGNKNLCYANTINWKKLFGTSGQKTKIISNRGENSCKATGQVCHALCSPEGCWGPEPRDCVSGGGGSGGGGSGGGGSGGGGSFWVLVVVGGVLACYSLLVTVAFIIFWVRSKRS

SEQ ID NO: 191 - protein, 257 aa, synthetic construct
  REGION 1..257: note = source = /note="Description of Artificial Sequence: Synthetic polypeptide"
  REGION 1..257: note = source = /note="EGFR truncated design 2 (Her1 truncated design 2) (HER1t2)"
RKVCNGIGIGEFKDSLSINATNIKHFKNCTSISGDLHILPVAFRGDSFTHTPPLDPQELDILKTVKEITGFLLIQAWPENRTDLHAFENLEIIRGRTKQHGQFSLAVVSLNITSLGLRSLKEISDGDVIISGNKNLCYANTINWKKLFGTSGQKTKIISNRGENSCKATGQVCHALCSPEGCWGPEPRDCVSCRNVSRGRECVDKGGGGSGGGGSGGGGSGGGGSFWVLVVVGGVLACYSLLVTVAFIIFWVRSKRS

SEQ ID NO: 192 - protein, 276 aa, synthetic construct
  REGION 1..276: note = source = /note="Description of Artificial Sequence: Synthetic polypeptide"
  REGION 1..276: note = source = /note="EGFR truncated design 3 (Her1 truncated design 3) (HER1t3)"
RKVCNGIGIGEFKDSLSINATNIKHFKNCTSISGDLHILPVAFRGDSFTHTPPLDPQELDILKTVKEITGFLLIQAWPENRTDLHAFENLEIIRGRTKQHGQFSLAVVSLNITSLGLRSLKEISDGDVIISGNKNLCYANTINWKKLFGTSGQKTKIISNRGENSCKATGQVCHALCSPEGCWGPEPRDCVSCRNVSRGRECVDKCNLLEGEPREFVENSECIQGGGGSGGGGSGGGGSGGGGSFWVLVVVGGVLACYSLLVTVAFIIFWVRSKRS

SEQ ID NO: 193 - protein, 295 aa, synthetic construct
  REGION 1..295: note = source = /note="Description of Artificial Sequence: Synthetic polypeptide"
  REGION 1..295: note = source = /note="EGFR truncated design 4 (Her1 truncated design 4) (HER1t4)"
RKVCNGIGIGEFKDSLSINATNIKHFKNCTSISGDLHILPVAFRGDSFTHTPPLDPQELDILKTVKEITGFLLIQAWPENRTDLHAFENLEIIRGRTKQHGQFSLAVVSLNITSLGLRSLKEISDGDVIISGNKNLCYANTINWKKLFGTSGQKTKIISNRGENSCKATGQVCHALCSPEGCWGPEPRDCVSCRNVSRGRECVDKCNLLEGEPREFVENSECIQCHPECLPQAMNITCTGRGPDNCIQGGGGSGGGGSGGGGSFWVLVVVGGVLACYSLLVTVAFIIFWVRSKRS

SEQ ID NO: 194 - protein, 308 aa, synthetic construct
  REGION 1..308: note = source = /note="Description of Artificial Sequence: Synthetic polypeptide"
  REGION 1..308: note = source = /note="EGFR truncated design 5 (Her1 truncated design 5) (HER1t5)"
RKVCNGIGIGEFKDSLSINATNIKHFKNCTSISGDLHILPVAFRGDSFTHTPPLDPQELDILKTVKEITGFLLIQAWPENRTDLHAFENLEIIRGRTKQHGQFSLAVVSLNITSLGLRSLKEISDGDVIISGNKNLCYANTINWKKLFGTSGQKTKIISNRGENSCKATGQVCHALCSPEGCWGPEPRDCVSCRNVSRGRECVDKCNLLEGEPREFVENSECIQCHPECLPQAMNITCTGRGPDNCIQCAHYIDGPHCVKTGGGGSGGGGSGGGGSFWVLVVVGGVLACYSLLVTVAFIIFWVRSKRS

SEQ ID NO: 195 - protein, 328 aa, synthetic construct
  REGION 1..328: note = source = /note="Description of Artificial Sequence: Synthetic polypeptide"
  REGION 1..328: note = source = /note="EGFR truncated design 6 (Her1 truncated design 6) (HER1t6)"
RKVCNGIGIGEFKDSLSINATNIKHFKNCTSISGDLHILPVAFRGDSFTHTPPLDPQELDILKTVKEITGFLLIQAWPENRTDLHAFENLEIIRGRTKQHGQFSLAVVSLNITSLGLRSLKEISDGDVIISGNKNLCYANTINWKKLFGTSGQKTKIISNRGENSCKATGQVCHALCSPEGCWGPEPRDCVSCRNVSRGRECVDKCNLLEGEPREFVENSECIQCHPECLPQAMNITCTGRGPDNCIQCAHYIDGPHCVKTCPAGVMGENNTLVWKYADAGHVCHLGGGGSGGGGSFWVLVVVGGVLACYSLLVTVAFIIFWVRSKRS

SEQ ID NO: 196 - protein, 343 aa, synthetic construct
  REGION 1..343: note = source = /note="Description of Artificial Sequence: Synthetic polypeptide"
  REGION 1..343: note = source = /note="EGFR truncated design 7 (Her1 truncated design 7) (HER1t7)"
RKVCNGIGIGEFKDSLSINATNIKHFKNCTSISGDLHILPVAFRGDSFTHTPPLDPQELDILKTVKEITGFLLIQAWPENRTDLHAFENLEIIRGRTKQHGQFSLAVVSLNITSLGLRSLKEISDGDVIISGNKNLCYANTINWKKLFGTSGQKTKIISNRGENSCKATGQVCHALCSPEGCWGPEPRDCVSCRNVSRGRECVDKCNLLEGEPREFVENSECIQCHPECLPQAMNITCTGRGPDNCIQCAHYIDGPHCVKTCPAGVMGENNTLVWKYADAGHVCHLCHPNCTYGCTGPGLEGCPGGGGGGSFWVLVVVGGVLACYSLLVTVAFIIFWVRSKRS

SEQ ID NO: 197 - protein, 242 aa, synthetic construct
  REGION 1..242: note = source = /note="Description of Artificial Sequence: Synthetic polypeptide"
  REGION 1..242: note = source = /note="EGFR truncated design 8 (Her1 truncated design 8) (HER1t8)"
RKVCNGIGIGEFKDSLSINATNIKHFKNCTSISGDLHILPVAFRGDSFTHTPPLDPQELDILKTVKEITGFLLIQAWPENRTDLHAFENLEIIRGRTKQHGQFSLAVVSLNITSLGLRSLKEISDGDVIISGNKNLCYANTINWKKLFGTSGQKTKIISNRGENSCKATGQVCHALCSPEGCWGPEPRDCVSGGGGSGGGGSGGGGSGGGGSEITLIIFGVMAGVIGTILLISYGIRRGGGS

SEQ ID NO: 198 - protein, 239 aa, synthetic construct
  REGION 1..239: note = source = /note="Description of Artificial Sequence: Synthetic polypeptide"
  REGION 1..239: note = source = /note="EGFR truncated design 9 (Her1 truncated design 9) (HER1t9)"
RKVCNGIGIGEFKDSLSINATNIKHFKNCTSISGDLHILPVAFRGDSFTHTPPLDPQELDILKTVKEITGFLLIQAWPENRTDLHAFENLEIIRGRTKQHGQFSLAVVSLNITSLGLRSLKEISDGDVIISGNKNLCYANTINWKKLFGTSGQKTKIISNRGENSCKATGQVCHALCSPEGCWGPEPRDCVSGGGGSGGGGSGGGGSGGGGSITLIIFGVMAGVIGTILLISYGIGGGS

SEQ ID NO: 199 - protein, 239 aa, synthetic construct
  REGION 1..239: note = source = /note="Description of Artificial Sequence: Synthetic polypeptide"
  REGION 1..239: note = source = /note="EGFR truncated design 10 (Her1 truncated design 10) (HER1t10)"
RKVCNGIGIGEFKDSLSINATNIKHFKNCTSISGDLHILPVAFRGDSFTHTPPLDPQELDILKTVKEITGFLLIQAWPENRTDLHAFENLEIIRGRTKQHGQFSLAVVSLNITSLGLRSLKEISDGDVIISGNKNLCYANTINWKKLFGTSGQKTKIISNRGENSCKATGQVCHALCSPEGCWGPEPRDCVSGGGGSGGGGSGGGGSGGGGSITLIIFGVMAGVIGTILLALLIWGGGS

SEQ ID NO: 200 - protein, 237 aa, synthetic construct
  REGION 1..237: note = source = /note="Description of Artificial Sequence: Synthetic polypeptide"
  REGION 1..237: note = source = /note="EGFR truncated design 11 (Her1 truncated design 11) (HER1t11)"
RKVCNGIGIGEFKDSLSINATNIKHFKNCTSISGDLHILPVAFRGDSFTHTPPLDPQELDILKTVKEITGFLLIQAWPENRTDLHAFENLEIIRGRTKQHGQFSLAVVSLNITSLGLRSLKEISDGDVIISGNKNLCYANTINWKKLFGTSGQKTKIISNRGENSCKATGQVCHALCSPEGCWGPEPRDCVSGGGGSGGGGSGGGGSGGGGSLCYLLDGILFIYGVILTALFLGGGS

SEQ ID NO: 201 - protein, 297 aa, synthetic construct
  REGION 1..297: note = source = /note="Description of Artificial Sequence: Synthetic polypeptide"
  REGION 1..297: note = source = /note="FL CD20"
MTTPRNSVNGTFPAEPMKGPIAMQSGPKPLFRRMSSLVGPTQSFFMRESKTLGAVQIMNGLFHIALGGLLMIPAGIYAPICVTVWYPLWGGIMYIISGSLLAATEKNSRKCLVKGKMIMNSLSLFAAISGMILSIMDILNIKISHFLKMESLNFIRAHTPYINIYNCEPANPSEKNSPSTQYCYSIQSLFLGILSVMLIFAFFQELVIAGIVENEWKRTCSRPKSNIVLLSAEEKKEQTIEIKEEVVGLTETSSQPKNEEDIEIIPIQEEEEEETETNFPEPPQDQESSPIENDSSP

SEQ ID NO: 202 - protein, 263 aa, synthetic construct
  REGION 1..263: note = source = /note="Description of Artificial Sequence: Synthetic polypeptide"
  REGION 1..263: note = source = /note="Truncated CD20 design 1 (CD20t1) [CD20(M1-E263]"
MTTPRNSVNGTFPAEPMKGPIAMQSGPKPLFRRMSSLVGPTQSFFMRESKTLGAVQIMNGLFHIALGGLLMIPAGIYAPICVTVWYPLWGGIMYIISGSLLAATEKNSRKCLVKGKMIMNSLSLFAAISGMILSIMDILNIKISHFLKMESLNFIRAHTPYINIYNCEPANPSEKNSPSTQYCYSIQSLFLGILSVMLIFAFFQELVIAGIVENEWKRTCSRPKSNIVLLSAEEKKEQTIEIKEEVVGLTETSSQPKNEEDIE

SEQ ID NO: 203 - protein, 114 aa, synthetic construct
  REGION 1..114: note = source = /note="Description of Artificial Sequence: Synthetic polypeptide"
  REGION 1..114: note = source = /note="Interleukin-15"
NWVNVISDLKKIEDLIQSMHIDATLYTESDVHPSCKVTAMKCFLLELQVISLESGDASIHDTVENLIILANNSLSSNGNVTESGCKECEELEEKNIKEFLQSFVHIVQMFINTS

SEQ ID NO: 204 - protein, 237 aa, synthetic construct
  REGION 1..237: note = source = /note="Description of Artificial Sequence: Synthetic polypeptide"
  REGION 1..237: note = source = /note="Interleukin-15 receptor alpha"
ITCPPPMSVEHADIWVKSYSLYSRERYICNSGFKRKAGTSSLTECVLNKATNVAHWTTPSLKCIRDPALVHQRPAPPSTVTTAGVTPQPESLSPSGKEPAASSPSSNNTAATTAAIVPGSQLMPSKSPSTGTTEISSHESSHGTPSQTTAKNWELTASASHQPPGVYPQGHSDTTVAISTSTVLLCGLSAVSLLACYLKSRQTPPLASVEMEAMEALPVTWGTSSRDEDLENCSHHL

SEQ ID NO: 205 - protein, 395 aa, synthetic construct [sequence omitted]

SEQ ID NO: 206 - protein, 335 aa, Mus sp.
  REGION 1..335: note = source = /note="Murine Interleukin-12 subunit beta (p40)"
MCPQKLTISWFAIVLLVSPLMAMWELEKDVYVVEVDWTPDAPGETVNLTCDTPEEDDITWTSDQRHGVIGSGKTLTITVKEFLDAGQYTCHKGGETLSHSHLLLHKKENGIWSTEILKNFKNKTFLKCEAPNYSGRFTCSWLVQRNMDLKFNIKSSSSSPDSRAVTCGMASLSAEKVTLDQRDYEKYSVSCQEDVTCPTAEETLPIELALEARQQNKYENYSTSFFIRDIIKPDPPKNLQMKPLKNSQVEVSWEYPDSWSTPHSYFSLKFFVRIQRKKEKMKETEEGCNQKGAFLVEKTSTEVQCKGGNVCVQAQDRYYNSSCSKWACVPCRVRS

SEQ ID NO: 207 - protein, 215 aa, Mus sp.
  REGION 1..215: note = source = /note="Murine Interleukin-12 subunit alpha (p35)"
MCQSRYLLFLATLALLNHLSLARVIPVSGPARCLSQSRNLLKTTDDMVKTAREKLKHYSCTAEDIDHEDITRDQTSTLKTCLPLELHKNESCLATRETSSTTRGSCLPPQKTSLMMTLCLGSIYEDLKMYQTEFQAINAALQNHNHQQIILDKGMLVAIDELMQSLNHNGETLRQKPPVGEADPYRVKMKLCILLHAFSTRVVTINRVMGYLSSA

SEQ ID NO: 208 - protein, 535 aa, Mus sp.
  REGION 1..535: note = source = /note="Murine single chain IL-12 (p40-linker-p35)"
MCPQKLTISWFAIVLLVSPLMAMWELEKDVYVVEVDWTPDAPGETVNLTCDTPEEDDITWTSDQRHGVIGSGKTLTITVKEFLDAGQYTCHKGGETLSHSHLLLHKKENGIWSTEILKNFKNKTFLKCEAPNYSGRFTCSWLVQRNMDLKFNIKSSSSSPDSRAVTCGMASLSAEKVTLDQRDYEKYSVSCQEDVTCPTAEETLPIELALEARQQNKYENYSTSFFIRDIIKPDPPKNLQMKPLKNSQVEVSWEYPDSWSTPHSYFSLKFFVRIQRKKEKMKETEEGCNQKGAFLVEKTSTEVQCKGGNVCVQAQDRYYNSSCSKWACVPCRVRSGGGGGGSRVIPVSGPARCLSQSRNLLKTTDDMVKTAREKLKHYSCTAEDIDHEDITRDQTSTLKTCLPLELHKNESCLATRETSSTTRGSCLPPQKTSLMMTLCLGSIYEDLKMYQTEFQAINAALQNHNHQQIILDKGMLVAIDELMQSLNHNGETLRQKPPVGEADPYRVKMKLCILLHAFSTRVVTINRVMGYLSSA

SEQ ID NO: 209 - protein, 532 aa, Homo sapiens
  REGION 1..532: note = source = /note="Human single chain IL-12 (p40-linker-p35)"
MCHQQLVISWFSLVFLASPLVAIWELKKDVYVVELDWYPDAPGEMVVLTCDTPEEDGITWTLDQSSEVLGSGKTLTIQVKEFGDAGQYTCHKGGEVLSHSLLLLHKKEDGIWSTDILKDQKEPKNKTFLRCEAKNYSGRFTCWWLTTISTDLTFSVKSSRGSSDPQGVTCGAATLSAERVRGDNKEYEYSVECQEDSACPAAEESLPIEVMVDAVHKLKYENYTSSFFIRDIIKPDPPKNLQLKPLKNSRQVEVSWEYPDTWSTPHSYFSLTFCVQVQGKSKREKKDRVFTDKTSATVICRKNASISVRAQDRYYSSSWSEWASVPCSGGGGGGSRNLPVATPDPGMFPCLHHSQNLLRAVSNMLQKARQTLEFYPCTSEEIDHEDITKDKTSTVEACLPLELTKNESCLNSRETSFITNGSCLASRKTSFMMALCLSSIYEDLKMYQVEFKTMNAKLLMDPKRQIFLDQNMLAVIDELMQALNFNSETVPQKSSLEEPDFYKTKIKLCILLHAFRIRAVTIDRVMSYLNAS

SEQ ID NO: 210 - protein, 473 aa, synthetic construct
  REGION 1..473: note = source = /note="Description of Artificial Sequence: Synthetic polypeptide"
  REGION 1..473: note = source = /note="CD19-specific chimeric antigen receptor (CD19-CD8a-CD28-CD3z)"
DIQMTQTTSSLSASLGDRVTISCRASQDISKYLNWYQQKPDGTVKLLIYHTSRLHSGVPSRFSGSGSGTDYSLTISNLEQEDIATYFCQQGNTLPYTFGGGTKLEITGSTSGSGKPGSGEGSTKGEVKLQESGPGLVAPSQSLSVTCTVSGVSLPDYGVSWIRQPPRKGLEWLGVIWGSETTYYNSALKSRLTIIKDNSKSQVFLKMNSLQTDDTAIYYCAKHYYYGGSYAMDYWGQGTSVTVSSKPTTTPAPRPPTPAPTIASQPLSLRPEACRPAAGGAVHTRGLDFACDIYIWAPLAGTCGVLLLSLVITLYCNHRNRSKRSRGGHSDYMNMTPRRPGPTRKHYQPYAPPRDFAAYRSRVKFSRSADAPAYQQGQNQLYNELNLGRREEYDVLDKRRGRDPEMGGKPRRKNPQEGLYNELQKDKMAEAYSEIGMKGERRRGKGHDGLYQGLSTATKDTYDALHMQALPPR

SEQ ID NO: 211 - protein, 495 aa, synthetic construct
  REGION 1..495: note = source = /note="Description of Artificial Sequence: Synthetic polypeptide"
  REGION 1..495: note = source = /note="CD19-specific chimeric antigen receptor (CD19-CD8a-CD28-CD3z) with Signal peptide"
MLLLVTSLLLCELPHPAFLLIPDIQMTQTTSSLSASLGDRVTISCRASQDISKYLNWYQQKPDGTVKLLIYHTSRLHSGVPSRFSGSGSGTDYSLTISNLEQEDIATYFCQQGNTLPYTFGGGTKLEITGSTSGSGKPGSGEGSTKGEVKLQESGPGLVAPSQSLSVTCTVSGVSLPDYGVSWIRQPPRKGLEWLGVIWGSETTYYNSALKSRLTIIKDNSKSQVFLKMNSLQTDDTAIYYCAKHYYYGGSYAMDYWGQGTSVTVSSKPTTTPAPRPPTPAPTIASQPLSLRPEACRPAAGGAVHTRGLDFACDIYIWAPLAGTCGVLLLSLVITLYCNHRNRSKRSRGGHSDYMNMTPRRPGPTRKHYQPYAPPRDFAAYRSRVKFSRSADAPAYQQGQNQLYNELNLGRREEYDVLDKRRGRDPEMGGKPRRKNPQEGLYNELQKDKMAEAYSEIGMKGERRRGKGHDGLYQGLSTATKDTYDALHMQALPPR

SEQ ID NO: 212 - protein, 120 aa, synthetic construct
  REGION 1..120: note = source = /note="Description of Artificial Sequence: Synthetic polypeptide"
  REGION 1..120: note = source = /note="Anti-CD19 monoclonal antibody clone FMC63 variable heavy chain"
EVKLQESGPGLVAPSQSLSVTCTVSGVSLPDYGVSWIRQPPRKGLEWLGVIWGSETTYYNSALKSRLTIIKDNSKSQVFLKMNSLQTDDTAIYYCAKHYYYGGSYAMDYWGQGTSVTVSS

SEQ ID NO: 213 - protein, 245 aa, synthetic construct
  REGION 1..245: note = source = /note="Description of Artificial Sequence: Synthetic polypeptide"
  REGION 1..245: note = source = /note="Anti-CD19 clone FMC63 single chain fragment variable (scFv) with Whitlow linker"
DIQMTQTTSSLSASLGDRVTISCRASQDISKYLNWYQQKPDGTVKLLIYHTSRLHSGVPSRFSGSGSGTDYSLTISNLEQEDIATYFCQQGNTLPYTFGGGTKLEITGSTSGSGKPGSGEGSTKGEVKLQESGPGLVAPSQSLSVTCTVSGVSLPDYGVSWIRQPPRKGLEWLGVIWGSETTYYNSALKSRLTIIKDNSKSQVFLKMNSLQTDDTAIYYCAKHYYYGGSYAMDYWGQGTSVTVSS

SEQ ID NO: 214 - protein, 111 aa, synthetic construct
  REGION 1..111: note = source = /note="Description of Artificial Sequence: Synthetic polypeptide"
  REGION 1..111: note = source = /note="hM195 VL"
DIQMTQSPSSLSASVGDRVTITCRASESVDNYGISFMNWFQQKPGKAPKLLIYAASNQGSGVPSRFSGSGSGTDFTLTISSLQPDDFATYYCQQSKEVPWTFGQGTKVEIK

SEQ ID NO: 215 - protein, 116 aa, synthetic construct
  REGION 1..116: note = source = /note="Description of Artificial Sequence: Synthetic polypeptide"
  REGION 1..116: note = source = /note="hM195 VH"
QVQLVQSGAEVKKPGSSVKVSCKASGYTFTDYNMHWVRQAPGQGLEWIGYIYPYNGGTGYNQKFKSKATITADESTNTAYMELSSLRSEDTAVYYCARGRPAMDYWGQGTLVTVSS

SEQ ID NO: 216 - protein, 242 aa, synthetic construct
  REGION 1..242: note = source = /note="Description of Artificial Sequence: Synthetic polypeptide"
  REGION 1..242: note = source = /note="hM195 scFv with linker"
DIQMTQSPSSLSASVGDRVTITCRASESVDNYGISFMNWFQQKPGKAPKLLIYAASNQGSGVPSRFSGSGSGTDFTLTISSLQPDDFATYYCQQSKEVPWTFGQGTKVEIKGGGGSGGGGSGGGGSQVQLVQSGAEVKKPGSSVKVSCKASGYTFTDYNMHWVRQAPGQGLEWIGYIYPYNGGTGYNQKFKSKATITADESTNTAYMELSSLRSEDTAVYYCARGRPAMDYWGQGTLVTVSS

SEQ ID NO: 217 - protein, 943 aa, synthetic construct
  REGION 1..943: note = source = /note="Description of Artificial Sequence: Synthetic polypeptide"
  REGION 1..943: note = source = /note="EGFR variant III (EGFRvIII)"
MRPSGTAGAALLALLAALCPASRALEEKKGNYVVTDHGSCVRACGADSYEMEEDGVRKCKKCEGPCRKVCNGIGIGEFKDSLSINATNIKHFKNCTSISGDLHILPVAFRGDSFTHTPPLDPQELDILKTVKEITGFLLIQAWPENRTDLHAFENLEIIRGRTKQHGQFSLAVVSLNITSLGLRSLKEISDGDVIISGNKNLCYANTINWKKLFGTSGQKTKIISNRGENSCKATGQVCHALCSPEGCWGPEPRDCVSCRNVSRGRECVDKCNLLEGEPREFVENSECIQCHPECLPQAMNITCTGRGPDNCIQCAHYIDGPHCVKTCPAGVMGENNTLVWKYADAGHVCHLCHPNCTYGCTGPGLEGCPTNGPKIPSIATGMVGALLLLLVVALGIGLFMRRRHIVRKRTLRRLLQERELVEPLTPSGEAPNQALLRILKETEFKKIKVLGSGAFGTVYKGLWIPEGEKVKIPVAIKELREATSPKANKEILDEAYVMASVDNPHVCRLLGICLTSTVQLITQLMPFGCLLDYVREHKDNIGSQYLLNWCVQIAKGMNYLEDRRLVHRDLAARNVLVKTPQHVKITDFGLAKLLGAEEKEYHAEGGKVPIKWMALESILHRIYTHQSDVWSYGVTVWELMTFGSKPYDGIPASEISSILEKGERLPQPPICTIDVYMIMVKCWMIDADSRPKFRELIIEFSKMARDPQRYLVIQGDERMHLPSPTDSNFYRALMDEEDMDDVVDADEYLIPQQGFFSSPSTSRTPLLSSLSATSNNSTVACIDRNGLQSCPIKEDSFLQRYSSDPTGALTEDSIDDTFLPVPEYINQSVPKRPAGSVQNPVYHNQPLNPAPSRDPHYQDPHSTAVGNPEYLNTVQPTCVNSTFDSPAHWAQKGSHQISLDNPDYQQDFFPKEAKPNGIFKGSTAENAEYLRVAPQSSEFIGA

SEQ ID NO: 218 - protein, 116 aa, synthetic construct
  REGION 1..116: note = source = /note="Description of Artificial Sequence: Synthetic polypeptide"
  REGION 1..116: note = source = /note="Anti- EGFRvIII Clone 139 VH"
EVQVLESGGGLVQPGGSLRLSCAASGFTFSSYAMSWVRQAPGKGLEWVSAISGSGGSTNYADSVKGRFTISRDNSKNTLYLQMNSLRAEDTAVYYCAGSSGWSEYWGQGTLVTVSS

SEQ ID NO: 219 - protein, 107 aa, synthetic construct
  REGION 1..107: note = source = /note="Description of Artificial Sequence: Synthetic polypeptide"
  REGION 1..107: note = source = /note="Anti- EGFRvIII Clone 139 VL"
DIQMTQSPSSLSASVGDRVTITCRASQGIRNNLAWYQQKPGKAPKRLIYAASNLQSGVPSRFTGSGSGTEFTLIVSSLQPEDFATYYCLQHHSYPLTSGGGTKVEIK

SEQ ID NO: 220 - protein, 120 aa, synthetic construct
  REGION 1..120: note = source = /note="Description of Artificial Sequence: Synthetic polypeptide"
  REGION 1..120: note = source = /note="Anti- EGFRvIII Clone MR1 VH"
QVKLQQSGGGLVKPGASLKLSCVTSGFTFRKFGMSWVRQTSDKRLEWVASISTGGYNTYYSDNVKGRFTISRENAKNTLYLQMSSLKSEDTALYYCTRGYSSTSYAMDYWGQGTTVTVSS

SEQ ID NO: 221 - protein, 107 aa, synthetic construct
  REGION 1..107: note = source = /note="Description of Artificial Sequence: Synthetic polypeptide"
  REGION 1..107: note = source = /note="Anti- EGFRvIII Clone MR1 VL"
DIELTQSPASLSVATGEKVTIRCMTSTDIDDDMNWYQQKPGEPPKFLISEGNTLRPGVPSRFSSSGTGTDFVFTIENTLSEDVGDYYCLQSFNVPLTFGDGTKLEIK

SEQ ID NO: 222 - protein, 120 aa, synthetic construct
  REGION 1..120: note = source = /note="Description of Artificial Sequence: Synthetic polypeptide"
  REGION 1..120: note = source = /note="Anti- EGFRvIII Clone MR1-1 VH"
QVKLQQSGGGLVKPGASLKLSCVTSGFTFRKFGMSWVRQTSDKRLEWVASISTGGYNTYYSDNVKGRFTISRENAKNTLYLQMSSLKSEDTALYYCTRGYSPYSYAMDYWGQGTTVTVSS

SEQ ID NO: 223 - protein, 107 aa, synthetic construct
  REGION 1..107: note = source = /note="Description of Artificial Sequence: Synthetic polypeptide"
  REGION 1..107: note = source = /note="Anti- EGFRvIII Clone MR1-1 VL"
DIELTQSPASLSVATGEKVTIRCMTSTDIDDDMNWYQQKPGEPPKFLISEGNTLRPGVPSRFSSSGTGTDFVFTIENTLSEDVGDYYCLQSWNVPLTFGDGTKLEIK

SEQ ID NO: 224 - protein, 120 aa, synthetic construct
  REGION 1..120: note = source = /note="Description of Artificial Sequence: Synthetic polypeptide"
  REGION 1..120: note = source = /note="Anti- EGFRvIII Clone humMR1-1 VH"
QVQLQESGGGLVKPGGSLKLSCAASGFTFSKFGMSWVRQTPDKRLEWVASISTGGYNTYYSDNVKGRFTISRDNAKNTLYLQMSSLKSEDTAMYYCARGYSPYSYAMDYWGQGTMVTVSS

SEQ ID NO: 225 - protein, 107 aa, synthetic construct
  REGION 1..107: note = source = /note="Description of Artificial Sequence: Synthetic polypeptide"
  REGION 1..107: note = source = /note="Anti- EGFRvIII Clone humMR1-1 VL"
DIQMTQSPSSLSASVGDRVTITCMTSTDIDDDMNWYQQKPGKTPKLLIYEGNTLRPGVPSRFSGSGSGTDFIFTISSLQPEDIATYYCLQSWNVPLTFGGGTKVEIK

SEQ ID NO: 226 - protein, 120 aa, synthetic construct
  REGION 1..120: note = source = /note="Description of Artificial Sequence: Synthetic polypeptide"
  REGION 1..120: note = source = /note="Anti- EGFRvIII Clone humMR1-2 VH"
QVQLQESGGGLVKPGGSLKLSCAASGFTFSKFGMSWVRQTPDKRLEWVASISTGGYNTFYSDNVKGRFTISRDNAKNTLYLQMSSLKSEDTAMYYCARGYSPYSFAMDYWGQGTMVTVSS

SEQ ID NO: 227 - protein, 107 aa, synthetic construct; identical to SEQ ID NO: 225
  REGION 1..107: note = source = /note="Description of Artificial Sequence: Synthetic polypeptide"
  REGION 1..107: note = source = /note="Anti- EGFRvIII Clone humMR1-2 VL"

SEQ ID NO: 228 - protein, 241 aa, synthetic construct
  REGION 1..241: note = source = /note="Description of Artificial Sequence: Synthetic polypeptide"
  REGION 1..241: note = source = /note="Anti- EGFRvIII scFv Clone 139"
DIQMTQSPSSLSASVGDRVTITCRASQGIRNNLAWYQQKPGKAPKRLIYAASNLQSGVPSRFTGSGSGTEFTLIVSSLQPEDFATYYCLQHHSYPLTSGGGTKVEIKGSTSGSGKPGSGEGSTKGEVQVLESGGGLVQPGGSLRLSCAASGFTFSSYAMSWVRQAPGKGLEWVSAISGSGGSTNYADSVKGRFTISRDNSKNTLYLQMNSLRAEDTAVYYCAGSSGWSEYWGQGTLVTVSS

SEQ ID NO: 229 - protein, 242 aa, synthetic construct
  REGION 1..242: note = source = /note="Description of Artificial Sequence: Synthetic polypeptide"
  REGION 1..242: note = source = /note="Anti-EGFRvIII scFv clone MR1"
DIELTQSPASLSVATGEKVTIRCMTSTDIDDDMNWYQQKPGEPPKFLISEGNTLRPGVPSRFSSSGTGTDFVFTIENTLSEDVGDYYCLQSFNVPLTFGDGTKLEIKGGGGSGGGGSGGGGSQVKLQQSGGGLVKPGASLKLSCVTSGFTFRKFGMSWVRQTSDKRLEWVASISTGGYNTYYSDNVKGRFTISRENAKNTLYLQMSSLKSEDTALYYCTRGYSSTSYAMDYWGQGTTVTVSS

SEQ ID NO: 230 - protein, 242 aa, synthetic construct
  REGION 1..242: note = source = /note="Description of Artificial Sequence: Synthetic polypeptide"
  REGION 1..242: note = source = /note="Anti EGFRvIII scFv clone MR1-1"
DIELTQSPASLSVATGEKVTIRCMTSTDIDDDMNWYQQKPGEPPKFLISEGNTLRPGVPSRFSSSGTGTDFVFTIENTLSEDVGDYYCLQSWNVPLTFGDGTKLEIKGGGGSGGGGSGGGGSQVKLQQSGGGLVKPGASLKLSCVTSGFTFRKFGMSWVRQTSDKRLEWVASISTGGYNTYYSDNVKGRFTISRENAKNTLYLQMSSLKSEDTALYYCTRGYSPYSYAMDYWGQGTTVTVSS

SEQ ID NO: 231 - protein, 242 aa, synthetic construct
  REGION 1..242: note = source = /note="Description of Artificial Sequence: Synthetic polypeptide"
  REGION 1..242: note = source = /note="Anti-EGFRvIII scFv clone huMR1-1"
DIQMTQSPSSLSASVGDRVTITCMTSTDIDDDMNWYQQKPGKTPKLLIYEGNTLRPGVPSRFSGSGSGTDFIFTISSLQPEDIATYYCLQSWNVPLTFGGGTKVEIKGGGGSGGGGSGGGGSQVQLQESGGGLVKPGGSLKLSCAASGFTFSKFGMSWVRQTPDKRLEWVASISTGGYNTYYSDNVKGRFTISRDNAKNTLYLQMSSLKSEDTAMYYCARGYSPYSYAMDYWGQGTMVTVSS

SEQ ID NO: 232 - protein, 242 aa, synthetic construct
  REGION 1..242: note = source = /note="Description of Artificial Sequence: Synthetic polypeptide"
  REGION 1..242: note = source = /note="Anti-EGFRvIII scFv clone huMR1-2"
DIQMTQSPSSLSASVGDRVTITCMTSTDIDDDMNWYQQKPGKTPKLLIYEGNTLRPGVPSRFSGSGSGTDFIFTISSLQPEDIATYYCLQSWNVPLTFGGGTKVEIKGGGGSGGGGSGGGGSQVQLQESGGGLVKPGGSLKLSCAASGFTFSKFGMSWVRQTPDKRLEWVASISTGGYNTFYSDNVKGRFTISRDNAKNTLYLQMSSLKSEDTAMYYCARGYSPYSFAMDYWGQGTMVTVSS

SEQ ID NO: 233 - protein, 470 aa, synthetic construct
  REGION 1..470: note = source = /note="Description of Artificial Sequence: Synthetic polypeptide"
  REGION 1..470: note = source = /note="EGFRvIII CAR (clone 139 scFv.CD8alpha hinge &TM.4-1BB.CD3-zeta)"
DIQMTQSPSSLSASVGDRVTITCRASQGIRNNLAWYQQKPGKAPKRLIYAASNLQSGVPSRFTGSGSGTEFTLIVSSLQPEDFATYYCLQHHSYPLTSGGGTKVEIKGSTSGSGKPGSGEGSTKGEVQVLESGGGLVQPGGSLRLSCAASGFTFSSYAMSWVRQAPGKGLEWVSAISGSGGSTNYADSVKGRFTISRDNSKNTLYLQMNSLRAEDTAVYYCAGSSGWSEYWGQGTLVTVSSKPTTTPAPRPPTPAPTIASQPLSLRPEACRPAAGGAVHTRGLDFACDIYIWAPLAGTCGVLLLSLVITLYCNHRNKRGRKKLLYIFKQPFMRPVQTTQEEDGCSCRFPEEEEGGCELRVKFSRSADAPAYQQGQNQLYNELNLGRREEYDVLDKRRGRDPEMGGKPRRKNPQEGLYNELQKDKMAEAYSEIGMKGERRRGKGHDGLYQGLSTATKDTYDALHMQALPPR

SEQ ID NO: 234 - protein, 471 aa, synthetic construct
  REGION 1..471: note = source = /note="Description of Artificial Sequence: Synthetic polypeptide"
  REGION 1..471: note = source = /note="EGFRvIII CAR (MR1 scFv.CD8alpha hinge &TM.4-1BB.CD3-zeta)"
DIELTQSPASLSVATGEKVTIRCMTSTDIDDDMNWYQQKPGEPPKFLISEGNTLRPGVPSRFSSSGTGTDFVFTIENTLSEDVGDYYCLQSFNVPLTFGDGTKLEIKGGGGSGGGGSGGGGSQVKLQQSGGGLVKPGASLKLSCVTSGFTFRKFGMSWVRQTSDKRLEWVASISTGGYNTYYSDNVKGRFTISRENAKNTLYLQMSSLKSEDTALYYCTRGYSSTSYAMDYWGQGTTVTVSSKPTTTPAPRPPTPAPTIASQPLSLRPEACRPAAGGAVHTRGLDFACDIYIWAPLAGTCGVLLLSLVITLYCNHRNKRGRKKLLYIFKQPFMRPVQTTQEEDGCSCRFPEEEEGGCELRVKFSRSADAPAYQQGQNQLYNELNLGRREEYDVLDKRRGRDPEMGGKPRRKNPQEGLYNELQKDKMAEAYSEIGMKGERRRGKGHDGLYQGLSTATKDTYDALHMQALPPR

SEQ ID NO: 235 - protein, 471 aa, synthetic construct
  REGION 1..471: note = source = /note="Description of Artificial Sequence: Synthetic polypeptide"
  REGION 1..471: note = source = /note="EGFRvIII CAR (MR1-1 scFv.CD8alpha hinge &TM.4-1BB.CD3-zeta)"
DIELTQSPASLSVATGEKVTIRCMTSTDIDDDMNWYQQKPGEPPKFLISEGNTLRPGVPSRFSSSGTGTDFVFTIENTLSEDVGDYYCLQSWNVPLTFGDGTKLEIKGGGGSGGGGSGGGGSQVKLQQSGGGLVKPGASLKLSCVTSGFTFRKFGMSWVRQTSDKRLEWVASISTGGYNTYYSDNVKGRFTISRENAKNTLYLQMSSLKSEDTALYYCTRGYSPYSYAMDYWGQGTTVTVSSKPTTTPAPRPPTPAPTIASQPLSLRPEACRPAAGGAVHTRGLDFACDIYIWAPLAGTCGVLLLSLVITLYCNHRNKRGRKKLLYIFKQPFMRPVQTTQEEDGCSCRFPEEEEGGCELRVKFSRSADAPAYQQGQNQLYNELNLGRREEYDVLDKRRGRDPEMGGKPRRKNPQEGLYNELQKDKMAEAYSEIGMKGERRRGKGHDGLYQGLSTATKDTYDALHMQALPPR

SEQ ID NO: 236 - protein, 471 aa, synthetic construct
  REGION 1..471: note = source = /note="Description of Artificial Sequence: Synthetic polypeptide"
  REGION 1..471: note = source = /note="EGFRvIII CAR (humMR1-1 scFv.CD8alpha hinge &TM.4-1BB.CD3-zeta)"
DIQMTQSPSSLSASVGDRVTITCMTSTDIDDDMNWYQQKPGKTPKLLIYEGNTLRPGVPSRFSGSGSGTDFIFTISSLQPEDIATYYCLQSWNVPLTFGGGTKVEIKGGGGSGGGGSGGGGSQVQLQESGGGLVKPGGSLKLSCAASGFTFSKFGMSWVRQTPDKRLEWVASISTGGYNTYYSDNVKGRFTISRDNAKNTLYLQMSSLKSEDTAMYYCARGYSPYSYAMDYWGQGTMVTVSSKPTTTPAPRPPTPAPTIASQPLSLRPEACRPAAGGAVHTRGLDFACDIYIWAPLAGTCGVLLLSLVITLYCNHRNKRGRKKLLYIFKQPFMRPVQTTQEEDGCSCRFPEEEEGGCELRVKFSRSADAPAYQQGQNQLYNELNLGRREEYDVLDKRRGRDPEMGGKPRRKNPQEGLYNELQKDKMAEAYSEIGMKGERRRGKGHDGLYQGLSTATKDTYDALHMQALPPR

SEQ ID NO: 237 - protein, 471 aa, synthetic construct
  REGION 1..471: note = source = /note="Description of Artificial Sequence: Synthetic polypeptide"
  REGION 1..471: note = source = /note="EGFRvIII CAR (humMR1-2 scFv.CD8alpha hinge &TM.4-1BB.CD3-zeta)"
DIQMTQSPSSLSASVGDRVTITCMTSTDIDDDMNWYQQKPGKTPKLLIYEGNTLRPGVPSRFSGSGSGTDFIFTISSLQPEDIATYYCLQSWNVPLTFGGGTKVEIKGGGGSGGGGSGGGGSQVQLQESGGGLVKPGGSLKLSCAASGFTFSKFGMSWVRQTPDKRLEWVASISTGGYNTFYSDNVKGRFTISRDNAKNTLYLQMSSLKSEDTAMYYCARGYSPYSFAMDYWGQGTMVTVSSKPTTTPAPRPPTPAPTIASQPLSLRPEACRPAAGGAVHTRGLDFACDIYIWAPLAGTCGVLLLSLVITLYCNHRNKRGRKKLLYIFKQPFMRPVQTTQEEDGCSCRFPEEEEGGCELRVKFSRSADAPAYQQGQNQLYNELNLGRREEYDVLDKRRGRDPEMGGKPRRKNPQEGLYNELQKDKMAEAYSEIGMKGERRRGKGHDGLYQGLSTATKDTYDALHMQALPPR

SEQ ID NO: 238 - protein, 518 aa, synthetic construct
  REGION 1..518: note = source = /note="Description of Artificial Sequence: Synthetic polypeptide"
  REGION 1..518: note = source = /note="EGFRvIII CAR (MR1-1 scFv.CD8alpha 2x hinge &TM.4-1BB.CD3-zeta)"
DIELTQSPASLSVATGEKVTIRCMTSTDIDDDMNWYQQKPGEPPKFLISEGNTLRPGVPSRFSSSGTGTDFVFTIENTLSEDVGDYYCLQSWNVPLTFGDGTKLEIKGGGGSGGGGSGGGGSQVKLQQSGGGLVKPGASLKLSCVTSGFTFRKFGMSWVRQTSDKRLEWVASISTGGYNTYYSDNVKGRFTISRENAKNTLYLQMSSLKSEDTALYYCTRGYSPYSYAMDYWGQGTTVTVSSKPTTTPAPRPPTPAPTIASQPLSLRPEASRPAAGGAVHTRGLDFASDKPTTTPAPRPPTPAPTIASQPLSLRPEACRPAAGGAVHTRGLDFACDIYIWAPLAGTCGVLLLSLVITLYCNHRNKRGRKKLLYIFKQPFMRPVQTTQEEDGCSCRFPEEEEGGCELRVKFSRSADAPAYQQGQNQLYNELNLGRREEYDVLDKRRGRDPEMGGKPRRKNPQEGLYNELQKDKMAEAYSEIGMKGERRRGKGHDGLYQGLSTATKDTYDALHMQALPPR

SEQ ID NO: 239 - protein, 565 aa, synthetic construct
  REGION 1..565: note = source = /note="Description of Artificial Sequence: Synthetic polypeptide"
  REGION 1..565: note = source = /note="EGFRvIII CAR (MR1-1 scFv.CD8alpha 3x hinge &TM.4-1BB.CD3-zeta)"
DIELTQSPASLSVATGEKVTIRCMTSTDIDDDMNWYQQKPGEPPKFLISEGNTLRPGVPSRFSSSGTGTDFVFTIENTLSEDVGDYYCLQSWNVPLTFGDGTKLEIKGGGGSGGGGSGGGGSQVKLQQSGGGLVKPGASLKLSCVTSGFTFRKFGMSWVRQTSDKRLEWVASISTGGYNTYYSDNVKGRFTISRENAKNTLYLQMSSLKSEDTALYYCTRGYSPYSYAMDYWGQGTTVTVSSKPTTTPAPRPPTPAPTIASQPLSLRPEASRPAAGGAVHTRGLDFASDKPTTTPAPRPPTPAPTIASQPLSLRPEASRPAAGGAVHTRGLDFASDKPTTTPAPRPPTPAPTIASQPLSLRPEACRPAAGGAVHTRGLDFACDIYIWAPLAGTCGVLLLSLVITLYCNHRNKRGRKKLLYIFKQPFMRPVQTTQEEDGCSCRFPEEEEGGCELRVKFSRSADAPAYQQGQNQLYNELNLGRREEYDVLDKRRGRDPEMGGKPRRKNPQEGLYNELQKDKMAEAYSEIGMKGERRRGKGHDGLYQGLSTATKDTYDALHMQALPPR

SEQ ID NO: 240 - protein, 612 aa, synthetic construct
  REGION 1..612: note = source = /note="Description of Artificial Sequence: Synthetic polypeptide"
  REGION 1..612: note = source = /note="EGFRvIII CAR (MR1-1 scFv.CD8alpha 4x hinge &TM.4-1BB.CD3-zeta)"
DIELTQSPASLSVATGEKVTIRCMTSTDIDDDMNWYQQKPGEPPKFLISEGNTLRPGVPSRFSSSGTGTDFVFTIENTLSEDVGDYYCLQSWNVPLTFGDGTKLEIKGGGGSGGGGSGGGGSQVKLQQSGGGLVKPGASLKLSCVTSGFTFRKFGMSWVRQTSDKRLEWVASISTGGYNTYYSDNVKGRFTISRENAKNTLYLQMSSLKSEDTALYYCTRGYSPYSYAMDYWGQGTTVTVSSKPTTTPAPRPPTPAPTIASQPLSLRPEASRPAAGGAVHTRGLDFASDKPTTTPAPRPPTPAPTIASQPLSLRPEASRPAAGGAVHTRGLDFASDKPTTTPAPRPPTPAPTIASQPLSLRPEASRPAAGGAVHTRGLDFASDKPTTTPAPRPPTPAPTIASQPLSLRPEACRPAAGGAVHTRGLDFACDIYIWAPLAGTCGVLLLSLVITLYCNHRNKRGRKKLLYIFKQPFMRPVQTTQEEDGCSCRFPEEEEGGCELRVKFSRSADAPAYQQGQNQLYNELNLGRREEYDVLDKRRGRDPEMGGKPRRKNPQEGLYNELQKDKMAEAYSEIGMKGERRRGKGHDGLYQGLSTATKDTYDALHMQALPPR

SEQ ID NO: 241 - protein, 565 aa, synthetic construct
  REGION 1..565: note = source = /note="Description of Artificial Sequence: Synthetic polypeptide"
  REGION 1..565: note = source = /note="EGFRvIII CAR (huMR1-1 scFv.CD8alpha 3x hinge & TM.4-1BB.CD3-zeta)"
DIQMTQSPSSLSASVGDRVTITCMTSTDIDDDMNWYQQKPGKTPKLLIYEGNTLRPGVPSRFSGSGSGTDFIFTISSLQPEDIATYYCLQSWNVPLTFGGGTKVEIKGGGGSGGGGSGGGGSQVQLQESGGGLVKPGGSLKLSCAASGFTFSKFGMSWVRQTPDKRLEWVASISTGGYNTYYSDNVKGRFTISRDNAKNTLYLQMSSLKSEDTAMYYCARGYSPYSYAMDYWGQGTMVTVSSKPTTTPAPRPPTPAPTIASQPLSLRPEASRPAAGGAVHTRGLDFASDKPTTTPAPRPPTPAPTIASQPLSLRPEASRPAAGGAVHTRGLDFASDKPTTTPAPRPPTPAPTIASQPLSLRPEACRPAAGGAVHTRGLDFACDIYIWAPLAGTCGVLLLSLVITLYCNHRNKRGRKKLLYIFKQPFMRPVQTTQEEDGCSCRFPEEEEGGCELRVKFSRSADAPAYQQGQNQLYNELNLGRREEYDVLDKRRGRDPEMGGKPRRKNPQEGLYNELQKDKMAEAYSEIGMKGERRRGKGHDGLYQGLSTATKDTYDALHMQALPPR

SEQ ID NO: 242 - protein, 612 aa, synthetic construct
  REGION 1..612: note = source = /note="Description of Artificial Sequence: Synthetic polypeptide"
  REGION 1..612: note = source = /note="EGFRvIII CAR (huMR1-1 scFv.CD8alpha 4x hinge & TM.4-1BB.CD3-zeta)"
DIQMTQSPSSLSASVGDRVTITCMTSTDIDDDMNWYQQKPGKTPKLLIYEGNTLRPGVPSRFSGSGSGTDFIFTISSLQPEDIATYYCLQSWNVPLTFGGGTKVEIKGGGGSGGGGSGGGGSQVQLQESGGGLVKPGGSLKLSCAASGFTFSKFGMSWVRQTPDKRLEWVASISTGGYNTYYSDNVKGRFTISRDNAKNTLYLQMSSLKSEDTAMYYCARGYSPYSYAMDYWGQGTMVTVSSKPTTTPAPRPPTPAPTIASQPLSLRPEASRPAAGGAVHTRGLDFASDKPTTTPAPRPPTPAPTIASQPLSLRPEASRPAAGGAVHTRGLDFASDKPTTTPAPRPPTPAPTIASQPLSLRPEASRPAAGGAVHTRGLDFASDKPTTTPAPRPPTPAPTIASQPLSLRPEACRPAAGGAVHTRGLDFACDIYIWAPLAGTCGVLLLSLVITLYCNHRNKRGRKKLLYIFKQPFMRPVQTTQEEDGCSCRFPEEEEGGCELRVKFSRSADAPAYQQGQNQLYNELNLGRREEYDVLDKRRGRDPEMGGKPRRKNPQEGLYNELQKDKMAEAYSEIGMKGERRRGKGHDGLYQGLSTATKDTYDALHMQALPPR

SEQ ID NO: 243 - protein, 565 aa, synthetic construct
  REGION 1..565: note = source = /note="Description of Artificial Sequence: Synthetic polypeptide"
  REGION 1..565: note = source = /note="EGFRvIII CAR (huMR1-2 scFv.CD8alpha 3x hinge & TM.4-1BB.CD3-zeta)"
DIQMTQSPSSLSASVGDRVTITCMTSTDIDDDMNWYQQKPGKTPKLLIYEGNTLRPGVPSRFSGSGSGTDFIFTISSLQPEDIATYYCLQSWNVPLTFGGGTKVEIKGGGGSGGGGSGGGGSQVQLQESGGGLVKPGGSLKLSCAASGFTFSKFGMSWVRQTPDKRLEWVASISTGGYNTFYSDNVKGRFTISRDNAKNTLYLQMSSLKSEDTAMYYCARGYSPYSFAMDYWGQGTMVTVSSKPTTTPAPRPPTPAPTIASQPLSLRPEASRPAAGGAVHTRGLDFASDKPTTTPAPRPPTPAPTIASQPLSLRPEASRPAAGGAVHTRGLDFASDKPTTTPAPRPPTPAPTIASQPLSLRPEACRPAAGGAVHTRGLDFACDIYIWAPLAGTCGVLLLSLVITLYCNHRNKRGRKKLLYIFKQPFMRPVQTTQEEDGCSCRFPEEEEGGCELRVKFSRSADAPAYQQGQNQLYNELNLGRREEYDVLDKRRGRDPEMGGKPRRKNPQEGLYNELQKDKMAEAYSEIGMKGERRRGKGHDGLYQGLSTATKDTYDALHMQALPPR

SEQ ID NO: 244 - protein, 1836 aa, synthetic construct
  REGION 1..1836: note = source = /note="Description of Artificial Sequence: Synthetic polypeptide"
  REGION 1..1836: note = source = /note="EGFRvIII CAR (huMR1-2 scFv.CD8alpha 4x hinge & TM.4-1BB.CD3-zeta"
ASPILEGLNMETTHRGLNSERPROSERSERLEUSERALASERVALGLYASPARGVALTHRILETHRCYSMETTHRSERTHRASPILEASPASPASPMETASNTRPTYRGLNGLNLYSPROGLYLYSTHRPROLYSLEULEUILETYRGLUGLYASNTHRLEUARGPROGLYVALPROSERARGPHESERGLYSERGLYSERGLYTHRASPPHEILEPHETHRILESERSERLEUGLNPROGLUASPILEALATHRTYRTYRCYSLEUGLNSERTRPASNVALPROLEUTHRPHEGLYGLYGLYTHRLYSVALGLUILELYSGLYGLYGLYGLYSERGLYGLYGLYGLYSERGLYGLYGLYGLYSERGLNVALGLNLEUGLNGLUSERGLYGLYGLYLEUVALLYSPROGLYGLYSERLEULYSLEUSERCYSALAALASERGLYPHETHRPHESERLYSPHEGLYMETSERTRPVALARGGLNTHRPROASPLYSARGLEUGLUTRPVALALASERILESERTHRGLYGLYTYRASNTHRPHETYRSERASPASNVALLYSGLYARGPHETHRILESERARGASPASNALALYSASNTHRLEUTYRLEUGLNMETSERSERLEULYSSERGLUASPTHRALAMETTYRTYRCYSALAARGGLYTYRSERPROTYRSERPHEALAMETASPTYRTRPGLYGLNGLYTHRMETVALTHRVALSERSERLYSPROTHRTHRTHRPROALAPROARGPROPROTHRPROALAPROTHRILEALASERGLNPROLEUSERLEUARGPROGLUALASERARGPROALAALAGLYGLYALAVALHISTHRARGGLYLEUASPPHEALASERASPLYSPROTHRTHRTHRPROALAPROARGPROPROTHRPROALAPROTHRILEALASERGLNPROLEUSERLEUARGPROGLUALASERARGPROALAALAGLYGLYALAVALHISTHRARGGLYLEUASPPHEALASERASPLYSPROTHRTHRTHRPROALAPROARGPROPROTHRPROALAPROTHRILEALASERGLNPROLEUSERLEUARGPROGLUALASERARGPROALAALAGLYGLYALAVALHISTHRARGGLYLEUASPPHEALASERASPLYSPROTHRTHRTHRPROALAPROARGPROPROTHRPROALAPROTHRILEALASERGLNPROLEUSERLEUARGPROGLUALACYSARGPROALAALAGLYGLYALAVALHISTHRARGGLYLEUASPPHEALACYSASPILETYRILETRPALAPROLEUALAGLYTHRCYSGLYVALLEULEULEUSERLEUVALILETHRLEUTYRCYSASNHISARGASNLYSARGGLYARGLYSLYSLEULEUTYRILEPHELYSGLNPROPHEMETARGPROVALGLNTHRTHRGLNGLUGLUASPGLYCYSSERCYSARGPHEPROGLUGLUGLUGLUGLYGLYCYSGLULEUARGVALLYSPHESERARGSERALAASPALAPROALATYRGLNGLNGLYGLNASNGLNLEUTYRASNGLULEUASNLEUGLYARGARGGLUGLUTYRASPVALLEUASPLYSARGARGGLYARGASPPROGLUMETGLYGLYLYSPROARGARGLYSASNPROGLNGLUGLYLEUTYRASNGLULEUGLNLYSASPLYSMETALAGLUALATYRSERGLUILEGLYMETLYSGLYGLUARGARGARGGLYLYSGLYHISASPGLYLEUTYRGLNGLYLEUSERTHRALATHRLYSASPTHRTYRASPALALEUHISMETGLNALALEUPROPROARG